European Patent Specification EP 3 589 733 B1, published January 7, 2026. Title: METHODS AND COMPOSITIONS FOR TRANSDUCING AND EXPANDING LYMPHOCYTES AND REGULATING THE ACTIVITY THEREOF. Applicant: F1 Oncology, Inc. The sequence listing filed with the application follows.

SEQUENCE LISTING (521 sequences)

SEQ ID NO: 1 - protein, 42 aa, Homo sapiens
KRGRKKLLYIFKQPFMRPVQTTQEEDGCSCRFPEEEEGGCEL

SEQ ID NO: 2 - protein, 41 aa, Homo sapiens
RSKRSRLLHSDYMNMTPRRPGPTRKHYQPYAPPRDFAAYRS

SEQ ID NO: 3 - protein, 41 aa, Homo sapiens
RSKRSRLLHSDYMNMTPRRPGPTRKHYQAYAAARDFAAYRS

SEQ ID NO: 4 - protein, 35 aa, Homo sapiens
TKKKYSSSVHDPNGEYMFMRAVNTAKKSRLTDVTL

SEQ ID NO: 5 - protein, 37 aa, Homo sapiens
RRDQRLPPDAHKPPGGGSFRTPIQEEQADAHSTLAKI

SEQ ID NO: 6 - protein, 49 aa, Homo sapiens
HQRRKYRSNKGESPVEPAEPCRYSCPREEEGSTIPIQEDYRKPEPACSP

SEQ ID NO: 7 - protein, 114 aa, Homo sapiens
CCLRRHQGKQNELSDTAGREINLVDAHLKSEQTEASTRQNSQVLLSETGIYDNDPDLCFRMQEGSEVYSNPCLEENKPGIVYASLNHSVIGPNSRLARNVKEAPTEYASICVRS

SEQ ID NO: 8 - protein, 187 aa, Homo sapiens
RRACRKRIRQKLHLCYPVQTSQPKLELVDSRPRRSSTQLRSGASVTEPVAEERGLMSQPLMETCHSVGAAYLESLPLQDASPAGGPSSPRDLPEPRVSTEHTNNKIEKIYIMKADTVIVGTVKAELPEGRGLAGPAEPELEEELEADHTPHYPEQETEPPLGSCSDVMLSVEEEGKEDPLPTAASGK

SEQ ID NO: 9 - protein, 54 aa, Homo sapiens
HIWQLRSQCMWPRETQLLLEVPPSTEDARSCQFPEEERGERSAEEKGRLGDLWV

SEQ ID NO: 10 - protein, 60 aa, Homo sapiens
CVKRRKPRGDVVKVIVSVQRKRQEAEGEATVIEALQAPPDVTTVAVEETIPSFTGRSPNH

SEQ ID NO: 11 - protein, 163 aa, Homo sapiens
MKWKALFTAAILQAQLPITEAQSFGLLDPKLCYLLDGILFIYGVILTALFLRVKFSRSADAPAYQQGQNQLYNELNLGRREEYDVLDKRRGRDPEMGGKPRRKNPQEGLYNELQKDKMAEAYSEIGMKGERRRGKGHDGLYQGLSTATKDTYDALHMQALPPR

SEQ ID NO: 12 - protein, 164 aa, Homo sapiens
MKWKALFTAAILQAQLPITEAQSFGLLDPKLCYLLDGILFIYGVILTALFLRVKFSRSADAPAYQQGQNQLYNELNLGRREEYDVLDKRRGRDPEMGGKPQRRKNPQEGLYNELQKDKMAEAYSEIGMKGERRRGKGHDGLYQGLSTATKDTYDALHMQALPPR

SEQ ID NO: 13 - protein, 112 aa, Homo sapiens
RVKFSRSADAPAYQQGQNQLYNELNLGRREEYDVLDKRRGRDPEMGGKPRRKNPQEGLYNELQKDKMAEAYSEIGMKGERRRGKGHDGLYQGLSTATKDTYDALHMQALPPR

SEQ ID NO: 14 - protein, 21 aa, Homo sapiens
NQLYNELNLGRREEYDVLDKR

SEQ ID NO: 15 - protein, 22 aa, Homo sapiens
EGLYNELQKDKMAEAYSEIGMK

SEQ ID NO: 16 - protein, 21 aa, Homo sapiens
DGLYQGLSTATKDTYDALHMQ

SEQ ID NO: 17 - protein, 171 aa, Homo sapiens
MEHSTFLSGLVLATLLSQVSPFKIPIEELEDRVFVNCNTSITWVEGTVGTLLSDITRLDLGKRILDPRGIYRCNGTDIYKDKESTVQVHYRMCQSCVELDPATVAGIIVTDVIATLLLALGVFCFAGHETGRLSGAADTQALLRNDQVYQPLRDRDDAQYSHLGGNWARNK

SEQ ID NO: 18 - protein, 127 aa, Homo sapiens
MEHSTFLSGLVLATLLSQVSPFKIPIEELEDRVFVNCNTSITWVEGTVGTLLSDITRLDLGKRILDPRGIYRCNGTDIYKDKESTVQVHYRTADTQALLRNDQVYQPLRDRDDAQYSHLGGNWARNK

SEQ ID NO: 19 - protein, 21 aa, Homo sapiens
DQVYQPLRDRDDAQYSHLGGN

SEQ ID NO: 20 - protein, 206 aa, Homo sapiens
MQSGTHWRVLGLCLLSVGVWGQDGNEEMGGITQTPYKVSISGTTVILTCPQYPGSEILWQHNDKNIGGDEDDKNIGSDEDHLSLKEFSELEQSGYYVCYPRGSKPEDANFYLYLRARVCENCMEMDMSVATIVIVDICITGGLLLLVYYWSKNRKAKAKPVTRGAGAGGRQRGQNKERPPPVPNPDYEPIRKGQRDLYSGLNQRRI

SEQ ID NO: 21 - protein, 21 aa, Homo sapiens
NPDYEPIRKGQRDLYSGLNQR

SEQ ID NO: 22 - protein, 182 aa, Homo sapiens
MEQGKGLAVLILAIILLQGTLAQSIKGNHLVKVYDYQEDGSVLLTCDAEAKNITWFKDGKMIGFLTEDKKKWNLGSNAKDPRGMYQCKGSQNKSKPLQVYYRMCQNCIELNAATISGFLFAEIVSIFVLAVGVYFIAGQDGVRQSRASDKQTLLPNDQLYQPLKDREDDQYSHLQGNQLRRN

SEQ ID NO: 23 - protein, 21 aa, Homo sapiens
DQLYQPLKDREDDQYSHLQGN

SEQ ID NO: 24 - protein, 226 aa, Homo sapiens
MPGGPGVLQALPATIFLLFLLSAVYLGPGCQALWMHKVPASLMVSLGEDAHFQCPHNSSNNANVTWWRVLHGNYTWPPEFLGPGEDPNGTLIIQNVNKSHGGIYVCRVQEGNESYQQSCGTYLRVRQPPPRPFLDMGEGTKNRIITAEGIILLFCAVVPGTLLLFRKRWQNEKLGLDAGDEYEDENLYEGLNLDDCSMYEDISRGLQGTYQDVGSLNIGDVQLEKP

SEQ ID NO: 25 - protein, 188 aa, Homo sapiens
MPGGPGVLQALPATIFLLFLLSAVYLGPGCQALWMHKVPASLMVSLGEDAHFQCPHNSSNNANVTWWRVLHGNYTWPPEFLGPGEDPNEPPPRPFLDMGEGTKNRIITAEGIILLFCAVVPGTLLLFRKRWQNEKLGLDAGDEYEDENLYEGLNLDDCSMYEDISRGLQGTYQDVGSLNIGDVQLEKP

SEQ ID NO: 26 - protein, 21 aa, Homo sapiens
ENLYEGLNLDDCSMYEDISRG

SEQ ID NO: 27 - protein, 113 aa, Homo sapiens
MGGLEPCSRLLLLPLLLAVSGLRPVQAQAQSDCSCSTVSPGVLAGIVMGDLVLTVLIALAVYFLGRLVPRGRGAAEAATRKQRITETESPYQELQGQRSDVYSDLNTQRPYYK

SEQ ID NO: 28 - protein, 107 aa, Homo sapiens
MGGLEPCSRLLLLPLLLAVSGLRPVQAQAQSDCSCSTVSPGVLAGIVMGDLVLTVLIALAVYFLGRLVPRGRGAAEATRKQRITETESPYQELQGQRSDVYSDLNTQ

SEQ ID NO: 29 - protein, 102 aa, Homo sapiens
MGGLEPCSRLLLLPLLLAVSDCSCSTVSPGVLAGIVMGDLVLTVLIALAVYFLGRLVPRGRGAAEAATRKQRITETESPYQELQGQRSDVYSDLNTQRPYYK

SEQ ID NO: 30 - protein, 101 aa, Homo sapiens
MGGLEPCSRLLLLPLLLAVSDCSCSTVSPGVLAGIVMGDLVLTVLIALAVYFLGRLVPRGRGAAEATRKQRITETESPYQELQGQRSDVYSDLNTQRPYYK

SEQ ID NO: 31 - protein, 21 aa, Homo sapiens
ESPYQELQGQRSDVYSDLNTQ

SEQ ID NO: 32 - protein, 86 aa, Homo sapiens
MIPAVVLLLLLLVEQAAALGEPQLCYILDAILFLYGIVLTLLYCRLKIQVRKAAITSYEKSDGVYTGLSTRNQETYETLKHEKPPQ

SEQ ID NO: 33 - protein, 21 aa, Homo sapiens
DGVYTGLSTRNQETYETLKHE

SEQ ID NO: 34 - protein, 20 aa, Homo sapiens
RPRRSPAQDGKVYINMPGRG

SEQ ID NO: 35 - protein, 68 aa, Homo sapiens
FWVLVVVGGVLACYSLLVTVAFIIFWVRSKRSRLLHSDYMNMTPRRPGPTRKHYQPYAPPRDFAAYRS

SEQ ID NO: 36 - protein, 619 aa, Homo sapiens
MPDPAAHLPFFYGSISRAEAEEHLKLAGMADGLFLLRQCLRSLGGYVLSLVHDVRFHHFPIERQLNGTYAIAGGKAHCGPAELCEFYSRDPDGLPCNLRKPCNRPSGLEPQPGVFDCLRDAMVRDYVRQTWKLEGEALEQAIISQAPQVEKLIATTAHERMPWYHSSLTREEAERKLYSGAQTDGKFLLRPRKEQGTYALSLIYGKTVYHYLISQDKAGKYCIPEGTKFDTLWQLVEYLKLKADGLIYCLKEACPNSSASNASGAAAPTLPAHPSTLTHPQRRIDTLNSDGYTPEPARITSPDKPRPMPMDTSVYESPYSDPEELKDKKLFLKRDNLLIADIELGCGNFGSVRQGVYRMRKKQIDVAIKVLKQGTEKADTEEMMREAQIMHQLDNPYIVRLIGVCQAEALMLVMEMAGGGPLHKFLVGKREEIPVSNVAELLHQVSMGMKYLEEKNFVHRDLAARNVLLVNRHYAKISDFGLSKALGADDSYYTARSAGKWPLKWYAPECINFRKFSSRSDVWSYGVTMWEALSYGQKPYKKMKGPEVMAFIEQGKRMECPPECPPELYALMSDCWIYKWEDRPDFLTVEQRMRACYYSLASKVEGPPGSTQKAEAACA

SEQ ID NO: 37 - protein, 9 aa, Artificial sequence
  synthetic HA Epitope
YPYDVPDYA

SEQ ID NO: 38 - protein, 8 aa, Artificial sequence
  synthetic FLAG Epitope
DYKDDDDK

SEQ ID NO: 39 - protein, 10 aa, Artificial sequence
  synthetic c-myc Epitope
EQKLISEEDL

SEQ ID NO: 40 - protein, 5 aa, Artificial sequence
  synthetic His5 Affinity
HHHHH

SEQ ID NO: 41 - protein, 6 aa, Artificial sequence
  synthetic HisX6 Affinity
HHHHHH

SEQ ID NO: 42 - protein, 8 aa, Artificial sequence
  synthetic Strep Tag Affinity
WSHPQFEK

SEQ ID NO: 43 - protein, 5 aa, Artificial sequence
  synthetic HisX6 Affinity
RYIRS

SEQ ID NO: 44 - protein, 4 aa, Artificial sequence
  synthetic Affinity
FHHT

SEQ ID NO: 45 - protein, 17 aa, Artificial sequence
  synthetic Affinity
WEAAAREACCRECCARA

SEQ ID NO: 46 - protein, 24 aa, Homo sapiens
IYIWAPLAGTCGVLLLSLVITLYC

SEQ ID NO: 47 - protein, 23 aa, Homo sapiens
LGLLVAGVLVLLVSLGVAIHLCC

SEQ ID NO: 48 - protein, 25 aa, Homo sapiens
ALIVLGGVAGLLLFIGLGIFFCVRC

SEQ ID NO: 49 - protein, 23 aa, Homo sapiens
LCYLLDGILFIYGVILTALFLRV

SEQ ID NO: 50 - protein, 27 aa, Homo sapiens
FWVLVVVGGVLACYSLLVTVAFIIFWV

SEQ ID NO: 51 - protein, 26 aa, Homo sapiens
VAAILGLGLVLGLLGPLAILLALYLL

SEQ ID NO: 52 - protein, 24 aa, Homo sapiens
ALPAALAVISFLLGLGLGVACVLA

SEQ ID NO: 53 - protein, 15 aa, Artificial sequence
  synthetic Linker 1
GGGGSGGGGSGGGGS

SEQ ID NO: 54 - protein, 30 aa, Artificial sequence
  synthetic Linker 2
GGGGSGGGGSGGGGSGGGGSGGGGSGGGGS

SEQ ID NO: 55 - protein, 14 aa, Artificial sequence
  synthetic Linker 3
GGGGSGGGSGGGGS

SEQ ID NO: 56 - protein, 4 aa, Artificial sequence
  synthetic Linker 4
GGSG

SEQ ID NO: 57 - protein, 5 aa, Artificial sequence
  synthetic Linker 5
GGSGG

SEQ ID NO: 58 - protein, 5 aa, Artificial sequence
  synthetic Linker 6
GSGSG

SEQ ID NO: 59 - protein, 5 aa, Artificial sequence
  synthetic Linker 7
GSGGG

SEQ ID NO: 60 - protein, 5 aa, Artificial sequence
  synthetic Linker 8
GGGSG

SEQ ID NO: 61 - protein, 5 aa, Artificial sequence
  synthetic Linker 9
GSSSG

SEQ ID NO: 62 - protein, 4 aa, Artificial sequence
  synthetic Hinge 1
CPPC

SEQ ID NO: 63 - protein, 5 aa, Artificial sequence
  synthetic Hinge 2
DKTHT

SEQ ID NO: 64 - protein, 15 aa, Artificial sequence
  synthetic Hinge 3
CPEPKSCDTPPPCPR

SEQ ID NO: 65 - protein, 12 aa, Artificial sequence
  synthetic Hinge 4
ELKTPLGDTTHT

SEQ ID NO: 66 - protein, 10 aa, Artificial sequence
  synthetic Hinge 5
KSCDKTHTCP

SEQ ID NO: 67 - protein, 7 aa, Artificial sequence
  synthetic Hinge 6
KCCVDCP

SEQ ID NO: 68 - protein, 7 aa, Artificial sequence
  synthetic Hinge 7
KYGPPCP

SEQ ID NO: 69 - protein, 15 aa, Artificial sequence
  synthetic Hinge 8
EPKSCDKTHTCPPCP

SEQ ID NO: 70 - protein, 12 aa, Artificial sequence
  synthetic Hinge 9
ERKCCVECPPCP

SEQ ID NO: 71 - protein, 17 aa, Artificial sequence
  synthetic Hinge 10
ELKTPLGDTTHTCPRCP

SEQ ID NO: 72 - protein, 12 aa, Artificial sequence
  synthetic Hinge 11
SPNMVPHAHHAQ

SEQ ID NO: 73 - protein, 45 aa, Artificial sequence
  synthetic Hinge 12
TTTPAPRPPTPAPTIASQPLSLRPEACRPAAGGAVHTRGLDFACD

SEQ ID NO: 74 - protein, 21 aa, Homo sapiens
MALPVTALLLPLALLLHAARP

SEQ ID NO: 75 - protein, 69 aa, Homo sapiens
TTTPAPRPPTPAPTIASQPLSLRPEACRPAAGGAVHTRGLDFACDIYIWAPLAGTCGVLLLSLVITLYC

SEQ ID NO: 76 - protein, 66 aa, Homo sapiens
IEVMYPPPYLDNEKSNGTIIHVKGKHLCPSPLFPGPSKPFWVLVVVGGVLACYSLLVTVAFIIFWV

SEQ ID NO: 77 - protein, 21 aa, Artificial sequence
  synthetic 2A-1 Cleavage signal
GSGEGRGSLLTCGDVEENPGP

SEQ ID NO: 78 - protein, 357 aa, Homo sapiens
MLLLVTSLLLCELPHPAFLLIPRKVCNGIGIGEFKDSLSINATNIKHFKNCTSISGDLHILPVAFRGDSFTHTPPLDPQELDILKTVKEITGFLLIQAWPENRTDLHAFENLEIIRGRTKQHGQFSLAVVSLNITSLGLRSLKEISDGDVIISGNKNLCYANTINWKKLFGTSGQKTKIISNRGENSCKATGQVCHALCSPEGCWGPEPRDCVSCRNVSRGRECVDKCNLLEGEPREFVENSECIQCHPECLPQAMNITCTGRGPDNCIQCAHYIDGPHCVKTCPAGVMGENNTLVWKYADAGHVCHLCHPNCTYGCTGPGLEGCPTNGPKIPSIATGMVGALLLLLVVALGIGLFM

SEQ ID NO: 79 - protein, 45 aa, Homo sapiens; identical to SEQ ID NO: 73

SEQ ID NO: 80 - protein, 39 aa, Homo sapiens
IEVMYPPPYLDNEKSNGTIIHVKGKHLCPSPLFPGPSKP

SEQ ID NO: 81 - protein, 113 aa, Homo sapiens
RVKFSRSADAPAYQQGQNQLYNELNLGRREEYDVLDKRRGRDPEMGGKPQRRKNPQEGLYNELQKDKMAEAYSEIGMKGERRRGKGHDGLYQGLSTATKDTYDALHMQALPPR

SEQ ID NO: 82 - protein, 463 aa, Homo sapiens
MTILGTTFGMVFSLLQVVSGESGYAQNGDLEDAELDDYSFSCYSQLEVNGSQHSLTCAFEDPDVNTTNLEFEICGALVEVKCLNFRKLQEIYFIETKKFLLIGKSNICVKVGEKSLTCKKIDLTTIVKPEAPFDLSVIYREGANDFVVTFNTSHLQKKYVKVLMHDVAYRQEKDENKWTHVNLSSTKLTLLQRKLQPAAMYEIKVRSIPDHYFKGFWSEWSPSYYFRTPEINNSSGEMDPILLPPCLTISILSFFSVALLVILACVLWKKRIKPIVWPSLPDHKKTLEHLCKKPRKNLNVSFNPESFLDCQIHRVDDIQARDEVEGFLQDTFPQQLEESEKQRLGGDVQSPNCPSEDVVVTPESFGRDSSLTCLAGNVSACDAPILSSSRSLDCRESGKNGPHVYQDLLLSLGTTNSTLPPPFSLQSGILTLNPVAQGQPILTSLGSNQEEAYVTMSSFYQNQ

SEQ ID NO: 83 - DNA, 13673 bp, Artificial sequence
  synthetic Dox-rapamycin inducible lentiviral genome with riboswitch
gatatctataacaagaaaatatatatataataagttatcacgtaagtagaacatgaaataacaatataattatcgtatgagttaaatcttaaaagtcacgtaaaagataatcatgcgtcattttgactcacgcggtcgttatagttcaaaatcagtgacacttaccgcattgacaagcacgcctcacgggagctccaagcggcgactgagatgtcctaaatgcacagcgacggattcgcgctatttagaaagagagagcaatatttcaagaatgcatgcgtcaattttacgcagactatctttctagggttaagacggatcgggagatctcccgatcccctatggtgcactctcagtacaatctgctctgatgccgcatagttaagccagtatctgctccctgcttgtgtgttggaggtcgctgagtagtgcgcgagcaaaatttaagctacaacaaggcaaggcttgaccgacaattgcatgaagaatctgcttagggttaggcgttttgcgctgcttcgcgatgtacgggccagatatacgcgttgacattgattattgactagttattaatagtaatcaattacggggtcattagttcatagcccatatatggagttccgcgttacataacttacggtaaatggcccgcctggctgaccgcccaacgacccccgcccattgacgtcaataatgacgtatgttcccatagtaacgccaatagggactttccattgacgtcaatgggtggagtatttacggtaaactgcccacttggcagtacatcaagtgtatcatatgccaagtacgccccctattgacgtcaatgacggtaaatggcccgcctggcattatgcccagtacatgaccttatgggactttcctacttggcagtacatctacgtattagtcatcgctattaccatggtgatgcggttttggcagtacatcaatgggcgtggatagcggtttgactcacggggatttccaagtctccaccccattgacgtcaatgggagtttgttttggaaccaaaatcaacgggactttccaaaatgtcgtaacaactccgccccattgacgcaaatgggcggtaggcgtgtacggtgggaggtctatataagcagagctctccctatcagtgatagagatctccctatcagtgatagagatcgtcgacgagctcgtttagtgaaccgtcagatcgcctggagacgccctcgaagccgcggtgcgggtgccagggcgtgccctgggtctctctggttagaccagatctgagcctgggagctctctggctaactagggaacccactgcttaagcctcaataaagcttgccttgagtgcttcaagtagtgtgtgcccgtctgttgtgtgactctggtaactagagatccctcagacccttttagtcagtgtggaaaatctctagcagtggcgcccgaacagggacttgaaagcgaaagggaaaccagaggagctctctcgacgcaggactcggcttgctgaagcgcgcacggcaagaggcgaggggcggcgactggtgagtacgccaaaaattttgactagcggaggctagaaggagagagatgggtgcgagagcgtcagtattaagcgggggagaattagatcgcgatgggaaaaaattcggttaaggccagggggaaagaaaaaatataaattaaaacatatagtatgggcaagcagggagctagaacgattcgcagttaatcctggcctgttagaaacatcagaaggctgtagacaaatactgggacagctacaaccatcccttcagacaggatcagaagaacttagatcattatataatacagtagcaaccctctattgtgtgcatcaaaggatagagataaaagacaccaaggaagctttagacaagatagaggaagagcaaaacaaaagtaagaccaccgcacagcaagcggccgctgatcttcagacctggaggaggagatatgagggacaattggagaagtgaattatataaatataaagtagtaaaaattgaaccattaggagtagcacccaccaaggcaaagagaagagtggtgcagagagaaaaaagagcagtgggaataggagctttgttccttgggttcttgggagcagcaggaagcactatgggcgcagcgtcaatgacgctgacggtacaggccagacaattattgtctggtatagtgcagcagcagaacaatttgctgagggctattgaggcgcaacagcatctgttgcaactcacagtctggggcatcaagcagctccaggcaagaatcctggctgtggaaagatacctaaaggatcaacagctcctggggatttggggttgctctggaaaactcatttgcaccactgctgtgccttggaatgctagttggagtaataaatctctggaacagatttggaatcacacgacctggatggagtgggacagagaaattaacaattacacaagcttaatacactccttaattgaagaatcgcaaaaccagcaagaaaagaatgaacaagaattattggaattagataaatgggcaagtttgtggaattggtttaacataacaaattggctgtggtatataaaattattcataatgatagtaggaggcttggtaggtttaagaatagtttttgctgtactttctatagtgaatagagttaggcagggatattcaccattatcgtttcagacccacctcccaaccccgaggggacccgacaggcccgaaggaatagaagaagaaggtggagagagagacagagacagatccattcgattagtgaacggatctcgacggtatcgattagactgtagcccaggaatatggcagctagattgtacacatttagaaggaaaagttatcttggtagcagttcatgtagccagtggatatatagaagcagaagtaattccagcagagacagggcaagaaacagcatacttcctcttaaaattagcaggaagatggccagtaaaaacagtacatacagacaatggcagcaatttcaccagtactacagttaaggccgcctgttggtgggcggggatcaagcaggaatttggcattccctacaatccccaaagtcaaggagtaatagaatctatgaataaagaattaaagaaaattataggacaggtaagagatcaggctgaacatcttaagacagcagtacaaatggcagtattcatccacaattttaaaagaaaaggggggattggggggtacagtgcaggggaaagaatagtagacataatagcaacagacatacaaactaaagaattacaaaaacaaattacaaaaattcaaaattttcgggtttattacagggacagcagagatccagtttggctgcattgatcacgtgaggggctctagactctagacacacaaaaaaccaacacacagatctaatgaaaataaagatcttttattgagaaacttatacagggtagcataatgggctactgaccccgccttcaaacctatttggagactataagtgaaaattatcactggttttggtagaagctggacatggtgacatatgcttcttcttgatttgatcccagggaagtaagaatgggctgaccctgagcaactgggttcaatgtcaggattccagattggagagaaaatggagggggcagcgtgctgtttgtagtcccaaggctaagcaggaggtcctggtacacatgaggcccattcttgccactctccctgcagtctagggacctggaagaggagagaataggggcgtcacatgcactgacattcccagccaggcatgtgagggatgaatctcttccaaagctttctggagtgacgactacatcctcagatgggcagttggggctctgcacatcccctccaagcctctgcttctcagattcttctagttgctgaggaaacgtatcttgcagaaaaccttccacttcatctctagcttgaatgtcatccaccctatgaatctggcagtccaggaaactttcaggattgaaactcacatttaaattttttcttggtttcttacaaagatgttccagagtcttcttatgatcggggagactgggccatacgataggcttaatcctttttttccataacacacaggccaagatgaccaacagagcgacagagaaaaaactcaaaatgctgatggtcaggcatggtggtagtaagataggatccatctcccctgagctattattgatctctggagttctgaagtaataacttggactccattcactccagaagcctttaaaatagtgatcagggatggatcgaactttaatctcatacattgctgccggttggagctttctctgcaggagtgtcagctttgtgctggataaattcacatgcgtccatttgttttcatccttttcctggcggtaagctacatcatgcattaaaacttttacatacttcttttgcaagtgtgatgtattaaatgtcaccacaaagtcattggctccttcccgatagatgacactcaggtcaaaaggagcctcaggtttaactatagtggttaggtctatttttttgcaggttagactcttttctccaaccttcacacatatattgctctttccaatcagtaagaatttctttgtctcgatgaaatatatctcttgtagtttcctgaaattcaggcactttacctccacgagggccccacatatttcaaattccagattggtggtgttgacatctgggtcctcaaaagcacatgtcagtgaatgctgcgatccattcacttccaactggctatagcatgagaatgagtagtcatccagttctgcatcttccaagtctccattttgagcatagccactttctccagaaacgacttgaagtaaagaaaaaaccatgccaaaagttgtacctagaattgtcattgggccgggattttcctccacgtccccgcatgttagtagacttcccctgccctcgccggagcgagggggcagggcctgcatgtgaagggcgtcgtaggtgtccttggtggctgtactgagaccctggtaaaggccatcgtgccccttgcccctccggcgctcgcctttcatcccaatctcactgtaggcctccgccatcttatctttctgcagttcattgtacaggccttcctgagggttcttccttctcggctttccccccatctcagggtcccggccacgtctcttgtccaaaacatcgtactcctctcttcgtcctagattgagctcgttatagagctggttctggccctgcttgtacgcgggggcgtctgcgctcctgctgaacttcactctcagttcacatcctccttcttcttcttctggaaatcggcagctacagccatcttcctcttgagtagtttgtactggtctcataaatggttgtttgaatatatacaggagtttctttctgccccgtttgcagtaaagggtgataaccagtgacaggagaaggaccccacaagtcccggccaagggcgcccagatgtagatatcacaggcgaagtccagccccctcgtgtgcactgcgccccccgccgctggccggcacgcctctgggcgcagggacaggggctgcgacgcgatggtgggcgccggtgttggtggtcgcggcgctggcgtcgtggttgaggagacggtgactgaggttccttggccccagtagtccatagcatagctaccaccgtagtaataatgtttggcacagtagtaaatggctgtgtcatcagtttgcagactgttcatttttaagaaaacttggctcttggagttgtccttgatgatggtcagtctggatttgagagctgaattatagtatgtggtttcactaccccatattactcccagccactccagaccctttcgtggaggctggcgaatccagcttacaccatagtcgggtaatgagacccctgagacagtgcatgtgacggacaggctctgtgagggcgccaccaggccaggtcctgactcctgcagtttcacctcagatccgccgccacccgacccaccaccgcccgagccaccgccacctgtgatctccagcttggtcccccctccgaacgtgtacggaagcgtattaccctgttggcgaagtaggtggcaatatcttcttgctccaggttgctaattgtcagagaataatctgttccagacccactgccactgaaccttgatgggactcctgagtgtaatcttgatgtatggtagatcaggagtttaacagttccatctggtttctgctgataccaatttaaatatttactaatgtcctgacttgccctgcaactgatggtgactctgtctcccagagaggcagacagggaggatgtagtctgtgtcatctggatgtccggcctggcggcgtggagcagcaaggccagcggcaggagcaaggcggtcactggtaaggccatggatcctctagatcacgacacctgaaatggaagaaaaaaactttgaaccactgtctgaggcttgagaatgaaccaagatccaaactcaaaaagggcaaattccaaggagaattacatcaagtgccaagctggcctaacttcagtctccacccactcagtgtggggaaactccatcgcataaaacccctccccccaacctaaagacgacgtactccaaaagctcgagaactaatcgaggtgcctggacggcgcccggtactcagtggagtcacatgaagcgacggctgaggacggaaaggcccttttcctttgtgtgggagaaacttatacagggtagcataatgggctactgaccccgccttcaaacctatttggagactataagtgaaaatgactcacccgcccgctctcccggcaccttcatcttgtcctttccctcagaaagaggctgggaggcagaggctgaggcagcggtggccgggacggttaggagaaaaggagtctctgctggttttattctgcagctacctccccaggaagtggaggactgtggggcctttgagaagcacctgccgacagggccaagaaattcgcactccccctttcggttcacaggcaggaagccctggaggtttgagggtttggggtgtgtgtatgtatctgtctgtctgaattttgctttttctctcatttgaccattgttttaatgctcctttttttaaaaaaaataattcttatctaattcctatcttgattggtaaagtccatctctaggcaaatacaagttctcgatggaaaacaataagtaatgtaaaatacagcatagcaaaactttaacctccaaatcaagcctctacttgaatccttttctgagggatgaataaggcataggcatcaggggctgttgccaatgtgcattagctgtttgcagcctcaccttctttcatggagtttaagatatagtgtattttcccaaggtttgaactagctcttcatttctttatgttttaaatgcactgacctcccacattccctttttagtaaaatattcagaaataatttaaatacatcattgcaatgaaaataaatgttttttattaggcagaatccagatgctcaaggcccttcataatatcccccagtttagtagttggacttagggaacaaaggaacctttaatagaaattggacagcaagaaagcgagcttagtgatacttgtgatcctctagatcacgacacctgaaatggaagaaaaaaactgcaccttcatcttgtcctttccctcagaaagaggctgggaggcagaggctgaggcagcggtggccgggacggttaggagaaaaggagtctctgctggttttattctgcagctacctccccaggaagtggaggactgtggggcctttgagaagcacctgccgacagggccaagaaattcgcactccccctttcggttcacaggcaggaagccctggaggtttgagggtttggggtgtgtgtatgtatctgtctgtctgaattttgctttttctctcatttgaccattgttttaatgctcctttttttaaaaaaaataattcttatctaattcctatcttgattggtaaagtccatctctaggcaaatacaagttctcgatggaaaacaataagtaatgtaaaatacagcatagcaaaactttaacctccaaatcaagcctctacttgaatccttttctgagggatgaataaggcataggcatcaggggctgttgccaatgtgcattagctgtttgcagcctcaccttctttcatggagtttaagatatagtgtattttcccaaggtttgaactagctcttcatttctttatgttttaaatgcactgacctcccacattccctttttagtaaaatattcagaaataatttaaatacatcattgcaatgaaaataaatgttttttattaggcagaatccagatgctcaaggcccttcataatatcccccagtttagtagttggacttagggaacaaaggaacctttaatagaaattggacagcaagaaagcgagcttagtgatacttgtaaaaagagacgcgtctctaaaagtcctttccatggctgctcgcctgtgttgccacctggattctgcgcgggacgtccttctgctacgtcccttcggccctcaatccagcggaccttccttcccgcggcctgctgccggctctgcggcctcttccgcgtcttcgccttcgccctcagacgagtcggatctccctttgggccgcctccccgcctggaattcgagctcggtacctttaagaccaatgacttacaaggcagctgtagatcttagccactttttaaaagaaaaggggggactggaagggctaattcactcccaacgaagacaagatctgctttttgcttgtactgggtctctctggttagaccagatctgagcctgggagctctctggctaactagggaacccactgcttaagcctcaataaagcttgccttgagtgcttcaagtagtgtgtgcccgtctgttgtgtgactctggtaactagagatccctcagacccttttagtcagtgtggaaaatctctagcagtagtagttcatgtcatcttattattcagtatttataacttgcaaagaaatgaatatcagagagtgagaggaacttgtttattgcagcttataatggttacaaataaagcaatagcatcacaaatttcacaaataaagcatttttttcactgcattctagttgtggtttgtccaaactcatcaatgtatcttatcatgtctggctctagctatcccgcccctaactccgcccatcccgcccctaactccgcccagttccgcccattctccgccccatggctgactaattttttttatttatgcagaggccgaggccgcctcggcctctgagctattccagaagtagtgaggaggcttttttggaggcctagggacgtatggccacaacctgggctccccgggcgcgtactccacctcacccatcatccacgctgttttatgagtaaaggagaagaacttttcactggagttgtcccaattcttgttgaattagatggtgatgttaatgggcacaaattttctgtcagtggagagggtgaaggtgatgcaacatacggaaaacttacccttaaatttatttgcactactggaaaactacctgttccatggccaacacttgtcactactttctcttatggtgttcaatgcttttcaagatacccagatcatatgaaacggcatgactttttcaagagtgccatgcccgaaggttatgtacaggaaagaactatatttttcaaagatgacgggaactacaagacacgtgctgaagtcaagtttgaaggtgatacccttgttaatagaatcgagttaaaaggtattgattttaaagaagatggaaacattcttggacacaaattggaatacaactataactcacacaatgtatacatcatggcagacaaacaaaagaatggaatcaaagttaacttcaaaattagacacaacattgaagatggaagcgttcaactagcagaccattatcaacaaaatactccaattggcgatggccctgtccttttaccagacaaccattacctgtccacacaatctgccctttcgaaagatcccaacgaaaagagagaccacatggtccttcttgagtttgtaacagctgctgggattacacatggcatggatgaactatacaaataggacctccatagaagacaccgggaccgatccaataacttcgtatagcatacattatacgaagttatgcctccggactctagcgtttaaacttaagcttgggaagttcctattccgaagttcctattctctagaaagtataggaacttctaccgagctcggatccactagtccagtgtggtggaattctgcagatatccagcacagtggcggccgctcgagtctagagggcccgtttaaacccgctgatcagcctcgactgtgccttctagttgccagccatctgttgtttgcccctcccccgtgccttccttgaccctggaaggtgccactcccactgtcctttcctaataaaatgaggaaattgcatcgcattgtctgagtaggtgtcattctattctggggggtggggtggggcaggacagcaagggggaggattgggaagacaatagcaggcatgctggggatgcggtgggctctatggcttctgaggcggaaagttaaccctagaaagataatcatattgtgacgtacgttaaagataatcatgcgtaaaattgacgcatgtgttttatcggtctgtatatcgaggtttatttattaatttgaatagatattaagttttattatatttacacttacatactaataataaattcaacaaacaatttatttatgtttatttatttattaaaaaaaaacaaaaactcaaaatttcttctataaagtaacaaaaaccagctggggctcgaagttcctatactttctagagaataggaacttctatagtgagtcgaataagggcgacacaaaatttattctaaatgcataataaatactgataacatcttatagtttgtattatattttgtattatcgttgacatgtataattttgatatcaaaaactgattttccctttattattttcgagatttattttcttaattctctttaacaaactagaaatattgtatatacaaaaaatcataaataatagatgaatagtttaattataggtgttcatcaatcgaaaaagcaacgtatcttatttaaagtgcgttgcttttttctcatttataaggttaaataattctcatatatcaagcaaagtgacaggcgcccttaaatattctgacaaatgctctttccctaaactccccccataaaaaaacccgccgaagcgggtttttacgttatttgcggattaacgattactcgttatcagaaccgcccagggggcccgagcttaagactggccgtcgttttacaacacagaaagagtttgtagaaacgcaaaaaggccatccgtcaggggccttctgcttagtttgatgcctggcagttccctactctcgccttccgcttcctcgctcactgactcgctgcgctcggtcgttcggctgcggcgagcggtatcagctcactcaaaggcggtaatacggttatccacagaatcaggggataacgcaggaaagaacatgtgagcaaaaggccagcaaaaggccaggaaccgtaaaaaggccgcgttgctggcgtttttccataggctccgcccccctgacgagcatcacaaaaatcgacgctcaagtcagaggtggcgaaacccgacaggactataaagataccaggcgtttccccctggaagctccctcgtgcgctctcctgttccgaccctgccgcttaccggatacctgtccgcctttctcccttcgggaagcgtggcgctttctcatagctcacgctgtaggtatctcagttcggtgtaggtcgttcgctccaagctgggctgtgtgcacgaaccccccgttcagcccgaccgctgcgccttatccggtaactatcgtcttgagtccaacccggtaagacacgacttatcgccactggcagcagccactggtaacaggattagcagagcgaggtatgtaggcggtgctacagagttcttgaagtggtgggctaactacggctacactagaagaacagtatttggtatctgcgctctgctgaagccagttaccttcggaaaaagagttggtagctcttgatccggcaaacaaaccaccgctggtagcggtggtttttttgtttgcaagcagcagattacgcgcagaaaaaaaggatctcaagaagatcctttgatcttttctacggggtctgacgctcagtggaacgacgcgcgcgtaactcacgttaagggattttggtcatgagcttgcgccgtcccgtcaagtcagcgtaatgctctgcttttagaaaaactcatcgagcatcaaatgaaactgcaatttattcatatcaggattatcaataccatatttttgaaaaagccgtttctgtaatgaaggagaaaactcaccgaggcagttccataggatggcaagatcctggtatcggtctgcgattccgactcgtccaacatcaatacaacctattaatttcccctcgtcaaaaataaggttatcaagtgagaaatcaccatgagtgacgactgaatccggtgagaatggcaaaagtttatgcatttctttccagacttgttcaacaggccagccattacgctcgtcatcaaaatcactcgcatcaaccaaaccgttattcattcgtgattgcgcctgagcgaggcgaaatacgcgatcgctgttaaaaggacaattacaaacaggaatcgagtgcaaccggcgcaggaacactgccagcgcatcaacaatattttcacctgaatcaggatattcttctaatacctggaacgctgtttttccggggatcgcagtggtgagtaaccatgcatcatcaggagtacggataaaatgcttgatggtcggaagtggcataaattccgtcagccagtttagtctgaccatctcatctgtaacatcattggcaacgctacctttgccatgtttcagaaacaactctggcgcatcgggcttcccatacaagcgatagattgtcgcacctgattgcccgacattatcgcgagcccatttatacccatataaatcagcatccatgttggaatttaatcgcggcctcgacgtttcccgttgaatatggctcatattcttcctttttcaatattattgaagcatttatcagggttattgtctcatgagcggatacatatttgaatgtatttagaaaaataaacaaataggggtcagtgttacaaccaattaaccaattctgaacattatcgcgagcccatttatacctgaatatggctcataacaccccttgtttgcctggcggcagtagcgcggtggtcccacctgaccccatgccgaactcagaagtgaaacgccgtagcgccgatggtagtgtggggactccccatgcgagagtagggaactgccaggcatcaaataaaacgaaaggctcagtcgaaagactgggcctttcgcccgggctaattagggggtgtcgcccttattcgactctatagtgaagttcctattctctagaaagtataggaacttctgaagt

SEQ ID NO: 84 - DNA, 15025 bp, Artificial sequence
  synthetic Dox-rapamycin inducible GAG POL ENV
gatatctataacaagaaaatatatatataataagttatcacgtaagtagaacatgaaataacaatataattatcgtatgagttaaatcttaaaagtcacgtaaaagataatcatgcgtcattttgactcacgcggtcgttatagttcaaaatcagtgacacttaccgcattgacaagcacgcctcacgggagctccaagcggcgactgagatgtcctaaatgcacagcgacggattcgcgctatttagaaagagagagcaatatttcaagaatgcatgcgtcaattttacgcagactatctttctagggttaagacggatcgggagatctcccgatcccctatggtgcactctcagtacaatctgctctgatgccgcatagttaagccagtatctgctccctgcttgtgtgttggaggtcgctgagtagtgcgcgagcaaaatttaagctacaacaaggcaaggcttgaccgacaattgcatgaagaatctgcttagggttaggcgttttgaagttcctatactttctagagaataggaacttcggaataggaacttcggatgcaatttcctcattttattaggaaaggacagtgggagtggcaccttccagggtcaaggaaggcacgggggaggggcaaacaacagatggctggcaactagaaggcacagcgttagtgatacttgtgggccagggcattagccacaccagccaccactttctgataggcagcctgcactggtggggtgaattccgcggaagcttgtgtaattgttaatttctctgtcccactccatccaggtcgtgtgattccaaatctgttccagagatttattactccaactagcattccaaggcacagcagtggtgcaaatgagttttccagagcaaccccaaatccccaggagctgttgatcctttaggtatctttccacagccaggattcttgcctggagctgcttgatgccccagactgtgagttgcaacagatgctgttgcgcctcaatagccctcagcaaattgttctgctgctgcactataccagacaataattgtctggcctgtaccgtcagcgtcattgacgctgcgcccatagtgcttcctgctgctcccaagaacccaaggaacaaagctcctgcggccgctccggaattccatgtgttaatcctcatcctgtctacttgccacacaatcatcacctgccatctgttttccataatccctgatgatctttgcttttcttcttggcactacttttatgtcactattatcttgtattactactgccccttcacctttccagaggagctttgctggtcctttccaaactggatctctgctgtccctgtaataaacccgaaaattttgaatttttgtaatttgtttttgtaattctttagtttgtatgtctgttgctattatgtctactattctttcccctgcactgtaccccccaatccccccttttcttttaaaattgtggatgaatactgccatttgtactgctgtcttaagatgttcagcctgatctcttacctgtcctataattttctttaattctttattcatagattctattactccttgactttggggattgtagggaatgccaaattcctgcttgatccccgcccaccaacaggcggccttaactgtagtactggtgaaattgctgccattgtctgtatgtactgtttttactggccatcttcctgctaattttaagaggaagtatgctgtttcttgccctgtctctgctggaattacttctgcttctatatatccactggctacatgaactgctaccaagataacttttccttctaaatgtgtacaatctagctgccatattcctgggctacagtctacttgtccatgcatggcttccccttttagctgacatttatcacagctggctactatttcttttgctactacaggtggtaggttaaaatcactagccattgctctccaattactgtgatatttctcatgttcttcttgggccttatctattccatctaaaaatagtactttcctgattccagcactgaccaatttatctacttgttcatttcctccaattcctttgtgtgctggtacccatgccaggtagactttttccttttttattaactgctctattatttgactgactaactctgattcactcttatctggttgtgcttgaatgattcccaatgcatattgtgagtctgtcactatgtttacttctaatcccgaatcctgcaaagctagatgaattgcttgtaactcagtcttctgatttgttgtgtccgttagggggacaactttttgtcttcctctgtcagttacatatcctgcttttcctaatttagtttccctattggctgccccatctacatagaaagtttctgctcctattatgggttctttctctaactggtaccataacttcactaagggaggggtattgacaaactcccactcaggaatccaggtggcttgccaatactctgtccaccatgcttcccatgtttccttttgtatgggtaatttaaatttaggagtctttccccatattactatgctttctgtggctattttttgtactgcctctgttaattgtttcacatcattagtgtgggcacccttcattcttgcatactttcctgttttcagatttttaaatggctcttgataaatttgatatgtccattggccttgcccctgcttctgtatttctgctattaagtcttttgatgggtcataatacactccatgtaccggttcttttagaatctccctgttttctgccagttctagctctgcttcttctgttagtggtactacttctgttagtgctttggttcccctaagaagtttacataattgccttactttaatccctgcataaatctgacttgcccaattcaattttcccactaatttctgtatgtcattgacagtccagctgtccttttctggcagcactataggctgtactgtccatttatcaggatggagttcataacccatccaaaggaatggaggttctttctgatgttttttgtctggtgtggtaaatccccacctcaacagatgttgtctcagttcctctatttttgttctatgctgccctatttctaagtcagatcctacatacaaatcatccatgtattgatagatgactatgtctggattttgttttctaaaaggctctaagatttttgtcatgctacactggaatattgctggtgatcctttccatccctgtggaagcacattgtactgatatctaatccctggtgtctcattgtttatactaggtatggtaaatgcagtatacttcctgaagtctttatctaagggaactgaaaaatatgcatcgcccacatccagtactgttactgattttttctgttttaaccctgcaggatgtggtattcctaattgaacttcccagaaatcttgagttctcttattaagttctctgaaatctactaattttctccatttagtactgtcttttttctttatggcaaatactggagtattgtatggattttcaggcccaatttttgaaatttttccttccttttccatttctgtacaaatttctactaatgcttttattttttcttctgtcaatggccattgtttaacttttgggccatccattcctggctttaattttactggtacagtctcaataggactaatgggaaaatttaaagtgcagccaatctgagtcaacagatttcttccaattatgttgacaggtgtaggtcctactaatactgtacctatagctttatgtccgcagatttctatgagtatctgatcatactgtcttactttgataaaacctccaattccccctatcatttttggtttccatcttcctggcaaattcatttcttctaatactgtatcatctgctcctgtatctaatagagcttcctttaattgcccccctatctttattgtgacgaggggtcgctgccaaagagtgatctgagggaagctaaaggatacagttccttgtctatcggctcctgcttctgagagggagttgttgtctcttccccaaacctgaagctctcttctggtggggctgttggctctggtctgctctgaagaaaattccctggccttcccttgtgggaaggccagatcttccctaaaaaattagcctgtctctcagtacaatctttcatttggtgtccttcctttccacatttccaacagccctttttcctaggggccctgcaatttttggctatgtgcccttctttgccacaattgaaacacttaacagtctttctttggttcctaaaattgcctttctgtatcattatggtagctggatttgttacttggctcattgcttcagccaaaactcttgctttatggccgggtccccccactccctgacatgctgtcatcatttcttctagtgtcgctcctggtcccaatgcttttaaaatagtcttacaatctgggttcgcattttggaccaacaaggtttctgtcatccaattttttacctcttgtgaagcttgctcggctcttagagttttatagaatcggtctacatagtctctaaagggttcctttggtccttgtcttatgtccagaatgctggtagggctatacattcttactattttatttaatcccaggattatccatcttttatagatttctcctactgggataggtggattatgtgtcatccatcctatttgttcctgaagggtactagtagttcctgctatgtcacttccccttggttctctcatctggcctggtgcaataggccctgcatgcactggatgcactctatcccattctgcagcttcctcattgatggtctcttttaacatttgcatggctgcttgatgtccccccactgtgtttagcatggtgtttaaatcttgtggggtggctccttctgataatgctgaaaacatgggtatcacttctgggctgaaagccttctcttctactacttttacccatgcatttaaagttctaggtgatatggcctgatgtaccatttgcccctggatgttctgcactatagggtaattttggctgacctgattgctgtgtcctgtgtcagctgctgcttgctgtgcttttttcttacttttgttttgctcttcctctatcttgtctaaagcttccttggtgtcttttatctctatcctttgatgcacacaatagagggttgctactgtattatataatgatctaagttcttctgatcctgtctgaagggatggttgtagctgtcccagtatttgtctacagccttctgatgtttctaacaggccaggattaactgcgaatcgttctagctccctgcttgcccatactatatgttttaatttatattttttctttccccctggccttaaccgaattttttcccatcgatctaattctcccccgcttaatactgacgctctcgcacccatggcggcggcagatctcgaattcagatctcacgtgctttgccaaagtgatgggccagcacacagaccagcacgttgcccaggagctgtgggaggaagataagaggtatgaacatgattagcaaaagggcctagcttggactcagaataatccagccttatcccaaccataaaataaaagcagaatggtagctggattgtagctgctattagcaatatgaaacctcttacatcagttacaatttatatgcagaaatatttatatgcagaaatattgctattgccttaacccagaaattatcactgttattctttagaatggtgcaaagaggcatgatacattgtatcattattgccctgaaagaaagagattagggaaagtattagaaataagataaacaaaaaagtatattaaaagaagaaagcattttttaaaattacaaatgcaaaattaccctgatttggtcaatatgtgtaccctgttacttctccccttcctatgacatgaacttaaccatagaaaagaaggggaaagaaaacatcaagggtcccatagactcaccctgaagttctcaggatccgagctcggtaccacatgtaagcttcgaggggaggctggatcggtcccggtgtcttctatggaggtcaaaacagcgtggatggcgtctccaggcgatctgacggttcactaaacgctgcttcgcgatgtacgggccagatatacgcgttgcgatctgacggttcactaaacgagctctgcttatataggcctcccaccgtacacgccacctcgacatactcgagtttactccctatcagtgatagagaacgtatgaagagtttactccctatcagtgatagagaacgtatgcagactttactccctatcagtgatagagaacgtataaggagtttactccctatcagtgatagagaacgtatgaccagtttactccctatcagtgatagagaacgtatctacagtttactccctatcagtgatagagaacgtatatccagtttactccctatcagtgatagagaacgtataagctttaggcgtgtacggtgggcgcctataaaagcagagctcgtttagtgaaccgtcagatcgcctggagcaattccacaacacttttgtcttataccaactttccgtaccacttcctaccctcgtaaatcgtcgacgagctcgtttagtgaaccgtcagatcgcctggagacgccctcgaagccgcggtgcgggtgccagggcgtgcccttgggctccatgtccatcatgggtctcaaggtgaacgtctctgccatattcatggcagtactgttaactctccaaacacccaccggtcaaatccattggggcaatctctctaagataggggtggtaggaataggaagtgcaagctacaaagttatgactcgttccagccatcaatcattagtcataaaattaatgcccaatataactctcctcaataactgcacgagggtagagattgcagaatacaggagactactgagaacagttttggaaccaattagagatgcacttaatgcaatgacccagaatataagaccggttcagagtgtagcttcaagtaggagacacaagagatttgcgggagtagtcctggcaggtgcggccctaggcgttgccacagctgctcagataacagccggcattgcacttcaccagtccatgctgaactctcaagccatcgacaatctgagagcgagcctggaaactactaatcaggcaattgaggcaatcagacaagcagggcaggagatgatattggctgttcagggtgtccaagactacatcaataatgagctgataccgtctatgaaccaactatcttgtgatttaatcggccagaagctcgggctcaaattgctcagatactatacagaaatcctgtcattatttggccccagcttacgggaccccatatctgcggagatatctatccaggctttgagctatgcgcttggaggagacatcaataaggtgttagaaaagctcggatacagtggaggtgatttactgggcatcttagagagcagaggaataaaggcccggataactcacgtcgacacagagtcctacttcattgtcctcagtatagcctatccgacgctgtccgagattaagggggtgattgtccaccggctagagggggtctcgtacaacataggctctcaagagtggtataccactgtgcccaagtatgttgcaacccaagggtaccttatctcgaattttgatgagtcatcgtgtactttcatgccagaggggactgtgtgcagccaaaatgccttgtacccgatgagtcctctgctccaagaatgcctccgggggtccaccaagtcctgtgctcgtacactcgtatccgggtcttttgggaaccggttcattttatcacaagggaacctaatagccaattgtgcatcaatcctttgcaagtgttacacaacaggaacgatcattaatcaagaccctgacaagatcctaacatacattgctgccgatcactgcccggtagtcgaggtgaacggcgtgaccatccaagtcgggagcaggaggtatccagacgctgtgtacttgcacagaattgacctcggtcctcccatatcattggagaggttggacgtagggacaaatctggggaatgcaattgctaagttggaggatgccaaggaattgttggagtcatcggaccagatattgaggagtatgaaaggtttatcgagcactagcatagtctacatcctgattgcagtgtgtcttggagggttgatagggatccccgctttaatatgttgctgcagggggcgttgacccctctccctcccccccccctaacgttactggccgaagccgcttggaataaggccggtgtgcgtttgtctatatgttattttccaccatattgccgtcttttggcaatgtgagggcccggaaacctggccctgtcttcttgacgagcattcctaggggtctttcccctctcgccaaaggaatgcaaggtctgttgaatgtcgtgaaggaagcagttcctctggaagcttcttgaagacaaacaacgtctgtagcgaccctttgcaggcagcggaaccccccacctggcgacaggtgcctctgcggccaaaagccacgtgtataagatacacctgcaaaggcggcacaaccccagtgccacgttgtgagttggatagttgtggaaagagtcaaatggctctcctcaagcgtattcaacaaggggctgaaggatgcccagaaggtaccccattgtatgggatctgatctggggcctcggtacacatgctttacatgtgtttagtcgaggttaaaaaaacgtctaggccccccgaaccacggggacgtggttttcctttgaaaaacacgatgataatatggccacaaccatgggaagtaggatagtcattaacagagaacatcttatgattgatagaccttatgttttgctggctgttctgtttgtcatgtttctgagcttgatcgggttgctagccattgcaggcattagacttcatcgggcagccatctacaccgcagagatccataaaagcctcagcaccaatctagatgtaactaactcaatcgagcatcaggtcaaggacgtgctgacaccactcttcaaaatcatcggtgatgaagtgggcctgaggacacctcagagattcactgacctagtgaaattcatctctgacaagattaaattccttaatccggatagggagtacgacttcagagatctcacttggtgtatcaacccgccagagagaatcaaattggattatgatcaatactgtgcagatgtggctgctgaagagctcatgaatgcattggtgaactcaactctactggagaccagaacaaccaatcagttcctagctgtctcaaagggaaactgctcagggcccactacaatcagaggtcaattctcaaacatgtcgctgtccctgttagacttgtatttaggtcgaggttacaatgtgtcatctatagtcactatgacatcccagggaatgtatgggggaacttacctagtggaaaagcctaatctgagcagcaaaaggtcagagttgtcacaactgagcatgtaccgagtgtttgaagtaggtgttatcagaaatccgggtttgggggctccggtgttccatatgacaaactatcttgagcaaccagtcagtaatgatctcagcaactgtatggtggctttgggggagctcaaactcgcagccctttgtcacggggaagattctatcacaattccctatcagggatcagggaaaggtgtcagcttccagctcgtcaagctaggtgtctggaaatccccaaccgacatgcaatcctgggtccccttatcaacggatgatccagtgatagacaggctttacctctcatctcacagaggtgttatcgctgacaaycaagcaaaatgggctgtcccgacaacacgaacagatgacaagttgcgaatggagacatgcttccaacaggcgtgtaagggtaaaatccaagcactctgcgagaatcccgagtgggcaccattgaaggataacaggattccttcatacggggtcttgtctgttgatctgagtctgacagttgagcttaaaatcaaaattgcttcgggattcgggccattgatcacacacggttcagggatggacctatacaaatccaaccacaacaatgtgtattggctgactatcccrccaatgaagaacctagccttaggtgtaatcaacacattggagtggataccgagattcaaggttagtccctacctcttcamtgtcccaattaaggaagcaggcgaagactgccatgccccaacatacctacctgcggaggtggatggtgatgtcaaactcagttccaatctggtgattctacctggtcaagatctccaatatgttttggcaacctacgatacttccagggttgaacatgctgtggtttattacgtttacagcccaagccgctcattttcttacttttatccttttaggttgcctataaagggggtccccatcgaattacaagtggaatgcttcacatgggaccaaaaactctggtgccgtcacttctgtgtgcttgcggactcagaatctggtggacatatcactcactctgggatggtgggcatgggagtcagctgcacagtcacccgggaagatggaaccaatcgcagatagggctgctagtgaacyaatcwcatgatgtcacccagacatcaggcatacccactagtgtgaaatagacatcagaattaagaaaaatgggctccccgggcgcgtactccacctcacccatcatccacgctcggcaataaaaagacagaataaaacgcacgggtgttgggtcgtttgttcgccgggcgcgtactccacctcacccatcatccacgctgttttatggatagcactgagaacgtcatcaagcccttcatgcgcttcaaggtgcacatggagggctccgtgaacggccacgagttcgagatcgagggcgagggcgagggcaagccctacgagggcacccagaccgccaagctgcaggtgaccaagggcggccccctgcccttcgcctgggacatcctgtccccccagttccagtacggctccaaggtgtacgtgaagcaccccgccgacatccccgactacaagaagctgtccttccccgagggcttcaagtgggagcgcgtgatgaacttcgaggacggcggcgtggtgaccgtgacccaggactcctccctgcaggacggcaccttcatctaccacgtgaagttcatcggcgtgaacttcccctccgacggccccgtaatgcagaagaagactctgggctgggagccctccaccgagcgcctgtacccccgcgacggcgtgctgaagggcgagatccacaaggcgctgaagctgaagggcggcggccactacctggtggagttcaagtcaatctacatggccaagaagcccgtgaagctgcccggctactactacgtggactccaagctggacatcacctcccacaacgaggactacaccgtggtggagcagtacgagcgcgccgaggcccgccaccacctgttccagtaggacctccatagaagacaccgggaccgatccaataacttcgtatagcatacattatacgaagttatgcctccggactctagcgtttaaacttaagcttggtaccgagctcggatccactagtccagtgtggtggaattctgcagatatccagcacagtggcggccgctcgagtctagagggcccgtttaaacccgctgatcagcctcgactgtgccttctagttgccagccatctgttgtttgcccctcccccgtgccttccttgaccctggaaggtgccactcccactgtcctttcctaataaaatgaggaaattgcatcgcattgtctgagtaggtgtcattctattctggggggtggggtggggcaggacagcaagggggaggattgggaagacaatagcaggcatgctggggatgcggtgggctctatggcttctgaggcggaaagttaaccctagaaagataatcatattgtgacgtacgttaaagataatcatgcgtaaaattgacgcatgtgttttatcggtctgtatatcgaggtttatttattaatttgaatagatattaagttttattatatttacacttacatactaataataaattcaacaaacaatttatttatgtttatttatttattaaaaaaaaacaaaaactcaaaatttcttctataaagtaacaaaaaccagctggggctcgaagttcctatactttctagagaataggaacttctatagtgagtcgaataagggcgacacaaaatttattctaaatgcataataaatactgataacatcttatagtttgtattatattttgtattatcgttgacatgtataattttgatatcaaaaactgattttccctttattattttcgagatttattttcttaattctctttaacaaactagaaatattgtatatacaaaaaatcataaataatagatgaatagtttaattataggtgttcatcaatcgaaaaagcaacgtatcttatttaaagtgcgttgcttttttctcatttataaggttaaataattctcatatatcaagcaaagtgacaggcgcccttaaatattctgacaaatgctctttccctaaactccccccataaaaaaacccgccgaagcgggtttttacgttatttgcggattaacgattactcgttatcagaaccgcccagggggcccgagcttaagactggccgtcgttttacaacacagaaagagtttgtagaaacgcaaaaaggccatccgtcaggggccttctgcttagtttgatgcctggcagttccctactctcgccttccgcttcctcgctcactgactcgctgcgctcggtcgttcggctgcggcgagcggtatcagctcactcaaaggcggtaatacggttatccacagaatcaggggataacgcaggaaagaacatgtgagcaaaaggccagcaaaaggccaggaaccgtaaaaaggccgcgttgctggcgtttttccataggctccgcccccctgacgagcatcacaaaaatcgacgctcaagtcagaggtggcgaaacccgacaggactataaagataccaggcgtttccccctggaagctccctcgtgcgctctcctgttccgaccctgccgcttaccggatacctgtccgcctttctcccttcgggaagcgtggcgctttctcatagctcacgctgtaggtatctcagttcggtgtaggtcgttcgctccaagctgggctgtgtgcacgaaccccccgttcagcccgaccgctgcgccttatccggtaactatcgtcttgagtccaacccggtaagacacgacttatcgccactggcagcagccactggtaacaggattagcagagcgaggtatgtaggcggtgctacagagttcttgaagtggtgggctaactacggctacactagaagaacagtatttggtatctgcgctctgctgaagccagttaccttcggaaaaagagttggtagctcttgatccggcaaacaaaccaccgctggtagcggtggtttttttgtttgcaagcagcagattacgcgcagaaaaaaaggatctcaagaagatcctttgatcttttctacggggtctgacgctcagtggaacgacgcgcgcgtaactcacgttaagggattttggtcatgagcttgcgccgtcccgtcaagtcagcgtaatgctctgcttttagaaaaactcatcgagcatcaaatgaaactgcaatttattcatatcaggattatcaataccatatttttgaaaaagccgtttctgtaatgaaggagaaaactcaccgaggcagttccataggatggcaagatcctggtatcggtctgcgattccgactcgtccaacatcaatacaacctattaatttcccctcgtcaaaaataaggttatcaagtgagaaatcaccatgagtgacgactgaatccggtgagaatggcaaaagtttatgcatttctttccagacttgttcaacaggccagccattacgctcgtcatcaaaatcactcgcatcaaccaaaccgttattcattcgtgattgcgcctgagcgaggcgaaatacgcgatcgctgttaaaaggacaattacaaacaggaatcgagtgcaaccggcgcaggaacactgccagcgcatcaacaatattttcacctgaatcaggatattcttctaatacctggaacgctgtttttccggggatcgcagtggtgagtaaccatgcatcatcaggagtacggataaaatgcttgatggtcggaagtggcataaattccgtcagccagtttagtctgaccatctcatctgtaacatcattggcaacgctacctttgccatgtttcagaaacaactctggcgcatcgggcttcccatacaagcgatagattgtcgcacctgattgcccgacattatcgcgagcccatttatacccatataaatcagcatccatgttggaatttaatcgcggcctcgacgtttcccgttgaatatggctcatattcttcctttttcaatattattgaagcatttatcagggttattgtctcatgagcggatacatatttgaatgtatttagaaaaataaacaaataggggtcagtgttacaaccaattaaccaattctgaacattatcgcgagcccatttatacctgaatatggctcataacaccccttgtttgcctggcggcagtagcgcggtggtcccacctgaccccatgccgaactcagaagtgaaacgccgtagcgccgatggtagtgtggggactccccatgcgagagtagggaactgccaggcatcaaataaaacgaaaggctcagtcgaaagactgggcctttcgcccgggctaattagggggtgtcgcccttattcgactctatagtgaagttcctattctctagaaagtataggaacttctgaagt

SEQ ID NO: 85 - DNA, 6584 bp, Artificial sequence
  synthetic Rapamycin-inducible TET activator
gatatctataacaagaaaatatatatataataagttatcacgtaagtagaacatgaaataacaatataattatcgtatgagttaaatcttaaaagtcacgtaaaagataatcatgcgtcattttgactcacgcggtcgttatagttcaaaatcagtgacacttaccgcattgacaagcacgcctcacgggagctccaagcggcgactgagatgtcctaaatgcacagcgacggattcgcgctatttagaaagagagagcaatatttcaagaatgcatgcgtcaattttacgcagactatctttctagggttaagacggatcgggagatctcccgatcccctatggtgcactctcagtacaatctgctctgatgccgcatagttaagccagtatctgctccctgcttgtgtgttggaggtcgctgagtagtgcgcgagcaaaatttaagctacaacaaggcaaggcttgaccgacaattgcatgaagaatctgcttagggttaggcgttttgcgctgcttcgcgatgtacgggccagatatacgcgttctccatagaagacaccgaataaaatatctttattttcattacatctgtgtgttggttttttgtgtgaatcgatagtactaacatacgctctccatcaaaacaaaacgaaacaaaacaaactagcaaaataggctgtccccagtgcaagtgcaggtgccagaacatttctctggaccgatccaataacttcgtatagcatacattatacgaagttatgcctccggactctagcgttttagttattactagcgctaccggactcagatctcgagctcaagcttcgaattctgcagtcgacggtaccgcggcttacgcgtgctagctaatgatgggcgctcgagtaatgatgggcggtcgactaatgatgggcgctcgagtaatgatgggcgtctagctaatgatgggcgctcgagtaatgatgggcggtcgactaatgatgggcgctcgagtaatgatgggcgtctagctaatgatgggcgctcgagtaatgatgggcggtcgactaatgatgggcgctcgagtaatgatgggcgtctagaacgcgaattaattcaacattttgacacccccataatatttttccagaattaacagtataaattgcatctcttgttcaagagttccctatcactctctttaatcactactcacagtaacctcaactcctgccacaagcttgccctgcagcgggaattccaaacttaagcttggtaccgagctcggatccactagtccagtgtggtggaattctgcagatatccagcacagtggcggccgctcgagtctagagggcccgtttaaacccgctgatcaatgtctagactggacaagagcaaagtcataaactctgctctggaattactcaatggagtcggtatcgaaggcctgacgacaaggaaactcgctcaaaagctgggagttgagcagcctaccctgtactggcacgtgaagaacaagcgggccctgctcgatgccctgccaatcgagatgctggacaggcatcatacccactcctgccccctggaaggcgagtcatggcaagactttctgcggaacaacgccaagtcataccgctgtgctctcctctcacatcgcgacggggctaaagtgcatctcggcacccgcccaacagagaaacagtacgaaaccctggaaaatcagctcgcgttcctgtgtcagcaaggcttctccctggagaacgcactgtacgctctgtccgccgtgggccactttacactgggctgcgtattggaggaacaggagcatcaagtagcaaaagaggaaagagagacacctaccaccgattctatgcccccacttctgaaacaagcaattgagctgttcgaccggcagggagccgaacctgccttccttttcggcctggaactaatcatatgtggcctggagaaacagctaaagtgcgaaagcggcgggccgaccgacgcccttgacgattttgacttagacatgctcccagccgatgcccttgacgactttgaccttgatatgctgcctgctgacgctcttgacgattttgaccttgacatgctccccgggtaagtccctcccccccccctaacgttactggccgaagccgcttggaataaggccggtgtgcgtttgtctatatgttattttccaccatattgccgtcttttggcaatgtgagggcccggaaacctggccctgtcttcttgacgagcattcctaggggtctttcccctctcgccaaaggaatgcaaggtctgttgaatgtcgtgaaggaagcagttcctctggaagcttcttgaagacaaacaacgtctgtagcgaccctttgcaggcagcggaaccccccacctggcgacaggtgcctctgcggccaaaagccacgtgtataagatacacctgcaaaggcggcacaaccccagtgccacgttgtgagttggatagttgtggaaagagtcaaatggctctcctcaagcgtattcaacaaggggctgaaggatgcccagaaggtaccccattgtatgggatctgatctggggcctcggtgcacatgctttacatgtgtttagtcgaggttaaaaaacgtctaggccccccgaaccacggggacgtggttttcctttgaaaaacacgatgataaatggatagcactgagaacgtcatcaagcccttcatgcgcttcaaggtgcacatggagggctccgtgaacggccacgagttcgagatcgagggcgagggcgagggcaagccctacgagggcacccagaccgccaagctgcaggtgaccaagggcggccccctgcccttcgcctgggacatcctgtccccccagttccagtacggctccaaggtgtacgtgaagcaccccgccgacatccccgactacaagaagctgtccttccccgagggcttcaagtgggagcgcgtgatgaacttcgaggacggcggcgtggtgaccgtgacccaggactcctccctgcaggacggcaccttcatctaccacgtgaagttcatcggcgtgaacttcccctccgacggccccgtaatgcagaagaagactctgggctgggagccctccaccgagcgcctgtacccccgcgacggcgtgctgaagggcgagatccacaaggcgctgaagctgaagggcggcggccactacctggtggagttcaagtcaatctacatggccaagaagcccgtgaagctgcccggctactactacgtggactccaagctggacatcacctcccacaacgaggactacaccgtggtggagcagtacgagcgcgccgaggcccgccaccacctgttccagtagctcgactgtgccttctagttgccagccatctgttgtttgcccctcccccgtgccttccttgaccctggaaggtgccactcccactgtcctttcctaataaaatgaggaaattgcatcgcattgtctgagtaggtgtcattctattctggggggtggggtggggcaggacagcaagggggaggattgggaagacaatagcaggcatgctggggatgcggtgggctctatggcttctgaggcggaaagttaaccctagaaagataatcatattgtgacgtacgttaaagataatcatgcgtaaaattgacgcatgtgttttatcggtctgtatatcgaggtttatttattaatttgaatagatattaagttttattatatttacacttacatactaataataaattcaacaaacaatttatttatgtttatttatttattaaaaaaaaacaaaaactcaaaatttcttctataaagtaacaaaaaccagctggggctcgaagttcctatactttctagagaataggaacttctatagtgagtcgaataagggcgacacaaaatttattctaaatgcataataaatactgataacatcttatagtttgtattatattttgtattatcgttgacatgtataattttgatatcaaaaactgattttccctttattattttcgagatttattttcttaattctctttaacaaactagaaatattgtatatacaaaaaatcataaataatagatgaatagtttaattataggtgttcatcaatcgaaaaagcaacgtatcttatttaaagtgcgttgcttttttctcatttataaggttaaataattctcatatatcaagcaaagtgacaggcgcccttaaatattctgacaaatgctctttccctaaactccccccataaaaaaacccgccgaagcgggtttttacgttatttgcggattaacgattactcgttatcagaaccgcccagggggcccgagcttaagactggccgtcgttttacaacacagaaagagtttgtagaaacgcaaaaaggccatccgtcaggggccttctgcttagtttgatgcctggcagttccctactctcgccttccgcttcctcgctcactgactcgctgcgctcggtcgttcggctgcggcgagcggtatcagctcactcaaaggcggtaatacggttatccacagaatcaggggataacgcaggaaagaacatgtgagcaaaaggccagcaaaaggccaggaaccgtaaaaaggccgcgttgctggcgtttttccataggctccgcccccctgacgagcatcacaaaaatcgacgctcaagtcagaggtggcgaaacccgacaggactataaagataccaggcgtttccccctggaagctccctcgtgcgctctcctgttccgaccctgccgcttaccggatacctgtccgcctttctcccttcgggaagcgtggcgctttctcatagctcacgctgtaggtatctcagttcggtgtaggtcgttcgctccaagctgggctgtgtgcacgaaccccccgttcagcccgaccgctgcgccttatccggtaactatcgtcttgagtccaacccggtaagacacgacttatcgccactggcagcagccactggtaacaggattagcagagcgaggtatgtaggcggtgctacagagttcttgaagtggtgggctaactacggctacactagaagaacagtatttggtatctgcgctctgctgaagccagttaccttcggaaaaagagttggtagctcttgatccggcaaacaaaccaccgctggtagcggtggtttttttgtttgcaagcagcagattacgcgcagaaaaaaaggatctcaagaagatcctttgatcttttctacggggtctgacgctcagtggaacgacgcgcgcgtaactcacgttaagggattttggtcatgagcttgcgccgtcccgtcaagtcagcgtaatgctctgcttttagaaaaactcatcgagcatcaaatgaaactgcaatttattcatatcaggattatcaataccatatttttgaaaaagccgtttctgtaatgaaggagaaaactcaccgaggcagttccataggatggcaagatcctggtatcggtctgcgattccgactcgtccaacatcaatacaacctattaatttcccctcgtcaaaaataaggttatcaagtgagaaatcaccatgagtgacgactgaatccggtgagaatggcaaaagtttatgcatttctttccagacttgttcaacaggccagccattacgctcgtcatcaaaatcactcgcatcaaccaaaccgttattcattcgtgattgcgcctgagcgaggcgaaatacgcgatcgctgttaaaaggacaattacaaacaggaatcgagtgcaaccggcgcaggaacactgccagcgcatcaacaatattttcacctgaatcaggatattcttctaatacctggaacgctgtttttccggggatcgcagtggtgagtaaccatgcatcatcaggagtacggataaaatgcttgatggtcggaagtggcataaattccgtcagccagtttagtctgaccatctcatctgtaacatcattggcaacgctacctttgccatgtttcagaaacaactctggcgcatcgggcttcccatacaagcgatagattgtcgcacctgattgcccgacattatcgcgagcccatttatacccatataaatcagcatccatgttggaatttaatcgcggcctcgacgtttcccgttgaatatggctcatattcttcctttttcaatattattgaagcatttatcagggttattgtctcatgagcggatacatatttgaatgtatttagaaaaataaacaaataggggtcagtgttacaaccaattaaccaattctgaacattatcgcgagcccatttatacctgaatatggctcataacaccccttgtttgcctggcggcagtagcgcggtggtcccacctgaccccatgccgaactcagaagtgaaacgccgtagcgccgatggtagtgtggggactccccatgcgagagtagggaactgccaggcatcaaataaaacgaaaggctcagtcgaaagactgggcctttcgcccgggctaattagggggtgtcgcccttattcgactctatagtgaagttcctattctctagaaagtataggaacttctgaagt

SEQ ID NO: 86 - DNA, 11528 bp, Artificial sequence
  synthetic Rapamycin inducer inducible REV srcVpx
gatatctataacaagaaaatatatatataataagttatcacgtaagtagaacatgaaataacaatataattatcgtatgagttaaatcttaaaagtcacgtaaaagataatcatgcgtcattttgactcacgcggtcgttatagttcaaaatcagtgacacttaccgcattgacaagcacgcctcacgggagctccaagcggcgactgagatgtcctaaatgcacagcgacggattcgcgctatttagaaagagagagcaatatttcaagaatgcatgcgtcaattttacgcagactatctttctagggttaagacggatcgggagatctcccgatcccctatggtgcactctcagtacaatctgctctgatgccgcatagttaagccagtatctgctccctgcttgtgtgttggaggtcgctgagtagtgcgcgagcaaaatttaagctacaacaaggcaaggcttgaccgacaattgcatgaagaatctgcttagggttaggcgttttgcgctgcttcgcgatgtacgggccagatatacgcgttgacattgattattgactagttattaatagtaatcaattacggggtcattagttcatagcccatatatggagttccgcgttacataacttacggtaaatggcccgcctggctgaccgcccaacgacccccgcccattgacgtcaataatgacgtatgttcccatagtaacgccaatagggactttccattgacgtcaatgggtggagtatttacggtaaactgcccacttggcagtacatcaagtgtatcatatgccaagtacgccccctattgacgtcaatgacggtaaatggcccgcctggcattatgcccagtacatgaccttatgggactttcctacttggcagtacatctacgtattagtcatcgctattaccatggtgatgcggttttggcagtacatcaatgggcgtggatagcggtttgactcacggggatttccaagtctccaccccattgacgtcaatgggagtttgttttggaaccaaaatcaacgggactttccaaaatgtcgtaacaactccgccccattgacgcaaatgggcggtaggcgtgtacggtgggaggtctatataagcagagctcggcattgattattgactagttattaatagtaatcaattacggggtcattagttcatagcccatatatggagttccgcgttacataacttacggtaaatggcccgcctggctgaccgcccaacgacccccgcccattgacgtcaataatgacgtatgttcccatagtaacgccaatagggactttccattgacgtcaatgggtggagtatttacggtaaactgcccacttggcagtacatcaagtgtatcatatgccaagtccgccccctattgacgtcaatgacggtaaatggcccgcctggcattatgcccagtacatgaccttacgggactttcctacttggcagtacatctacgtattagtcatcgctattaccatggtgatgcggttttggcagtacaccaatgggcgtggatagcggtttgactcacggggatttccaagtctccaccccattgacgtcaatgggagtttgttttggcaccaaaatcaacgggactttccaaaatgtcgtaacaactgcgatcgcccgccccgttgacgcaaatgggcggtaggcgtgtacggtgggaggtctatataagcagagctcgtttagtgaaccgtcagatcactagaagctttattgcggtagtttatcacagttaaattgctaacgcagtcagtgcttctgacacaacagtctcgaacttaagctgcagtgactctcttaaggtagccttgcagaagttggtcgtgaggcactgggcaggtaagtatcaaggttacaagacaggtttaaggagaccaatagaaactgggcttgtcgagacagagaagactcttgcgtttctgataggcacctattggtcttactgacatccactttgcctttctctccacaggtgtccactcccagttcaattacagctcttaaggctagagtacttaatacgactcactataggctagcctcgagaattcatggcttctagaatcctctggcatgagatgtggcatgaaggcctggaagaggcatctcgtttgtactttggggaaaggaacgtgaaaggcatgtttgaggtgctggagcccttgcatgctatgatggaacggggcccccagactctgaaggaaacatcctttaatcaggcctatggtcgagatttaatggaggcccaagagtggtgcaggaagtacatgaaatcagggaatgtcaaggacctcctccaagcctgggacctctattatcatgtgttccgacgaatctcaaagactagagatgagtttcccaccatggtgtttccttctgggcagatcagccaggcctcggccttggccccggcccctccccaagtcctgccccaggctccagcccctgcccctgctccagccatggtatcagctctggcccaggccccagcccctgtcccagtcctagccccaggccctcctcaggctgtggccccacctgcccccaagcccacccaggctggggaaggaacgctgtcagaggccctgctgcagctgcagtttgatgatgaagacctgggggccttgcttggcaacagcacagacccagctgtgttcacagacctggcatccgtcgacaactccgagtttcagcagctgctgaaccagggcatacctgtggccccccacacaactgagcccatgctgatggagtaccctgaggctataactcgcctagtgacaggggcccagaggccccccgacccagctcctgctccactgggggccccggggctccccaatggcctcctttcaggagatgaagacttctcctccattgcggacatggacttctcagccctgctgagtcagatcagctccactagttattaagaattcacgcgtcgagcatgcatctagggcggccaattccgcccctctcccccccccccctctccctcccccccccctaacgttactggccgaagccgcttggaataaggccggtgtgcgtttgtctatatgttattttccaccatattgccgtcttttggcaatgtgagggcccggaaacctggccctgtcttcttgacgagcattcctaggggtctttcccctctcgccaaaggaatgcaaggtctgttgaatgtcgtgaaggaagcagttcctctggaagcttcttgaagacaaacaacgtctgtagcgaccctttgcaggcagcggaaccccccacctggcgacaggtgcctctgcggccaaaagccacgtgtataagatacacctgcaaaggcggcacaaccccagtgccacgttgtgagttggatagttgtggaaagagtcaaatggctctcctcaagcgtattcaacaaggggctgaaggatgcccagaaggtaccccattgtatgggatctgatctggggcctcggtgcacatgctttacatgtgtttagtcgaggttaaaaaaacgtctaggccccccgaaccacggggacgtggttttcctttgaaaaacacgatgataagcttgccacaacccgggatcctctagagtcgacatggactatcctgctgccaagagggtcaagttggactctagagaacgcccatatgcttgccctgtcgagtcctgcgatcgccgcttttctcgctcggatgagcttacccgccatatccgcatccacacaggccagaagcccttccagtgtcgaatctgcatgcgtaacttcagtcgtagtgaccaccttaccacccacatccgcacccacacaggcggcggccgcaggaggaagaaacgcaccagcatagagaccaacatccgtgtggccttagagaagagtttcttggagaatcaaaagcctacctcggaagagatcactatgattgctgatcagctcaatatggaaaaagaggtgattcgtgtttggttctgtaaccgccgccagaaagaaaaaagaatcaacactagaggagtgcaggtggaaaccatctccccgggagacgggcgcaccttccccaagcgcggccagacctgcgtggtgcactacaccgggatgcttgaagatggaaagaaatttgattcctcccgggacagaaacaagccctttaagtttatgctaggcaagcaggaggtgatccgaggctgggaagaaggggttgcccagatgagtgtgggtcagagagccaaactgactatatctccagattatgcctatggtgccactgggcacccaggcatcatcccaccacatgccactctcgtcttcgatgtggagcttctaaaactggaagtcgagggcgtgcaggtggaaaccatctccccaggagacgggcgcaccttccccaagcgcggccagacctgcgtggtgcactacaccgggatgcttgaagatggaaagaaatttgattcctcccgggacagaaacaagccctttaagtttatgctaggcaagcaggaggtgatccgaggctgggaagaaggggttgcccagatgagtgtgggtcagagagccaaactgactatatctccagattatgcctatggtgccactgggcacccaggcatcatcccaccacatgccactctcgtcttcgatgtggagcttctaaaactggaaactagaggagtgcaggtggaaaccatctccccaggagacgggcgcaccttccccaagcgcggccagacctgcgtggtgcactacaccgggatgcttgaagatggaaagaaatttgattcctcccgggacagaaacaagccctttaagtttatgctaggcaagcaggaggtgatccgaggctgggaagaaggggttgcccagatgagtgtgggtcagagagccaaactgactatatctccagattatgcctatggtgccactgggcacccaggcatcatcccaccacatgccactctcgtcttcgatgtggagcttctaaaactggaaactagttattaagtcgacccgggcggccgcttccctttagtgagggttaatgcttcgagcagacatgataagatacattgatgagtttggacaaaccacaactagaatgcagtgaaaaaaatgctttatttgtgaaatttgtgatgctattgctttatttgtaaccattataagctgcaataaacaagttaacctccatagaagacaccgggaccgatccaataacttcgtatagcatacattatacgaagttatggctgctagtgaacyaatcwcatgatgtcacccagacatcaggcatacccactagtgtgaaatagacatcagaattaagaaaaatgggctccccgggcgcgtactccacctcacccatcatccacgctcggcaataaaaagacagaataaaacgcacgggtgttgggtcgtttgttcgttttatggatagcactgagaacgtcatcaagcccttcatgcgcttcaaggtgcacatggagggctccgtgaacggccacgagttcgagatcgagggcgagggcgagggcaagccctacgagggcacccagaccgccaagctgcaggtgaccaagggcggccccctgcccttcgcctgggacatcctgtccccccagttccagtacggctccaaggtgtacgtgaagcaccccgccgacatccccgactacaagaagctgtccttccccgagggcttcaagtgggagcgcgtgatgaacttcgaggacggcggcgtggtgaccgtgacccaggactcctccctgcaggacggcaccttcatctaccacgtgaagttcatcggcgtgaacttcccctccgacggccccgtaatgcagaagaagactctgggctgggagccctccaccgagcgcctgtacccccgcgacggcgtgctgaagggcgagatccacaaggcgctgaagctgaagggcggcggccactacctggtggagttcaagtcaatctacatggccaagaagcccgtgaagctgcccggctactactacgtggactccaagctggacatcacctcccacaacgaggactacaccgtggtggagcagtacgagcgcgccgaggcccgccaccacctgttccagtaggacctccatagaagacaccgaataaaatatctttattttcattacatctgtgtgttggttttttgtgtgaatcgatagtactaacatacgctctccatcaaaacaaaacgaaacaaaacaaactagcaaaataggctgtccccagtgcaagtgcaggtgccagaacatttctctggaccgatccaataacttcgtatagcatacattatacgaagttatgcctccggactctagcgttttagttattactagcgctaccggactcagatctcgagctcaagcttcgaattctgcagtcgacggtaccgcggcttacgcgtgctagctaatgatgggcgctcgagtaatgatgggcggtcgactaatgatgggcgctcgagtaatgatgggcgtctagctaatgatgggcgctcgagtaatgatgggcggtcgactaatgatgggcgctcgagtaatgatgggcgtctagctaatgatgggcgctcgagtaatgatgggcggtcgactaatgatgggcgctcgagtaatgatgggcgtctagaacgcgaattaattcaacattttgacacccccataatatttttccagaattaacagtataaattgcatctcttgttcaagagttccctatcactctctttaatcactactcacagtaacctcaactcctgccacaagcttgccctgcagcgggaattccaaacttaagcttggtaccgagctcggatccactagtccagtgtggtggaattctgcagatatccagcacagtggcggccgctcgagtctagagggcccgtttaaacccgctgatcagatggcaggaagaagcggagacagcgacgaagacctcctcaaggcagtcagactcatcaagtttctctatcaaagcaacccacctcccaaccccgaggggacccgacaggcccgaaggaatagaagaagaaggtggagagagagacagagacagatccattcgattagtgaacggatccttagcacttatttgggacgatctgcggacgctgtgcctcttcagctaccaccgcttgagagacttactcttgattgtgacgaggattgtggaacttctgggacgcagggggtgggaagccctcaaatattggtggaatctcctacaatattggagtcaggagctaaagaatagtccctcccccccccctaacgttactggccgaagccgcttggaataaggccggtgtgcgtttgtctatatgttattttccaccatattgccgtcttttggcaatgtgagggcccggaaacctggccctgtcttcttgacgagcattcctaggggtctttcccctctcgccaaaggaatgcaaggtctgttgaatgtcgtgaaggaagcagttcctctggaagcttcttgaagacaaacaacgtctgtagcgaccctttgcaggcagcggaaccccccacctggcgacaggtgcctctgcggccaaaagccacgtgtataagatacacctgcaaaggcggcacaaccccagtgccacgttgtgagttggatagttgtggaaagagtcaaatggctctcctcaagcgtattcaacaaggggctgaaggatgcccagaaggtaccccattgtatgggatctgatctggggcctcggtgcacatgctttacatgtgtttagtcgaggttaaaaaacgtctaggccccccgaaccacggggacgtggttttcctttgaaaaacacgatgataatggggaggaggaagaggaagccgaaggatccgaaggcgagggtgttggcggaggcggattacaaggacgacgatgacaagatgtcagatcccagggagagaatcccacctggaaacagtggagaagagacaataggagaggccttcgaatggctaaacagaacagtagaggagataaacagagaggcagtaaaccacctaccaagggagctgattttccaggtttggcaaaggtcttgggaatactggcatgatgaacaagggatgtcacaaagctatgtaaaatacagatacttgtgtttaatgcaaaaggctttatttatgcattgcaagaaaggctgtagatgtctaggggaaggacacggggcaggaggatggagaccaggacctcctcctcctccccctccaggactagcataacctcgactgtgccttctagttgccagccatctgttgtttgcccctcccccgtgccttccttgaccctggaaggtgccactcccactgtcctttcctaataaaatgaggaaattgcatcgcattgtctgagtaggtgtcattctattctggggggtggggtggggcaggacagcaagggggaggattgggaagacaatagcaggcatgctggggatgcggtgggctctatggcttctgaggcggaaagttaaccctagaaagataatcatattgtgacgtacgttaaagataatcatgcgtaaaattgacgcatgtgttttatcggtctgtatatcgaggtttatttattaatttgaatagatattaagttttattatatttacacttacatactaataataaattcaacaaacaatttatttatgtttatttatttattaaaaaaaaacaaaaactcaaaatttcttctataaagtaacaaaaaccagctggggctcgaagttcctatactttctagagaataggaacttctatagtgagtcgaataagggcgacacaaaatttattctaaatgcataataaatactgataacatcttatagtttgtattatattttgtattatcgttgacatgtataattttgatatcaaaaactgattttccctttattattttcgagatttattttcttaattctctttaacaaactagaaatattgtatatacaaaaaatcataaataatagatgaatagtttaattataggtgttcatcaatcgaaaaagcaacgtatcttatttaaagtgcgttgcttttttctcatttataaggttaaataattctcatatatcaagcaaagtgacaggcgcccttaaatattctgacaaatgctctttccctaaactccccccataaaaaaacccgccgaagcgggtttttacgttatttgcggattaacgattactcgttatcagaaccgcccagggggcccgagcttaagactggccgtcgttttacaacacagaaagagtttgtagaaacgcaaaaaggccatccgtcaggggccttctgcttagtttgatgcctggcagttccctactctcgccttccgcttcctcgctcactgactcgctgcgctcggtcgttcggctgcggcgagcggtatcagctcactcaaaggcggtaatacggttatccacagaatcaggggataacgcaggaaagaacatgtgagcaaaaggccagcaaaaggccaggaaccgtaaaaaggccgcgttgctggcgtttttccataggctccgcccccctgacgagcatcacaaaaatcgacgctcaagtcagaggtggcgaaacccgacaggactataaagataccaggcgtttccccctggaagctccctcgtgcgctctcctgttccgaccctgccgcttaccggatacctgtccgcctttctcccttcgggaagcgtggcgctttctcatagctcacgctgtaggtatctcagttcggtgtaggtcgttcgctccaagctgggctgtgtgcacgaaccccccgttcagcccgaccgctgcgccttatccggtaactatcgtcttgagtccaacccggtaagacacgacttatcgccactggcagcagccactggtaacaggattagcagagcgaggtatgtaggcggtgctacagagttcttgaagtggtgggctaactacggctacactagaagaacagtatttggtatctgcgctctgctgaagccagttaccttcggaaaaagagttggtagctcttgatccggcaaacaaaccaccgctggtagcggtggtttttttgtttgcaagcagcagattacgcgcagaaaaaaaggatctcaagaagatcctttgatcttttctacggggtctgacgctcagtggaacgacgcgcgcgtaactcacgttaagggattttggtcatgagcttgcgccgtcccgtcaagtcagcgtaatgctctgcttttagaaaaactcatcgagcatcaaatgaaactgcaatttattcatatcaggattatcaataccatatttttgaaaaagccgtttctgtaatgaaggagaaaactcaccgaggcagttccataggatggcaagatcctggtatcggtctgcgattccgactcgtccaacatcaatacaacctattaatttcccctcgtcaaaaataaggttatcaagtgagaaatcaccatgagtgacgactgaatccggtgagaatggcaaaagtttatgcatttctttccagacttgttcaacaggccagccattacgctcgtcatcaaaatcactcgcatcaaccaaaccgttattcattcgtgattgcgcctgagcgaggcgaaatacgcgatcgctgttaaaaggacaattacaaacaggaatcgagtgcaaccggcgcaggaacactgccagcgcatcaacaatattttcacctgaatcaggatattcttctaatacctggaacgctgtttttccggggatcgcagtggtgagtaaccatgcatcatcaggagtacggataaaatgcttgatggtcggaagtggcataaattccgtcagccagtttagtctgaccatctcatctgtaacatcattggcaacgctacctttgccatgtttcagaaacaactctggcgcatcgggcttcccatacaagcgatagattgtcgcacctgattgcccgacattatcgcgagcccatttatacccatataaatcagcatccatgttggaatttaatcgcggcctcgacgtttcccgttgaatatggctcatattcttcctttttcaatattattgaagcatttatcagggttattgtctcatgagcggatacatatttgaatgtatttagaaaaataaacaaataggggtcagtgttacaaccaattaaccaattctgaacattatcgcgagcccatttatacctgaatatggctcataacaccccttgtttgcctggcggcagtagcgcggtggtcccacctgaccccatgccgaactcagaagtgaaacgccgtagcgccgatggtagtgtggggactccccatgcgagagtagggaactgccaggcatcaaataaaacgaaaggctcagtcgaaagactgggcctttcgcccgggctaattagggggtgtcgcccttattcgactctatagtgaagttcctattctctagaaagtataggaacttctgaagt

SEQ ID NO: 87 - RNA, 76 nt, Artificial sequence
  synthetic Evolved aptamer
gggcggcacuuauacagcgaagcauaauggcuacugacgcccucaaacccuauuugcagacuauaagugucgcgcg

SEQ ID NO: 88 - RNA, 73 nt, Artificial sequence
  synthetic Evolved aptamer
gggcggcacuuauacaggguagcauaauggcuuaggacgccuucaaaccuaucaagacuauaagugucgcgcg

SEQ ID NO: 89 - RNA, 75 nt, Artificial sequence
  synthetic Evolved aptamer
gggcggcacuuauacaggguagcauaaugggcuacuugacgccuucaccuauuuguagacuauaagugucgcgcg

SEQ ID NO: 90 - RNA, 76 nt, Artificial sequence
  synthetic Evolved aptamer
gggcggcacuuauacagcguagcauaaugggcugcagacgccgucaaaccuauuugcagacuauaagugucgcgcg

SEQ ID NO: 91 - RNA, 74 nt, Artificial sequence
  synthetic Evolved aptamer
gggcggcacuuauacaccguagcauaaugggcuacugccgccgucgaccuuuuggagacuauaagugucgcgcg

SEQ ID NO: 92 - RNA, 75 nt, Artificial sequence
  synthetic Evolved aptamer
gggcggcacuuauacaggucagcauaaugugcuagugcgccuucaaaccuauuuagagacuauaagugucgcgcg

SEQ ID NO: 93 - RNA, 76 nt, Artificial sequence
  synthetic Evolved aptamer
gggcggcacuuauacagcuuagcguaauggcuacugacgccguccaaaccuauuuacagacuauaagugucgcgcg

SEQ ID NO: 94 - RNA, 76 nt, Artificial sequence
  synthetic Evolved aptamer
gggcggcacuuauacaggggagcauaaugggcuacugacgccuuuaaaccuauuugaggacuauaagugucgcgcg

SEQ ID NO: 95 - RNA, 74 nt, Artificial sequence
  synthetic Evolved aptamer
gggcggcacuuauacauggaagcauaaugggcugccgacggcccuuaaccuuuggagacuauaagugucgcgcg

SEQ ID NO: 96 - RNA, 79 nt, Artificial sequence
  synthetic Evolved aptamer
gggcggcacuuauacagauuagcauaaugggcuacugaccccgccggcaaaccuauuugaagacuauaagugucgcgcg

SEQ ID NO: 97 - RNA, 75 nt, Artificial sequence
  synthetic Evolved aptamer
gggcggcacuuauacaguguagcauaaugggcuacugucgcaucaaaccuauuuggagacuauaagugucgcgcg

SEQ ID NO: 98 - RNA, 76 nt, Artificial sequence
  synthetic Evolved aptamer
gggcggcacuuauacagugaagcauaaugggcuacugacacccuuaaaccuauuugcagacuauaagugucgcgcg

SEQ ID NO: 99 - RNA, 76 nt, Artificial sequence
  synthetic Evolved aptamer
gggcggcacuuauacagaguagcauaaugggcuacagacgccgucaaaccuauuuaccgacuauaagugucgcgcg

SEQ ID NO: 100 - RNA, 75 nt, Artificial sequence
  synthetic Evolved aptamer
gggcggcacuuauacagggugcauaaugggcuagugacgccuucaaaccuauuuguagacuauaagugucgcgcg

SEQ ID NO: 101 - protein, 461 aa, Homo sapiens
MTILGTTFGMVFSLLQVVSGESGYAQNGDLEDAELDDYSFSCYSQLEVNGSQHSLTCAFEDPDVNTTNLEFEICGALVEVKCLNFRKLQEIYFIETKKFLLIGKSNICVKVGEKSLTCKKIDLTTIVKPEAPFDLSVIYREGANDFVVTFNTSHLQKKYVKVLMHDVAYRQEKDENKWTHVNLSSTKLTLLQRKLQPAAMYEIKVRSIPDHYFKGFWSEWSPSYYFRTPEINNSSGEMDPILLTISKCHLSFFSVALLVILACVLWKKRIKPIVWPSLPDHKKTLEHLCKKPRKNLNVSFNPESFLDCQIHRVDDIQARDEVEGFLQDTFPQQLEESEKQRLGGDVQSPNCPSEDVVVTPESFGRDSSLTCLAGNVSACDAPILSSSRSLDCRESGKNGPHVYQDLLLSLGTTNSTLPPPFSLQSGILTLNPVAQGQPILTSLGSNQEEAYVTMSSFYQNQ

SEQ ID NO: 102 - protein, 463 aa, Homo sapiens
MTILGTTFGMVFSLLQVVSGESGYAQNGDLEDAELDDYSFSCYSQLEVNGSQHSLTCAFEDPDVNTTNLEFEICGALVEVKCLNFRKLQEIYFIETKKFLLIGKSNICVKVGEKSLTCKKIDLTTIVKPEAPFDLSVIYREGANDFVVTFNTSHLQKKYVKVLMHDVAYRQEKDENKWTHVNLSSTKLTLLQRKLQPAAMYEIKVRSIPDHYFKGFWSEWSPSYYFRTPEINNSSGEMDPIFSCGPLTISILSFFSVALLVILACVLWKKRIKPIVWPSLPDHKKTLEHLCKKPRKNLNVSFNPESFLDCQIHRVDDIQARDEVEGFLQDTFPQQLEESEKQRLGGDVQSPNCPSEDVVVTPESFGRDSSLTCLAGNVSACDAPILSSSRSLDCRESGKNGPHVYQDLLLSLGTTNSTLPPPFSLQSGILTLNPVAQGQPILTSLGSNQEEAYVTMSSFYQNQ

SEQ ID NO: 103 - protein, 462 aa, Homo sapiens
MTILGTTFGMVFSLLQVVSGESGYAQNGDLEDAELDDYSFSCYSQLEVNGSQHSLTCAFEDPDVNTTNLEFEICGALVEVKCLNFRKLQEIYFIETKKFLLIGKSNICVKVGEKSLTCKKIDLTTIVKPEAPFDLSVIYREGANDFVVTFNTSHLQKKYVKVLMHDVAYRQEKDENKWTHVNLSSTKLTLLQRKLQPAAMYEIKVRSIPDHYFKGFWSEWSPSYYFRTPEINNSSGEMDPILLTCHLISILSFFSVALLVILACVLWKKRIKPIVWPSLPDHKKTLEHLCKKPRKNLNVSFNPESFLDCQIHRVDDIQARDEVEGFLQDTFPQQLEESEKQRLGGDVQSPNCPSEDVVVTPESFGRDSSLTCLAGNVSACDAPILSSSRSLDCRESGKNGPHVYQDLLLSLGTTNSTLPPPFSLQSGILTLNPVAQGQPILTSLGSNQEEAYVTMSSFYQNQ

SEQ ID NO: 104 - protein, 466 aa, Homo sapiens
MTILGTTFGMVFSLLQVVSGESGYAQNGDLEDAELDDYSFSCYSQLEVNGSQHSLTCAFEDPDVNTTNLEFEICGALVEVKCLNFRKLQEIYFIETKKFLLIGKSNICVKVGEKSLTCKKIDLTTIVKPEAPFDLSVIYREGANDFVVTFNTSHLQKKYVKVLMHDVAYRQEKDENKWTHVNLSSTKLTLLQRKLQPAAMYEIKVRSIPDHYFKGFWSEWSPSYYFRTPEINNSSGEMDPILLTPPVCSVTISILSFFSVALLVILACVLWKKRIKPIVWPSLPDHKKTLEHLCKKPRKNLNVSFNPESFLDCQIHRVDDIQARDEVEGFLQDTFPQQLEESEKQRLGGDVQSPNCPSEDVVVTPESFGRDSSLTCLAGNVSACDAPILSSSRSLDCRESGKNGPHVYQDLLLSLGTTNSTLPPPFSLQSGILTLNPVAQGQPILTSLGSNQEEAYVTMSSFYQNQ

SEQ ID NO: 105 - protein, 523 aa, Artificial sequence
  synthetic Fc-delta-30
MSIMGLKVNVSAIFMAVLLTLQTPTGQIHWGNLSKIGVVGIGSASYKVMTRSSHQSLVIKLMPNITLLNNCTRVEIAEYRRLLRTVLEPIRDALNAMTQNIRPVQSVASSRRHKRFAGVVLAGAALGVATAAQITAGIALHQSMLNSQAIDNLRASLETTNQAIEAIRQAGQEMILAVQGVQDYINNELIPSMNQLSCDLIGQKLGLKLLRYYTEILSLFGPSLRDPISAEISIQALSYALGGDINKVLEKLGYSGGDLLGILESRGIKARITHVDTESYFIVLSIAYPTLSEIKGVIVHRLEGVSYNIGSQEWYTTVPKYVATQGYLISNFDESSCTFMPEGTVCSQNALYPMSPLLQECLRGSTKSCARTLVSGSFGNRFILSQGNLIANCASILCKCYTTGTIINQDPDKILTYIAADHCPVVEVNGVTIQVGSRRYPDAVYLHRIDLGPPISLERLDVGTNLGNAIAKLEDAKELLESSDQILRSMKGLSSTSIVYILIAVCLGGLIGIPALICCCRGR

SEQ ID NO: 106 - protein, 599 aa, Artificial sequence
  synthetic Hc-delta-18
MGSRIVINREHLMIDRPYVLLAVLFVMSLSLIGLLAIAGIRLHRAAIYTAEIHKSLSTNLDVTNSIEHQVKDVLTPLFKIIGDEVGLRTPQRFTDLVKFISDKIKFLNPDREYDFRDLTWCINPPERIKLDYDQYCADVAAEELMNALVNSTLLETRTTNQFLAVSKGNCSGPTTIRGQFSNMSLSLLDLYLSRGYNVSSIVTMTSQGMYGGTYLVEKPNLSSKRSELSQLSMYRVFEVGVIRNPGLGAPVFHMTNYLEQPVSNDLSNCMVALGELKLAALCHGEDSITIPYQGSGKGVSFQLVKLGVWKSPTDMQSWVPLSTDDPVIDRLYLSSHRGVIADNQAKWAVPTTRTDDKLRMETCFQQACKGKIQALCENPEWAPLKDNRIPSYGVLSVDLSLTVELKIKIASGFGPLITHGSGMDLYKSNHNNVYWLTIPPMKNLALGVINTLEWIPRFKVSPNLFTVPIKEAGEDCHAPTYLPAEVDGDVKLSSNLVILPGQDLQYVLATYDTSRVEHAVVYYVYSPGRSFSYFYPFRLPIKGVPIELQVECFTWDQKLWCRHFCVLADSESGGHITHSGMVGMGVSCTVTREDGTNRR

SEQ ID NO: 107 - protein, 529 aa, Artificial sequence
  synthetic DAFss-IL7-DAF fusion
MTVARPSVPAALPLLGELPRLLLLVLLCLPADCDIEGKDGKQYESVLMVSIDQLLDSMKEIGSNCLNNEFNFFKRHICDANKEGMFLFRAARKLRQFLKMNSTGDFDLHLLKVSEGTTILLNCTGQVKGRKPAALGEAQPTKSLEENKSLKEQKKLNDLCFLKRLLQEIKTCWNKILMGTKEHCGLPPDVPNAQPALEGRTSFPEDTVITYKCEESFVKIPGEKDSVICLKGSQWSDIEEFCNRSCEVPTRLNSASLKQPYITQNYFPVGTVVEYECRPGYRREPSLSPKLTCLQNLKWSTAVEFCKKKSCPNPGEIRNGQIDVPGGILFGATISFSCNTGYKLFGSTSSFCLISGSSVQWSDPLPECREIYCPAPPQIDNGIIQGERDHYGYRQSVTYACNKGFTMIGEHSIYCTVNNDEGEWSGPPPECRGKSLTSKVPPTVQKPTTVNVPTTEVSPTSQKTTTKTTTPNAQATRSTPVSRTTKHFHETTPNKGSGTTSGTTRLLSGHTCFTLTGLLGTLVTMGLLT

SEQ ID NO: 108 - DNA, 49 bp, Artificial sequence
  synthetic 582-1
acagcttagcgtaatggctactgacgccgtccaaacctatttacagact

SEQ ID NO: 109 - DNA, 49 bp, Artificial sequence
  synthetic 582-2
acagcttaggataatggctactgacgccgtccaaacctatttacagact

SEQ ID NO: 110 - DNA, 49 bp, Artificial sequence
  synthetic 582-3
acagcttagcataatggctactgacgccgtccaaacctattcacagact

SEQ ID NO: 111 - DNA, 49 bp, Artificial sequence
  synthetic 582-4
acagcttagcataatggctactgacgccgtccaaacctattgacagact

SEQ ID NO: 112 - DNA, 49 bp, Artificial sequence
  synthetic 582-5
acagcatagcataatggctactgacgccgtccaaacctatttacagact

SEQ ID NO: 113 - DNA, 49 bp, Artificial sequence
  synthetic 582-6
acagcttagcataatggctactgacgccgtccaaacctatgtacagact

SEQ ID NO: 114 - DNA, 48 bp, Artificial sequence
  synthetic 582-7
acagctagcgtaatggctactgacgccgtccaaacctatttacagact

SEQ ID NO: 115 - DNA, 49 bp, Artificial sequence
  synthetic 582-8
acagcttagcattatggctactgacgccgtccaaacctatttacagact

SEQ ID NO: 116 - DNA, 48 bp, Artificial sequence
  synthetic 582-9
acagttagcataatggctactgacgccgtccaaacctatttacagact

SEQ ID NO: 117 - DNA, 49 bp, Artificial sequence
  synthetic 582-10
acagcttagcataatggctactgacgcggtccaaacctatttacagact

SEQ ID NO: 118 - DNA, 49 bp, Artificial sequence
  synthetic 582-11
acagcttagcttaatggctactgacgccgtccaaacctatttacagact

SEQ ID NO: 119 - DNA, 49 bp, Artificial sequence
  synthetic 582-12
acagcttagcataatggctactgacgccgtccaaacccatttacagact

SEQ ID NO: 120 - DNA, 49 bp, Artificial sequence
  synthetic 582-13
acagcttagcataatggctactgacgccgtccaaaccaatttacagact

SEQ ID NO: 121 - DNA, 49 bp, Artificial sequence
  synthetic 582-14
acagcttagcataatggatactgacgccgtccaaacctatttacagact

SEQ ID NO: 122 - DNA, 49 bp, Artificial sequence
  synthetic 582-15
acagcttagcattgtggctactgacgccgtccaaacctatttacagact

SEQ ID NO: 123 - DNA, 49 bp, Artificial sequence
  synthetic 582-16
acaggttagcataatggctaccgacgccgtccaaacctatttacagact

SEQ ID NO: 124 - DNA, 49 bp, Artificial sequence
  synthetic 582-17
acagcttagcgtaatggctactgacgccgcccaaacctatttacagact

SEQ ID NO: 125 - DNA, 49 bp, Artificial sequence
  synthetic 582-18
acagcttagcataatggctactgacgccgtccaaaactatttccagact

SEQ ID NO: 126 - DNA, 49 bp, Artificial sequence
  synthetic 582-19
acagcctagcataagggctactgacgccgtccaaacctatttacagact

SEQ ID NO: 127 - DNA, 49 bp, Artificial sequence
  synthetic 582-20
acagcttagcataatggctactgaggccgtccaaacctatttacagact

SEQ ID NO: 128 - DNA, 49 bp, Artificial sequence
  synthetic 582-21
acagcttaccttaatggctactgacgccgtccaaacctatttacagact

SEQ ID NO: 129 - DNA, 49 bp, Artificial sequence
  synthetic 582-22
acagcttagcataatggctaccgacgctgtccaaacctatttacagact

SEQ ID NO: 130 - DNA, 49 bp, Artificial sequence
  synthetic 582-23
acagcttagcgtaatggctactggcgccgtccaaacctatttacagact

SEQ ID NO: 131 - DNA, 49 bp, Artificial sequence
  synthetic 582-24
acagcttagcatactggctactgacgccgcccaaacctatttacagact

SEQ ID NO: 132 - DNA, 49 bp, Artificial sequence
  synthetic 582-25
acagcttagcataatggctactgacgccgtcctaacctatttacagact

SEQ ID NO: 133 - DNA, 49 bp, Artificial sequence
  synthetic 582-26
acaggttagcataatgcctactgacgccgtccaaacctatttacagact

SEQ ID NO: 134 - DNA, 49 bp, Artificial sequence
  synthetic 582-27
acagcttagcataattgctactgacgccgttcaaacctatttacagact

SEQ ID NO: 135 - DNA, 49 bp, Artificial sequence
  synthetic 582-28
acagcttagcataaaggctactgacgccgtccaaacctatttacagact

SEQ ID NO: 136 - DNA, 49 bp, Artificial sequence
  synthetic 582-29
acagcttagcgtaatggctactgacgccgtctaaacctatttccagact

SEQ ID NO: 137 - DNA, 49 bp, Artificial sequence
  synthetic 582-30
acaggttagcataatggctactgacgccgtccaaacctatttagagact

SEQ ID NO: 138 - DNA, 49 bp, Artificial sequence
  synthetic 582-31
acagggtagcgtaatggctactgacgccgtccaaacctatttacagact

SEQ ID NO: 139 - DNA, 49 bp, Artificial sequence
  synthetic 582-32
acagcgtagcataatggctactgacgccgttcaaacctatttacagact

SEQ ID NO: 140 - DNA, 49 bp, Artificial sequence
  synthetic 582-33
acagcttagcataatggctactgacgccgtccaaactcatttacagact

SEQ ID NO: 141 - DNA, 49 bp, Artificial sequence
  synthetic 582-34
acagcgtagcatagtggctactgacgccgtccaaacctatttacagact

SEQ ID NO: 142 - DNA, 49 bp, Artificial sequence
  synthetic 582-35
acagcttagtgtaatggctactgacgctgtccaaacctatttacagact

SEQ ID NO: 143 - DNA, 49 bp, Artificial sequence
  synthetic 582-36
acagcttagcataatggctactgacggcgttcaaacctatttacagact

SEQ ID NO: 144 - DNA, 49 bp, Artificial sequence
  synthetic 582-37
acaggttagcataatggctactgacgccgtccaaacctatttatagact

SEQ ID NO: 145 - DNA, 48 bp, Artificial sequence
  synthetic 582-38
acagcttagcataatggctactgacgccgtccaaacctattgtcgact

SEQ ID NO: 146 - DNA, 48 bp, Artificial sequence
  synthetic 582-39
acagcttagcataatggctactgacgccgtccaaacctatttacgact

SEQ ID NO: 147 - DNA, 48 bp, Artificial sequence
  synthetic 769-1
acaggtcagcataatgtgctagtgcgccttcaaacctatttagagact

SEQ ID NO: 148 - DNA, 48 bp, Artificial sequence
  synthetic 769-2
acaggtcagcataatgtgctagtgcgccctcaaacctatttagagact

SEQ ID NO: 149 - DNA, 48 bp, Artificial sequence
  synthetic 769-3
acaggttagcataatgtgctattgcgccttcaaacctatttagagact

SEQ ID NO: 150 - DNA, 48 bp, Artificial sequence
  synthetic 769-4
acaggtcagcataatgtgctagtgcgcattcaaacctatttagagact

SEQ ID NO: 151 - DNA, 48 bp, Artificial sequence
  synthetic 769-5
acaggttagcataatgtgctagtgcgccttcaaacctattttgagact

SEQ ID NO: 152 - DNA, 48 bp, Artificial sequence
  synthetic 769-6
acaggttatcataatgtgctagtgcgccttcaaacctatttagagact

SEQ ID NO: 153 - DNA, 48 bp, Artificial sequence
  synthetic 769-7
acaggttagcatgatgtgctagtgcgccttcaaacctatttagagact

SEQ ID NO: 154 - DNA, 48 bp, Artificial sequence
  synthetic 769-8
acaggttagcataatgggctagtgcgccttcaaacctatttagagact

SEQ ID NO: 155 - DNA, 48 bp, Artificial sequence
  synthetic 769-9
acaggtcagcaaaatgtgcaagtgcgccttcaaacctatttagagact

SEQ ID NO: 156 - DNA, 48 bp, Artificial sequence
  synthetic 769-10
acaggtcagcataatgtgctagtgcgccttcaaacctatctggagact

SEQ ID NO: 157 - DNA, 48 bp, Artificial sequence
  synthetic 769-11
acagcttagcataatgtgctagtgcgccttcaaacctatttagagact

SEQ ID NO: 158 - DNA, 48 bp, Artificial sequence
  synthetic 769-12
acaggtcagcataatgtgctagtgcgccttcaaacctatttacagact

SEQ ID NO: 159 - DNA, 48 bp, Artificial sequence
  synthetic 769-13
acaggtcagcataatgtgctagtgcgccttcaaacatatttagagact

SEQ ID NO: 160 - DNA, 48 bp, Artificial sequence
  synthetic 769-14
acagggtagcataatgtgctagtgcgccttcaaacctatttagagact

SEQ ID NO: 161 - DNA, 48 bp, Artificial sequence
  synthetic 769-15
acaggttagcataatgtgctagtgcgccctcaaacctatttagagact

SEQ ID NO: 162 - DNA, 48 bp, Artificial sequence
  synthetic 769-16
acaggttagcataatgtgccagtgcgccttcaaacctatttagagact

SEQ ID NO: 163 - DNA, 48 bp, Artificial sequence
  synthetic 769-17
acaggtcagcataatgggctagtgcgccttcaaacctatttagagact

SEQ ID NO: 164 - DNA, 49 bp, Artificial sequence
  synthetic 795-1
acagcgaagcataatggctactgacgccctcaaaccctatttgcagact

SEQ ID NO: 165 - DNA, 49 bp, Artificial sequence
  synthetic 795-2
acagcgaagcataatggctactgacgccctcaaaccctatttacagact

SEQ ID NO: 166 - DNA, 49 bp, Artificial sequence
  synthetic 795-3
acagcgaagcataatggcttctgacgccctcaaaccctatttgcagact

SEQ ID NO: 167 - DNA, 49 bp, Artificial sequence
  synthetic 795-4
acagccaagcatactggctactgacgccctcaaaccctatttgcagact

SEQ ID NO: 168 - DNA, 49 bp, Artificial sequence
  synthetic 795-5
acagcgaagcataatggctactgacgcccgcaaaccctatttgcagact

SEQ ID NO: 169 - DNA, 49 bp, Artificial sequence
  synthetic 795-6
acagcgaagcataatggctactgacggcctcaaaccctatttgcagact

SEQ ID NO: 170 - DNA, 49 bp, Artificial sequence
  synthetic 795-7
acagcgaggcataatggctactgacgccctcaaaccctatttgcagact

SEQ ID NO: 171 - DNA, 49 bp, Artificial sequence
  synthetic 795-8
acagcgaagcataatggctactgacgccttcaaaccctatttgcagact

SEQ ID NO: 172 - DNA, 49 bp, Artificial sequence
  synthetic 795-9
acagcgaagcataatggctacagacgccctcaaaacctatttgcagact

SEQ ID NO: 173 - DNA, 48 bp, Artificial sequence
  synthetic 795-10
acagcgaagcataatggctactgacgccctcaaaccctatttgagact

SEQ ID NO: 174 - DNA, 48 bp, Artificial sequence
  synthetic 795-11
acagcgaagcataatggctactgacgccctcaaaccctattgtcgact

SEQ ID NO: 175 - DNA, 49 bp, Artificial sequence
  synthetic 795-12
acagccaagcataatggctactgacgccctcaaaccctatttgcagact

SEQ ID NO: 176 - DNA, 49 bp, Artificial sequence
  synthetic 795-13
acagcgaagcataatggctactgacgccctcaaaccctatttggcgact

SEQ ID NO: 177 - DNA, 49 bp, Artificial sequence
  synthetic 795-14
acagcgaagcataatgtctactgacgccctcaaaccctatttgcagact

SEQ ID NO: 178 - DNA, 49 bp, Artificial sequence
  synthetic 795-15
acagcgaagcataatggctactgacgccgtcaaaccctatttgtagact

SEQ ID NO: 179 - DNA, 49 bp, Artificial sequence
  synthetic 795-16
acagcgaagcataatggctactgacgccctcaaaccttatttgcagact

SEQ ID NO: 180 - DNA, 48 bp, Artificial sequence
  synthetic 795-17
acaggtagcataatggctactgacgccctcaaaccctatttgcagact

SEQ ID NO: 181 - DNA, 49 bp, Artificial sequence
  synthetic 795-18
acagcgaagcataatggctactgacgccctcaaaccctatttctagact

SEQ ID NO: 182 - DNA, 49 bp, Artificial sequence
  synthetic 795-19
acagcgaagcataatggctactgacgccctcaaaccctatttgtagact

SEQ ID NO: 183 - DNA, 48 bp, Artificial sequence
  synthetic 935-1
acagggtagcataatgggctacttgacgccttcacctatttgtagact

SEQ ID NO: 184 - DNA, 47 bp, Artificial sequence
  synthetic 935-2
acagggtagcataatgggctacttgacgccttcacctatttgagact

SEQ ID NO: 185 - DNA, 48 bp, Artificial sequence
  synthetic 935-3
acagggtagcataatgggctactttacgccttcacctatttgtagact

SEQ ID NO: 186 - DNA, 48 bp, Artificial sequence
  synthetic 935-4
acagggtagcataatgggctacttgacgccttcacctatttctagact

SEQ ID NO: 187 - DNA, 48 bp, Artificial sequence
  synthetic 935-5
acagggtagcataatgggctacttgacgccttcacctatttggagact

SEQ ID NO: 188 - DNA, 48 bp, Artificial sequence
  synthetic 935-6
acagggtagcatagtgggctacttgacgccttcacctatttgtagact

SEQ ID NO: 189 - DNA, 48 bp, Artificial sequence
  synthetic 935-7
acagggtagcatgatgggctacttgacgccttcacctatttgtagact

SEQ ID NO: 190 - DNA, 48 bp, Artificial sequence
  synthetic 935-8
acagggtagcataatgggctacttgacgccttcacctattagtagact

SEQ ID NO: 191 - DNA, 48 bp, Artificial sequence
  synthetic 935-9
acagggtagcataatgggctatttgacgccttcacctatttgtagact

SEQ ID NO: 192 - DNA, 48 bp, Artificial sequence
  synthetic 935-10
acagggtagcataatgggctacttgccgccttcacctatttgtagact

SEQ ID NO: 193 - DNA, 48 bp, Artificial sequence
  synthetic 935-11
acagtgtagcataattggctacttgacgccttcacctatttgtagact

SEQ ID NO: 194 - DNA, 48 bp, Artificial sequence
  synthetic 935-12
acagggtagcataatgggctacttgacgctttcacctttttgtagact

SEQ ID NO: 195 - DNA, 48 bp, Artificial sequence
  synthetic 935-13
acagggtagcataaggggctacttgacgccttcacctatttgtagact

SEQ ID NO: 196 - DNA, 48 bp, Artificial sequence
  synthetic 935-14
acagggtagcataatggactacttgacgcctccacctatttgtagact

SEQ ID NO: 197 - DNA, 48 bp, Artificial sequence
  synthetic 935-15
acagggtagcataatgggctacttgtcgccttcacctatttgtagact

SEQ ID NO: 198 - DNA, 49 bp, Artificial sequence
  synthetic 946-1
acagcgtagcataatgggctgcagacgccgtcaaacctatttgcagact

SEQ ID NO: 199 - DNA, 49 bp, Artificial sequence
  synthetic 946-2
acagcgtagcataatgggctgcagacgcagtcaaacctatttgcagact

SEQ ID NO: 200 - DNA, 48 bp, Artificial sequence
  synthetic 946-3
acatgtagcataatgggctactgacgccgtcaaacctatttgcagact

SEQ ID NO: 201 - DNA, 49 bp, Artificial sequence
  synthetic 946-4
acagcgtagcatagtgggctgcagacgccgtcaaacctatttgcagact

SEQ ID NO: 202 - DNA, 49 bp, Artificial sequence
  synthetic 946-5
acagtgtagcataatgggctgcagacgccttcaaacctatttggagact

SEQ ID NO: 203 - DNA, 49 bp, Artificial sequence
  synthetic 946-6
acagtgtagcataatgggctgctgacgccgtcaaacctatttgaagact

SEQ ID NO: 204 - DNA, 49 bp, Artificial sequence
  synthetic 946-7
acagcgtagcataatgggctacaggcgccgtcaaacctatttgcagact

SEQ ID NO: 205 - DNA, 49 bp, Artificial sequence
  synthetic 946-8
acagcgtagcataatgggctactggcgccgtcaaacctatttgcagact

SEQ ID NO: 206 - DNA, 48 bp, Artificial sequence
  synthetic 946-9
acagcgtagcataatgggctgcagacgccgtcaaacctatttgagact

SEQ ID NO: 207 - DNA, 48 bp, Artificial sequence
  synthetic 946-10
acaggtagcataatgggctgcagacgccgtcaaacctatttgcagact

SEQ ID NO: 208 - DNA, 48 bp, Artificial sequence
  synthetic 946-11
acaggtagcataatgggctgctgacgccgtcaaacctatttacagact

SEQ ID NO: 209 - DNA, 49 bp, Artificial sequence
  synthetic 946-12
acagcgtagcatattgggctgcagacgccgtcaaacctatttgcagact

SEQ ID NO: 210 - DNA, 49 bp, Artificial sequence
  synthetic 946-13
acagcgtagcataatgggctgcagacgccttcaaacctatttggagact

SEQ ID NO: 211 - DNA, 48 bp, Artificial sequence
  synthetic 946-14
acagtgtagcataatgggctgcagacgccgtcaaacctatttgagact

SEQ ID NO: 212 - DNA, 49 bp, Artificial sequence
  synthetic 946-15
acagcgtagcataatgggctgctgacgccgtcaaacctatttggagact

SEQ ID NO: 213 - DNA, 49 bp, Artificial sequence
  synthetic 946-16
acagcgtagcataatgggctgcagacgccgtcaaacctatttacagact

SEQ ID NO: 214 - DNA, 49 bp, Artificial sequence
  synthetic 946-17
acagcgtagcataatgggctgctgacgccgtcaaacctatttgcagact

SEQ ID NO: 215 - DNA, 49 bp, Artificial sequence
  synthetic 946-18
acagggtagcataatgggctgcagacgccgtcaaacctatttggagact

SEQ ID NO: 216 - DNA, 49 bp, Artificial sequence
  synthetic 946-19
acagcgtagcataatgggctacagacgccgtcaaacctatttgcagact

SEQ ID NO: 217 - DNA, 49 bp, Artificial sequence
  synthetic 946-20
acagcgtcgcataatgggctgcagacgccgtcaaatctatttgcagact

SEQ ID NO: 218 - DNA, 49 bp, Artificial sequence
  synthetic 946-21
acagcgtagcataatgggcttcagacgccgtcaaacctatttgcagact

SEQ ID NO: 219 - DNA, 48 bp, Artificial sequence
  synthetic 946-22
acatgtagcataatgggctgcagacgccgtcaaacctatttggagact

SEQ ID NO: 220 - DNA, 47 bp, Artificial sequence
  synthetic 961-1
acaccgtagcataatgggctactgccgccgtcgaccttttggagact

SEQ ID NO: 221 - DNA, 46 bp, Artificial sequence
  synthetic 996-1
acagggtagcataatggcttaggacgccttcaaacctatcaagact

SEQ ID NO: 222 - DNA, 49 bp, Artificial sequence
  synthetic Family 582 Consensus
  misc_feature (5)..(5): n at position 5 can be C, G, or no nucleotide
  misc_feature (6)..(6): n at position 6 can be A, C, G, T, or no nucleotide
  misc_feature (45)..(45): n at position 45 can be A or no nucleotide
acagnntasbdtwvdksmtacygrsgsbgyyywaamyhatkbhbngact

SEQ ID NO: 223 - DNA, 48 bp, Artificial sequence
  synthetic Family 769 Consensus
acagskyakcawratgkgchaktgcgcmytcaaacmtatytdsagact

SEQ ID NO: 224 - DNA, 49 bp, Artificial sequence
  synthetic Family 795 Consensus
  misc_feature (5)..(5): n at position 5 can be C or no nucleotide
  misc_feature (40)..(40): n at position 40 can be T or no nucleotide
  misc_feature (44)..(44): n at position 44 can be C, G, T, or no nucleotide
acagnswrgcatamtgkctwcwgacgscbkcaaamcytanttvnmgact

SEQ ID NO: 225 - DNA, 48 bp, Artificial sequence
  synthetic Family 935 Consensus
  misc_feature (43)..(43): n at position 43 can be G, T, or no nucleotide
acagkgtcgcatrrkkgrctayttkhcgcytycacctwttwsnagact

SEQ ID NO: 226 - DNA, 49 bp, Artificial sequence
  synthetic Family 946 Consensus
  misc_feature (4)..(4): n at position 4 can be G or no nucleotide
  misc_feature (5)..(5): n at position 5 can be C, G, T, or no nucleotide
  misc_feature (44)..(44): n at position 44 can be A, C, G, or no nucleotide
acanngtmgcatadtgggctdcwgrcgcmktcaaayctatttrnagact

SEQ ID NO: 227 - protein, 11 aa, Artificial sequence
  synthetic Membrane-targeting domain of Src-Flag-Vpx
MGSSKSKPKDP

SEQ ID NO: 228 - protein, 8 aa, Artificial sequence
  synthetic Viral protease cleavage domain
KARVLAEA

SEQ ID NO: 229 - protein, 458 aa, Homo sapiens
MTILGTTFGMVFSLLQVVSGESGYAQNGDLEDAELDDYSFSCYSQLEVNGSQHSLTCAFEDPDVNITNLEFEICGALVEVKCLNFRKLQEIYFIETKKFLLIGKSNICVKVGEKSLTCKKIDLTTIVKPEAPFDLSVVYREGANDFVVTFNTSHLQKKYVKVLMHDVAYRQEKDENKWTHVNLSSTKLTLLQRKLQPAAMYEIKVRSIPDHYFKGFWSEWSPSYYFRTPEINNSSGEMDPILLTISILSFFSVALLVILACVLWKKRIKPIVWPSLPDHKKTLEHLCKKPRKNLNVSFNPESFLDCQIHRVDDIQARDEVEGFLQDTFPQQLEESEKQRLGGDVQSPNCPSEDVVITPESFGRDSSLTCLAGNVSACDAPILSSSRSLDCRESGKNGPHVYQDLLLSLGTTNSTLPPPFSLQSGILTLNPVAQGQPILTSLGSNQEEAYVTMSSFYQN

SEQ ID NO: 230 - protein, 723 aa, Artificial sequence
  synthetic GFP - linker - P2A -IL7Ra IncPPCL codon(exceptP2A) and splice optimized
MSGGEELFAGIVPVLIELDGDVHGHKFSVRGEGEGDADYGKLEIKFICTTGKLPVPWPTLVTTLCYGIQCFARYPEHMKMNDFFKSAMPEGYIQERTIQFQDDGKYKTRGEVKFEGDTLVNRIELKGKDFKEDGNILGHKLEYSFNSHNVYIRPDKANNGLEANFKTRHNIEGGGVQLADHYQTNVPLGDGPVLIPINHYLSTQTKISKDRNEARDHMVLLESFSACCHTHGMDELYRGSGATNFSLLKQAGDVEENPGPMTILGTTFGMVFSLLQVVSGESGYAQNGDLEDAELDDYSFSCYSQLEVNGSQHSLTCAFEDPDVNITNLEFEICGALVEVKCLNFRKLQEIYFIETKKFLLIGKSNICVKVGEKSLTCKKIDLTTIVKPEAPFDLSVVYREGANDFVVTFNTSHLQKKYVKVLMHDVAYRQEKDENKWTHVNLSSTKLTLLQRKLQPAAMYEIKVRSIPDHYFKGFWSEWSPSYYFRTPEINNSSGEMDPILLPPCLTISILSFFSVALLVILACVLWKKRIKPIVWPSLPDHKKTLEHLCKKPRKNLNVSFNPESFLDCQIHRVDDIQARDEVEGFLQDTFPQQLEESEKQRLGGDVQSPNCPSEDVVITPESFGRDSSLTCLAGNVSACDAPILSSSRSLDCRESGKNGPHVYQDLLLSLGTTNSTLPPPFSLQSGILTLNPVAQGQPILTSLGSNQEEAYVTMSSFYQNQ

SEQ ID NO: 231 - protein, 733 aa, Artificial sequence
  synthetic GFP - linker - P2A - Myc Tag - IL7Ra IncPPCL codon(exceptP2A) and splice optimized
MSGGEELFAGIVPVLIELDGDVHGHKFSVRGEGEGDADYGKLEIKFICTTGKLPVPWPTLVTTLCYGIQCFARYPEHMKMNDFFKSAMPEGYIQERTIQFQDDGKYKTRGEVKFEGDTLVNRIELKGKDFKEDGNILGHKLEYSFNSHNVYIRPDKANNGLEANFKTRHNIEGGGVQLADHYQTNVPLGDGPVLIPINHYLSTQTKISKDRNEARDHMVLLESFSACCHTHGMDELYRGSGATNFSLLKQAGDVEENPGPMTILGTTFGMVFSLLQVVSGEQKLISEEDLESGYAQNGDLEDAELDDYSFSCYSQLEVNGSQHSLTCAFEDPDVNITNLEFEICGALVEVKCLNFRKLQEIYFIETKKFLLIGKSNICVKVGEKSLTCKKIDLTTIVKPEAPFDLSVVYREGANDFVVTFNTSHLQKKYVKVLMHDVAYRQEKDENKWTHVNLSSTKLTLLQRKLQPAAMYEIKVRSIPDHYFKGFWSEWSPSYYFRTPEINNSSGEMDPILLPPCLTISILSFFSVALLVILACVLWKKRIKPIVWPSLPDHKKTLEHLCKKPRKNLNVSFNPESFLDCQIHRVDDIQARDEVEGFLQDTFPQQLEESEKQRLGGDVQSPNCPSEDVVITPESFGRDSSLTCLAGNVSACDAPILSSSRSLDCRESGKNGPHVYQDLLLSLGTTNSTLPPPFSLQSGILTLNPVAQGQPILTSLGSNQEEAYVTMSSFYQNQ

SEQ ID NO: 232 - protein, 572 aa, Artificial sequence
  synthetic GFP - linker - P2A - IL7RaSP - Myc Tag - IL7RaIncPPCL C-terminal truncation codon(exceptP2A) and splice
MSGGEELFAGIVPVLIELDGDVHGHKFSVRGEGEGDADYGKLEIKFICTTGKLPVPWPTLVTTLCYGIQCFARYPEHMKMNDFFKSAMPEGYIQERTIQFQDDGKYKTRGEVKFEGDTLVNRIELKGKDFKEDGNILGHKLEYSFNSHNVYIRPDKANNGLEANFKTRHNIEGGGVQLADHYQTNVPLGDGPVLIPINHYLSTQTKISKDRNEARDHMVLLESFSACCHTHGMDELYRGSGATNFSLLKQAGDVEENPGPMTILGTTFGMVFSLLQVVSGEQKLISEEDLESGYAQNGDLEDAELDDYSFSCYSQLEVNGSQHSLTCAFEDPDVNITNLEFEICGALVEVKCLNFRKLQEIYFIETKKFLLIGKSNICVKVGEKSLTCKKIDLTTIVKPEAPFDLSVVYREGANDFVVTFNTSHLQKKYVKVLMHDVAYRQEKDENKWTHVNLSSTKLTLLQRKLQPAAMYEIKVRSIPDHYFKGFWSEWSPSYYFRTPEINNSSGEMDPILLPPCLTISILSFFSVALLVILACVLWKKRIKPIVWPSLPDHKKTLEHLCKKPRKVSVFGA

SEQ ID NO: 233 - protein, 562 aa, Artificial sequence
  synthetic GFP - linker - P2A - IL7RaSP - IL7RaIncPPCL C-terminal truncation codon(exceptP2A) and splice optimized
MSGGEELFAGIVPVLIELDGDVHGHKFSVRGEGEGDADYGKLEIKFICTTGKLPVPWPTLVTTLCYGIQCFARYPEHMKMNDFFKSAMPEGYIQERTIQFQDDGKYKTRGEVKFEGDTLVNRIELKGKDFKEDGNILGHKLEYSFNSHNVYIRPDKANNGLEANFKTRHNIEGGGVQLADHYQTNVPLGDGPVLIPINHYLSTQTKISKDRNEARDHMVLLESFSACCHTHGMDELYRGSGATNFSLLKQAGDVEENPGPMTILGTTFGMVFSLLQVVSGESGYAQNGDLEDAELDDYSFSCYSQLEVNGSQHSLTCAFEDPDVNITNLEFEICGALVEVKCLNFRKLQEIYFIETKKFLLIGKSNICVKVGEKSLTCKKIDLTTIVKPEAPFDLSVVYREGANDFVVTFNTSHLQKKYVKVLMHDVAYRQEKDENKWTHVNLSSTKLTLLQRKLQPAAMYEIKVRSIPDHYFKGFWSEWSPSYYFRTPEINNSSGEMDPILLPPCLTISILSFFSVALLVILACVLWKKRIKPIVWPSLPDHKKTLEHLCKKPRKVSVFGA

SEQ ID NO: 234 - protein, 824 aa, Artificial sequence
  synthetic GFP - linker - P2A - eTag -  IL7RaIncPPCL N-terminal deletion codon(exceptP2A) and splice optimized
MSGGEELFAGIVPVLIELDGDVHGHKFSVRGEGEGDADYGKLEIKFICTTGKLPVPWPTLVTTLCYGIQCFARYPEHMKMNDFFKSAMPEGYIQERTIQFQDDGKYKTRGEVKFEGDTLVNRIELKGKDFKEDGNILGHKLEYSFNSHNVYIRPDKANNGLEANFKTRHNIEGGGVQLADHYQTNVPLGDGPVLIPINHYLSTQTKISKDRNEARDHMVLLESFSACCHTHGMDELYRGSGATNFSLLKQAGDVEENPGPMLLLVTSLLLCELPHPAFLLIPRKVCNGIGIGEFKDSLSINATNIKHFKNCTSISGDLHILPVAFRGDSFTHTPPLDPQELDILKTVKEITGFLLIQAWPENRTDLHAFENLEIIRGRTKQHGQFSLAVVSLNITSLGLRSLKEISDGDVIISGNKNLCYANTINWKKLFGTSGQKTKIISNRGENSCKATGQVCHALCSPEGCWGPEPRDCVSCRNVSRGRECVDKCNLLEGEPREFVENSECIQCHPECLPQAMNITCTGRGPDNCIQCAHYIDGPHCVKTCPAGVMGENNTLVWKYADAGHVCHLCHPNCTYGCTGPGLEGCPTNGPEINNSSGEMDPILLPPCLTISILSFFSVALLVILACVLWKKRIKPIVWPSLPDHKKTLEHLCKKPRKNLNVSFNPESFLDCQIHRVDDIQARDEVEGFLQDTFPQQLEESEKQRLGGDVQSPNCPSEDVVITPESFGRDSSLTCLAGNVSACDAPILSSSRSLDCRESGKNGPHVYQDLLLSLGTTNSTLPPPFSLQSGILTLNPVAQGQPILTSLGSNQEEAYVTMSSFYQNQ

SEQ ID NO: 235 - protein, 593 aa, Artificial sequence
  synthetic MV(ed)-HD24
MNREHLMIDRPYVLLAVLFVMSLSLIGLLAIAGIRLHRAAIYTAEIHKSLSTNLDVTNSIEHQVKDVLTPLFKIIGDEVGLRTPQRFTDLVKFISDKIKFLNPDREYDFRDLTWCINPPERIKLDYDQYCADVAAEELMNALVNSTLLETRTTNQFLAVSKGNCSGPTTIRGQFSNMSLSLLDLYLSRGYNVSSIVTMTSQGMYGGTYLVEKPNLSSKRSELSQLSMYRVFEVGVIRNPGLGAPVFHMTNYLEQPVSNDLSNCMVALGELKLAALCHGEDSITIPYQGSGKGVSFQLVKLGVWKSPTDMQSWVPLSTDDPVIDRLYLSSHRGVIADNQAKWAVPTTRTDDKLRMETCFQQACKGKIQALCENPEWAPLKDNRIPSYGVLSVDLSLTVELKIKIASGFGPLITHGSGMDLYKSNHNNVYWLTIPPMKNLALGVINTLEWIPRFKVSPNLFTVPIKEAGEDCHAPTYLPAEVDGDVKLSSNLVILPGQDLQYVLATYDTSRVEHAVVYYVYSPGRSFSYFYPFRLPIKGVPIELQVECFTWDQKLWCRHFCVLADSESGGHITHSGMVGMGVSCTVTREDGTNRR

SEQ ID NO: 236 - DNA, 1275 bp, Mesoplasma florum
aaaaaaaataaaatcaatagcaaatattaagatttttaagaaataaaaaattaatattaatttacaactgaatataaaagaaacttatacagggtagcataatgggctactgaccccgccttcaaacctatttggagactataagtgaaaaaccactctttaattattaaagtttctttttatgtccaaaagacaagaagaaacttttttatttagttgaatttataataagagaaaaagaaaggatattatatggcaaaaataaaaaaccaatattacaacgagtctgtttcgccaattgaatatgcgcaacaaggatttaaaggaaaaatgcgttcagtaaactgaaacgtagtaaatgatgaaaaagatttagaggtatgaaatagaattacacaaaacttctgattgcctgaaaaaattccagtttcaaatgatttaacttcatgaagaactttgacaccagaatgacaagaattaattacaagaacttttacaggattaacattgttagatacaattcaagctactgttggtgatgtggctcaagttcctaactcattaactgaccatgaacaagtaatttacacaaactttgcatttatggttgcagttcacgctagatcatatggttcaatcttttcaactttatgttcaagtgaacaaattgaagaggctcatgaatgagttatcaatacagaaacattacaagaaagagctaaagcattaattccttattatgtgaatgatgaccctttaaagtcaaaagttgcagctgctttaatgccaggcttcttattatatggaggcttctatttaccattttacctatcagctagaggtaaattaccaaacacttcagatattattagattaatattaagagataaagttatacataactactatagtggttataaatatcaaaagaaagttgctaaactttctccagaaaaacaagctgaaatgaaagaatttgtttttaaattattatatgaattaatagatttagaaaaagcttatttgaaagaattgtatgaggattttggattagctgatgatgctattagatttagtgtttacaacgcaggtaaatttttacaaaatttaggttatgattcaccgtttacagaagaagaaacaagaattgagccagaaatattcacacaattatcagctagagctgatgaaaaccatgatttcttttcagggaatggctcatcatatattatgggagtttcagaagaaactgaagatgacgattgggagttttaa

SEQ ID NO: 237 - RNA, 64 nt, Mesoplasma florum
acuuauacaggguagcauaaugggcuacugaccccgccuucaaaccuauuuggagacuauaagu

SEQ ID NO: 238 - RNA, 69 nt, Artificial sequence
  synthetic Deoxyguanosine riboswitch aptamer mutations
  misc_feature (10)..(13): n at positions 10-13 can be A, C, G, or T
  misc_feature (27)..(29): n at positions 27-29 can be A, C, G, or T
  misc_feature (31)..(32): n at positions 31-32 can be A, C, G, or T
  misc_feature (33)..(40): n at positions 33-40 can be A, C, G, T, or no nucleotide
  misc_feature (44)..(46): n at positions 44-46 can be A, C, G, or T
  misc_feature (57)..(59): n at positions 57-59 can be A, C, G, or T
acuuauacannnnagcauaaugggcunnngnnnnnnnnnngccnnnaaaccuauuunnngacuauaagu

SEQ ID NO: 239 - DNA, 84 bp, Artificial sequence
  synthetic Oligo library for screen
  misc_feature (19)..(21): n at positions 19-21 can be A, C, G, or T
  misc_feature (32)..(34): n at positions 32-34 can be A, C, G, or T
  misc_feature (38)..(39): n at positions 38-39 can be A, C, G, or T
  misc_feature (40)..(47): n at positions 40-47 can be A, C, G, T, or no nucleotide
  misc_feature (49)..(51): n at positions 49-51 can be A, C, G, or T
  misc_feature (65)..(68): n at positions 65-68 can be A, C, G, or T
cgcgcgacacttatagtcnnnaaataggtttnnnggcnnnnnnnnnncnnnagcccattatgctnnnntgtataagtgccgccc

SEQ ID NO: 240 - DNA, 33 bp, Artificial sequence
  synthetic T7 promoter amplification primer
taatacgactcactatagggcggcacttataca

SEQ ID NO: 241 - DNA, 18 bp, Artificial sequence
  synthetic Reverse amplification primer
cgcgcgacacttatagtc

SEQ ID NO: 242 - DNA, 915 bp, Bacillus subtilis
tcaaaagcctggcggcgcggtcgtcagactcttttatatcgaatccccttgaaatacgaatgatatctaaaaaaacaaaattaaagttcgggaatttttattttcagcctatgcaagagattagaatcttgatataatttattacaatataataggaacactcatataatcgcgtggatatggcacgcaagtttctaccgggcaccgtaaatgtccgactatgggtgagcaatggaaccgcacgtgtacggttttttgtgatatcagcattgcttgctctttatttgagcgggcaatgctttttttattctcataacggaggtagacaggatggaagcactgaaacggaaaatagaggaagaaggcgtcgtattatctgatcaggtattgaaagtggattcttttttgaatcaccaaattgatccgctgcttatgcagagaattggtgatgaatttgcgtctaggtttgcaaaagacggtattaccaaaattgtgacaatcgaatcatcaggtatcgctcccgctgtaatgacgggcttgaagctgggtgtgccagttgtcttcgcgagaaagcataaatcgttaacactcaccgacaacttgctgacagcgtctgtttattcctttacgaagcaaacagaaagccaaatcgcagtgtctgggacccacctgtcggatcaggatcatgtgctgattatcgatgattttttggcaaatggacaggcagcgcacgggcttgtgtcgattgtgaagcaagcgggagcttctattgcgggaatcggcattgttattgaaaagtcatttcagccgggaagagatgaacttgtaaaactgggctaccgagtggaatctttggcaagaattcagtctttagaagaaggaaaagtgtccttcgtacaggaggttcattcatga

SEQ ID NO: 243 - RNA, 69 nt, Bacillus subtilis
cacucauauaaucgcguggauauggcacgcaaguuucuaccgggcaccguaaauguccgacuaugggug

SEQ ID NO: 244 - RNA, 74 nt, Artificial sequence
  synthetic Guanosine xpt riboswitch aptamer mutations
  misc_feature (11)..(14): n at positions 11-14 can be A, C, G, or T
  misc_feature (30)..(35): n at positions 30-35 can be A, C, G, or T
  misc_feature (36)..(43): n at positions 36-43 can be A, C, G, T, or no nucleotide
  misc_feature (47)..(49): n at positions 47-49 can be A, C, G, or T
  misc_feature (61)..(63): n at positions 61-63 can be A, C, G, or T
cacucauauannnncguggauauggcacgnnngnnnnnnnnnnaccnnnuaccguaaaugnnngacuaugggug

SEQ ID NO: 245 - DNA, 89 bp, Artificial sequence
  synthetic Oligo library for screen
  misc_feature (20)..(22): n at positions 20-22 can be A, C, G, or T
  misc_feature (34)..(36): n at positions 34-36 can be A, C, G, or T
  misc_feature (40)..(41): n at positions 40-41 can be A, C, G, or T
  misc_feature (42)..(49): n at positions 42-49 can be A, C, G, T, or no nucleotide
  misc_feature (51)..(53): n at positions 51-53 can be A, C, G, or T
  misc_feature (69)..(72): n at positions 69-72 can be A, C, G, or T
cgcgcgaccacccatagtcnnncatttacggtgnnnggtnnnnnnnnnncnnncgtgccatatccacgnnnntatatgagtggccgccc

SEQ ID NO: 246 - DNA, 34 bp, Artificial sequence
  synthetic T7 promoter amplification primer
taatacgactcactatagggcggccactcatata

SEQ ID NO: 247 - DNA, 19 bp, Artificial sequence
  synthetic Reverse amplification primer
cgcgcgaccacccatagtc

SEQ ID NO: 248 - RNA, 152 nt, Artificial sequence
  synthetic Oligo 1 Transcribed RNA
gggcggcacuuauacaggguagcauaaugggcuacugacgccuucaaaccuauuuggagacuauaagugucgcgcggggcggcacuuauacaggguagcauaaugggcuacugacgccuucaaaccuauuuggagacuauaagugucgcgcg

SEQ ID NO: 249 - DNA, 76 bp, Artificial sequence
  synthetic Oligo 1 Synthesized template
cgcgcgacacttatagtctccaaataggtttgaaggcgtcagtagcccattatgctaccctgtataagtgccgccc

SEQ ID NO: 250 - RNA, 79 nt, Artificial sequence
  synthetic Oligo 2 Transcribed RNA
gggcggcacuuauacaggguagcauaaugggcuacugaccccgccuucaaaccuauuuggagacuauaagugucgcgcg

SEQ ID NO: 251 - DNA, 79 bp, Artificial sequence
  synthetic Oligo 2 Synthesized template
cgcgcgacacttatagtctccaaataggtttgaaggcggggtcagtagcccattatgctaccctgtataagtgccgccc

SEQ ID NO: 252 - protein, 560 aa, Artificial sequence
  synthetic DAFss-aCD3scFv(UCHT1)IgG1 Fc-CD14GPI
MTVARPSVPAALPLLGELPRLLLLVLLCLPDIQMTQSPSSLSASVGDRVTITCRASQDIRNYLNWYQQKPGKAPKLLIYYTSRLESGVPSRFSGSGSGTDYTLTISSLQPEDFATYYCQQGNTLPWTFGQGTKVEIKGGGGSGGGGSGGGGSEVQLVESGGGLVQPGGSLRLSCAASGYSFTGYTMNWVRQAPGKGLEWVALINPYKGVSTYNQKFKDRFTISVDKSKNTAYLQMNSLRAEDTAVYYCARSGYYGDSDWYFDVWGQGTLVTVSSEPKSCDKTHTCPPCPAPELLGGPSVFLFPPKPKDTLMISRTPEVTCVVVDVSHEDPEVKFNWYVDGVEVHNAKTKPREEQYNSTYRVVSVLTVLHQDWLNGKEYKCKVSNKALPAPIEKTISKAKGQPREPQVYTLPPSREEMTKNQVSLTCLVKGFYPSDIAVEWESNGQPENNYKTTPPVLDSDGSFFLYSKLTVDKSRWQQGNVFSCSVMHEALHNHYTQKSLSLSPGVDNLTLDGNPFLVPGTALPHEGSMNSGVVPACARSTLSVGVSGTLVLLQGARGFA

SEQ ID NO: 253 - protein, 276 aa, Artificial sequence
  synthetic DAFss-CD80ECD-CD16GPI
MTVARPSVPAALPLLGELPRLLLLVLLCLPVIHVTKEVKEVATLSCGHNVSVEELAQTRIYWQKEKKMVLTMMSGDMNIWPEYKNRTIFDITNNLSIVILALRPSDEGTYECVVLKYEKDAFKREHLAEVTLSVKADFPTPSISDFEIPTSNIRRIICSTSGGFPEPHLSWLENGEELNAINTTVSQDPETELYAVSSKLDFNMTTNHSFMCLIKYGHLRVNQTFNWNTTKQEHFPDNVSTISSFSPPGYQVSFCLVMVLLFAVDTGLYFSVKTNI

SEQ ID NO: 254 - protein, 533 aa, Artificial sequence
  synthetic DAFss-IL7-DAF
MATTMTVARPSVPAALPLLGELPRLLLLVLLCLPADCDIEGKDGKQYESVLMVSIDQLLDSMKEIGSNCLNNEFNFFKRHICDANKEGMFLFRAARKLRQFLKMNSTGDFDLHLLKVSEGTTILLNCTGQVKGRKPAALGEAQPTKSLEENKSLKEQKKLNDLCFLKRLLQEIKTCWNKILMGTKEHCGLPPDVPNAQPALEGRTSFPEDTVITYKCEESFVKIPGEKDSVICLKGSQWSDIEEFCNRSCEVPTRLNSASLKQPYITQNYFPVGTVVEYECRPGYRREPSLSPKLTCLQNLKWSTAVEFCKKKSCPNPGEIRNGQIDVPGGILFGATISFSCNTGYKLFGSTSSFCLISGSSVQWSDPLPECREIYCPAPPQIDNGIIQGERDHYGYRQSVTYACNKGFTMIGEHSIYCTVNNDEGEWSGPPPECRGKSLTSKVPPTVQKPTTVNVPTTEVSPTSQKTTTKTTTPNAQATRSTPVSRTTKHFHETTPNKGSGTTSGTTRLLSGHTCFTLTGLLGTLVTMGLLT

SEQ ID NO: 255 - DNA, 1823 bp, Artificial sequence
  synthetic EF-1a promoter with miRs
ggctccggtgcccgtcagtgggcagagcgcacatcgcccacagtccccgagaagttggggggaggggtcggcaattgaaccggtgcctagagaaggtggcgcggggtaaactgggaaagtgatgtcgtgtactggctccgcctttttcccgagggtgggggagaaccgtatataagtgcagtagtcgccgtgaacgttctttttcgcaacgggtttgccgccagaacacaggtaagtgccgtgtgtggttcccgcgggcctggcctctttacgggttatggcccttgcgtgccttgaattacttccacctggctgcagtacgtgattcttgatcccgagcttcgggttggaagtgggtgggagagttcgaggccttgcgcttaaggagccccttcgcctcgtgcttgagttgaggcctggcctgggcgctggggccgccgcgtgcgaatctggtggcaccttcgcgcctgtctcgctgctttcgataagtctctagccatttaaaatttttgatgacctgctgcgacgctttttttctggcaagatagtcttgtaaatgcgggccaagatctgcacactggtatttcggtttttggggccgcgggcggcgacggggcccgtgcgtcccagcgcacatgttcggcgaggcggggcctgcgagcgcggccaccgagaatcggacgggggtagtctcaagctggccggcctgctctggtgcctggcctcgcgccgccgtgtatcgccccgccctgggcggcaaggctggcccggtcggcaccagttgcgtgagcggaaagatggccgcttcccggccctgctgcagggagctcaaaatggaggacgcggcgctcgggagagcgggcgggtgagtcacccacacaaaggaaaagggcctttccgtcctcagccgtcgcttcatgtgactccactgagtaccgggcgccgtccaggcacctcgattagttcctggaggcttgctgaaggctgtatgctgacatggtacagttcaatggtggttttggccactgactgaccaccattgctgtaccatgtcaggacacaaggcctgttactagcactcacatggaacaaatggcccacattggtgccggatgaagctcttatgttgcacggtcatctggaggcttgctgaaggctgtatgctgtcagtctgttcatcttctggcgttttggccactgactgacgccagaaggaacagactgacaggacacaaggcctgttactagcactcacatggaacaaatggccgttgccggagtcttggcagcgagagatcactatcaactaactggaggcttgctgaaggctgtatgctgaagcgtgaagtgaatcaacgggttttggccactgactgacccgttgatacttcacgcttcaggacacaaggcctgttactagcactcacatggaacaaatggccgtgttaattgtccatgtagcgaggcatccttatggcgtggctggaggcttgctgaaggctgtatgctggcagtatcctagtacattgacgttttggccactgactgacgtcaatgttaggatactgccaggacacaaggcctgttactagcactcacatggaacaaatggccgcttttggagtacgtcgtctttaggttggggggaggggttttatgcgatggagtttccccacactgagtgggtggagactgaagttaggccagcttggcacttgatgtaattctccttggaatttgccctttttgagtttggatcttggttcattctcaagcctcagacagtggttcaaagtttttttcttccatttcaggtgtcgtga

SEQ ID NO: 256 - DNA, 28 bp, Mus musculus
ctggaggcttgctgaaggctgtatgctg

SEQ ID NO: 257 - DNA, 21 bp, Artificial sequence
  Synthetic DNA encoding MiRNA stem
acatggtacagttcaatggtg

SEQ ID NO: 258 - DNA, 19 bp, Artificial sequence
  synthetic DNA encoding loop
gttttggccactgactgac

SEQ ID NO: 259 - DNA, 19 bp, Artificial sequence
  synthetic DNA encoding stem
caccattgctgtaccatgt

SEQ ID NO: 260 - DNA, 45 bp, Mus musculus
caggacacaaggcctgttactagcactcacatggaacaaatggcc

SEQ ID NO: 261 - DNA, 21 bp, Artificial sequence
  Synthetic DNA encoding MiRNA stem
tcagtctgttcatcttctggc

SEQ ID NO: 262 - DNA, 19 bp, Artificial sequence
  Synthetic DNA encoding MiRNA stem
gccagaaggaacagactga

SEQ ID NO: 263 - DNA, 21 bp, Artificial sequence
  Synthetic DNA encoding MiRNA stem
aagcgtgaagtgaatcaacgg

SEQ ID NO: 264 - DNA, 19 bp, Artificial sequence
  Synthetic DNA encoding MiRNA stem
ccgttgatacttcacgctt

SEQ ID NO: 265 - DNA, 21 bp, Artificial sequence
  Synthetic DNA encoding MiRNA stem
gcagtatcctagtacattgac

SEQ ID NO: 266 - DNA, 19 bp, Artificial sequence
  Synthetic DNA encoding MiRNA stem
gtcaatgttaggatactgc

SEQ ID NO: 267 - DNA, 21 bp, Artificial sequence
  Synthetic DNA encoding MiRNA stem
atatgtacttggctggacagc

SEQ ID NO: 268 - DNA, 19 bp, Artificial sequence
  Synthetic DNA encoding MiRNA stem
gctgtccacaagtacatat

SEQ ID NO: 269 - DNA, 39 bp, Artificial sequence
  synthetic DNA encoding linker
cacattggtgccggatgaagctcttatgttgccggtcat

SEQ ID NO: 270 - DNA, 21 bp, Artificial sequence
  Synthetic DNA encoding MiRNA stem
ctgttaatgctaatcgtgata

SEQ ID NO: 271 - DNA, 18 bp, Artificial sequence
  Synthetic DNA encoding MiRNA stem
tatcacgattattaacag

SEQ ID NO: 272 - DNA, 40 bp, Artificial sequence
  synthetic DNA encoding linker
gttgccggagtcttggcagcgagagatcactatcaactaa

SEQ ID NO: 273 - DNA, 21 bp, Artificial sequence
  Synthetic DNA encoding MiRNA stem
taccagtttagcacgaagctc

SEQ ID NO: 274 - DNA, 19 bp, Artificial sequence
  Synthetic DNA encoding MiRNA stem
gagcttcgctaaactggta

SEQ ID NO: 275 - DNA, 40 bp, Artificial sequence
  synthetic DNA encoding linker
gtgttaattgtccatgtagcgaggcatccttatggcgtgg

SEQ ID NO: 276 - DNA, 21 bp, Artificial sequence
  Synthetic DNA encoding MiRNA stem
tgccgctgaaatccaaggcaa

SEQ ID NO: 277 - DNA, 19 bp, Artificial sequence
  Synthetic DNA encoding MiRNA stem
ttgccttgtttcagcggca

SEQ ID NO: 278 - protein, 534 aa, Artificial sequence
  Synthetic UCHT1scFvFc-GPI
MDMRVPAQLLGLLLLWLSGARCDIQMTQSPSSLSASVGDRVTITCRASQDIRNYLNWYQQKPGKAPKLLIYYTSRLESGVPSRFSGSGSGTDYTLTISSLQPEDFATYYCQQGNTLPWTFGQGTKVEIKGGGGSGGGGSGGGGSEVQLVESGGGLVQPGGSLRLSCAASGYSFTGYTMNWVRQAPGKGLEWVALINPYKGVSTYNQKFKDRFTISVDKSKNTAYLQMNSLRAEDTAVYYCARSGYYGDSDWYFDVWGQGTLVTVSSEPKSCDKTHTCPPCPAPELLGGPSVFLFPPKPKDTLMISRTPEVTCVVVDVSHEDPEVKFNWYVDGVEVHNAKTKPREEQYNSTYRVVSVLTVLHQDWLNGKEYKCKVSNKALPTPIEKTISKAKGQPREPQVYTLPPSREEMTKNQVSLTCLVKGFYPSDIAVEWESNGQPENNYKTTPPVLDSDGSFFLYSKLTVDKSRWQQGNVFSCSVMHEALHNHYTQKSLSLSPGPNKGSGTTSGTTRLLSGHTCFTLTGLLGTLVTMGLLT

SEQ ID NO: 279 - protein, 530 aa, Artificial sequence
  Synthetic OKT3scFvFc-GPI
MDMRVPAQLLGLLLLWLSGARCQIVLTQSPAIMSASPGEKVTMTCSASSSVSYMNWYQQKSGTSPKRWIYDTSKLASGVPAHFRGSGSGTSYSLTISGMEAEDAATYYCQQWSSNPFTFGSGTKLEINGGGGSGGGGSGGGGSQVQLQQSGAELARPGASVKMSCKASGYTFTRYTMHWVKQRPGQGLEWIGYINPSRGYTNYNQKFKDKATLTTDKSSSTAYMQLSSLTSEDSAVYYCARYYDDHYCLDYWGQGTTLTVSSEPKSCDKTHTCPPCPAPELLGGPSVFLFPPKPKDTLMISRTPEVTCVVVDVSHEDPEVKFNWYVDGVEVHNAKTKPREEQYNSTYRVVSVLTVLHQDWLNGKEYKCKVSNKALPAPIEKTISKAKGQPREPQVYTLPPSREEMTKNQVSLTCLVKGFYPSDIAVEWESNGQPENNYKTTPPVLDSDGSFFLYSKLTVDKSRWQQGNVFSCSVMHEALHNHYTQKSLSLSPGPNKGSGTTSGTTRLLSGHTCFTLTGLLGTLVTMGLLT

SEQ ID NO: 280 - protein, 280 aa, Artificial sequence
  Synthetic hCD80-CD16 GPI
MGHTRRQGTSPSKCPYLNFFQLLVLAGLSHFCSGVIHVTKEVKEVATLSCGHNVSVEELAQTRIYWQKEKKMVLTMMSGDMNIWPEYKNRTIFDITNNLSIVILALRPSDEGTYECVVLKYEKDAFKREHLAEVTLSVKADFPTPSISDFEIPTSNIRRIICSTSGGFPEPHLSWLENGEELNAINTTVSQDPETELYAVSSKLDFNMTTNHSFMCLIKYGHLRVNQTFNWNTTKQEHFPDNVSTISSFSPPGYQVSFCLVMVLLFAVDTGLYFSVKTNI

SEQ ID NO: 281 - protein, 120 aa, Artificial sequence
  Synthetic Target 1 MRB VH
EVQLVQSGAEVKKPGATVKISCKVSGYSFWGATMNWIRQPPGKGLEWIGLIKPSNGGTSYNQKFKGRVTISADKSISTAYLQWSSLKASDTAMYYCAHGHYESYEAMDYWGQGTLVTVSS

SEQ ID NO: 282 - protein, 107 aa, Artificial sequence
  Synthetic Target 1 MRB VL
DIQMTQSPSSLSASVGDRVTITCKASQDVVSAVAWYQQKPGQAPRLLIYWQDTRHTGVPSRFSGSGSGTEFTLTISSLQPDDFATYYCQEHFSPPLTFGQGTKVEIK

SEQ ID NO: 283 - protein, 15 aa, Artificial sequence
  Synthetic Linker 1
GGGGSGGGGSGGGGS

SEQ ID NO: 284 - protein, 357 aa, Artificial sequence; identical to SEQ ID NO: 78
  Synthetic C1 control polypeptide containing GMCSF alpha chain signal sequence (amino acids 1-22) and eTAG (amino acids 23-357)

SEQ ID NO: 285 - protein, 240 aa, Artificial sequence
  Synthetic OKT3 ScFv
QIVLTQSPAIMSASPGEKVTMTCSASSSVSYMNWYQQKSGTSPKRWIYDTSKLASGVPAHFRGSGSGTSYSLTISGMEAEDAATYYCQQWSSNPFTFGSGTKLEINGGGGSGGGGSGGGGSQVQLQQSGAELARPGASVKMSCKASGYTFTRYTMHWVKQRPGQGLEWIGYINPSRGYTNYNQKFKDKATLTTDKSSSTAYMQLSSLTSEDSAVYYCARYYDDHYCLDYWGQGTTLTVSS

SEQ ID NO: 286 - protein, 532 aa, Artificial sequence
  Synthetic DAFss-IL7-DAF fusion
MTVARPSVPAALPLLGELPRLLLLVLLCLPAVWGDCDIEGKDGKQYESVLMVSIDQLLDSMKEIGSNCLNNEFNFFKRHICDANKEGMFLFRAARKLRQFLKMNSTGDFDLHLLKVSEGTTILLNCTGQVKGRKPAALGEAQPTKSLEENKSLKEQKKLNDLCFLKRLLQEIKTCWNKILMGTKEHCGLPPDVPNAQPALEGRTSFPEDTVITYKCEESFVKIPGEKDSVICLKGSQWSDIEEFCNRSCEVPTRLNSASLKQPYITQNYFPVGTVVEYECRPGYRREPSLSPKLTCLQNLKWSTAVEFCKKKSCPNPGEIRNGQIDVPGGILFGATISFSCNTGYKLFGSTSSFCLISGSSVQWSDPLPECREIYCPAPPQIDNGIIQGERDHYGYRQSVTYACNKGFTMIGEHSIYCTVNNDEGEWSGPPPECRGKSLTSKVPPTVQKPTTVNVPTTEVSPTSQKTTTKTTTPNAQATRSTPVSRTTKHFHETTPNKGSGTTSGTTRLLSGHTCFTLTGLLGTLVTMGLLT

SEQ ID NO: 287 - protein, 564 aa, Artificial sequence
  Synthetic DAFss-aCD3scFv(UCHT1)IgG1 Fc-CD14GPI
MTVARPSVPAALPLLGELPRLLLLVLLCLPAVWGDIQMTQSPSSLSASVGDRVTITCRASQDIRNYLNWYQQKPGKAPKLLIYYTSRLESGVPSRFSGSGSGTDYTLTISSLQPEDFATYYCQQGNTLPWTFGQGTKVEIKGGGGSGGGGSGGGGSEVQLVESGGGLVQPGGSLRLSCAASGYSFTGYTMNWVRQAPGKGLEWVALINPYKGVSTYNQKFKDRFTISVDKSKNTAYLQMNSLRAEDTAVYYCARSGYYGDSDWYFDVWGQGTLVTVSSEPKSCDKTHTCPPCPAPELLGGPSVFLFPPKPKDTLMISRTPEVTCVVVDVSHEDPEVKFNWYVDGVEVHNAKTKPREEQYNSTYRVVSVLTVLHQDWLNGKEYKCKVSNKALPAPIEKTISKAKGQPREPQVYTLPPSREEMTKNQVSLTCLVKGFYPSDIAVEWESNGQPENNYKTTPPVLDSDGSFFLYSKLTVDKSRWQQGNVFSCSVMHEALHNHYTQKSLSLSPGVDNLTLDGNPFLVPGTALPHEGSMNSGVVPACARSTLSVGVSGTLVLLQGARGFA

SEQ ID NO: 288 - protein, 280 aa, Artificial sequence
  Synthetic DAFss-CD80ECD-CD16GPI
MTVARPSVPAALPLLGELPRLLLLVLLCLPAVWGVIHVTKEVKEVATLSCGHNVSVEELAQTRIYWQKEKKMVLTMMSGDMNIWPEYKNRTIFDITNNLSIVILALRPSDEGTYECVVLKYEKDAFKREHLAEVTLSVKADFPTPSISDFEIPTSNIRRIICSTSGGFPEPHLSWLENGEELNAINTTVSQDPETELYAVSSKLDFNMTTNHSFMCLIKYGHLRVNQTFNWNTTKQEHFPDNVSTISSFSPPGYQVSFCLVMVLLFAVDTGLYFSVKTNI

SEQ ID NO: 289 - protein, 119 aa, Artificial sequence
  Synthetic Target 2 MRB VH
QVQLQESGPGLVKPSQTLSLTCTVSGYSITTGEYWNWVRQARGQRLEWIGYITYDGSKNYNPSLKNRVTISVDTSKNQFSLKLSSVTAADTAVYYCSRFEGVWYGLDYWGQGTLVTVSS

SEQ ID NO: 290 - protein, 111 aa, Artificial sequence
  Synthetic Target 2 MRB VL
AIQLTQSPSSLSASVGDRVTITCRASESVDRYGNSFIHWYQQKPGKAPKLLIYRTYNLESGIPARFSGSGSGTEFTLTISSLQSEDFAVYYCQQTNEDPWTFGQGTKVEIK

SEQ ID NO: 291 - protein, 30 aa, Artificial sequence; identical to SEQ ID NO: 54
  Synthetic Linker2

SEQ ID NO: 292 - protein, 368 aa, Artificial sequence
  synthetic polypeptide M001
MLLLVTSLLLCELPHPAFLLIPRKVCNGIGIGEFKDSLSINATNIKHFKNCTSISGDLHILPVAFRGDSFTHTPPLDPQELDILKTVKEITGFLLIQAWPENRTDLHAFENLEIIRGRTKQHGQFSLAVVSLNITSLGLRSLKEISDGDVIISGNKNLCYANTINWKKLFGTSGQKTKIISNRGENSCKATGQVCHALCSPEGCWGPEPRDCVSCRNVSRGRECVDKCNLLEGEPREFVENSECIQCHPECLPQAMNITCTGRGPDNCIQCAHYIDGPHCVKTCPAGVMGENNTLVWKYADAGHVCHLCHPNCTYGCTGPGLEGCPTNGPEINNSSGEMDPILLPPCLTISILSFFSVALLVILACVL

SEQ ID NO: 293 - protein, 232 aa, Artificial sequence
  synthetic polypeptide M002
MLLLVTSLLLCELPHPAFLLIPRKVCNGIGIGEFKDSLSINATNIKHFKNCTSISGDLHILPVAFRGDSFTHTPPLDPQELDILKTVKEITGFLLIQAWPENRTDLHAFENLEIIRGRTKQHGQFSLAVVSLNITSLGLRSLKEISDGDVIISGNKNLCYANTINWKKLFGTSGQKTKIISNRGENSCKATGQPEINNSSGEMDPILLPPCLTISILSFFSVALLVILACVL

SEQ ID NO: 294 - protein, 194 aa, Artificial sequence
  synthetic polypeptide M007
MEQKLISEEDLEHDLERGPPGPRRPPRGPPLSSSLGLALLLLLLALLFWLYIVMSDWTGGALLVLYSFALMLIIIILIIFIFRRDLLCPLGALCILLLMITLLLIALWNLHGQALFLGIVLFIFGCLLVLGIWIYLLEMLWRLGATIWQLLAFFLAFFLDLILLIIALYLQQNWWTLLVDLLWLLLFLAILIWM

SEQ ID NO: 295 - protein, 174 aa, Artificial sequence
  synthetic polypeptide M008
MEQKLISEEDLSSSLGLALLLLLLALLFWLYIVMSDWTGGALLVLYSFALMLIIIILIIFIFRRDLLCPLGALCILLLMITLLLIALWNLHGQALFLGIVLFIFGCLLVLGIWIYLLEMLWRLGATIWQLLAFFLAFFLDLILLIIALYLQQNWWTLLVDLLWLLLFLAILIWM

SEQ ID NO: 296 - protein, 184 aa, Artificial sequence
  synthetic polypeptide M009
MEHDLERGPPGPRRPPRGPPLSSSLGLALLLLLLALLFWLYIVMSDWTGGALLVLYSFALMLIIIILIIFIFRRDLLCPLGALCILLLMITLLLIALWNLHGQALFLGIVLFIFGCLLVLGIWIYLLEMLWRLGATIWQLLAFFLAFFLDLILLIIALYLQQNWWTLLVDLLWLLLFLAILIWM

SEQ ID NO: 297 - protein, 162 aa, Artificial sequence
  synthetic polypeptide M010
MSLGLALLLLLLALLFWLYIVMSDWTGGALLVLYSFALMLIIIILIIFIFRRDLLCPLGALCILLLMITLLLIALWNLHGQALFLGIVLFIFGCLLVLGIWIYLLEMLWRLGATIWQLLAFFLAFFLDLILLIIALYLQQNWWTLLVDLLWLLLFLAILIWM

SEQ ID NO: 298 - protein, 363 aa, Artificial sequence
  synthetic polypeptide M012
MLLLVTSLLLCELPHPAFLLIPRKVCNGIGIGEFKDSLSINATNIKHFKNCTSISGDLHILPVAFRGDSFTHTPPLDPQELDILKTVKEITGFLLIQAWPENRTDLHAFENLEIIRGRTKQHGQFSLAVVSLNITSLGLRSLKEISDGDVIISGNKNLCYANTINWKKLFGTSGQKTKIISNRGENSCKATGQVCHALCSPEGCWGPEPRDCVSCRNVSRGRECVDKCNLLEGEPREFVENSECIQCHPECLPQAMNITCTGRGPDNCIQCAHYIDGPHCVKTCPAGVMGENNTLVWKYADAGHVCHLCHPNCTYGCTGPGLEGCPTNGAETPTPPKPKLSKCILISSLAILLMVSLLLLSLW

SEQ ID NO: 299 - protein, 227 aa, Artificial sequence
  synthetic polypeptide M013
MLLLVTSLLLCELPHPAFLLIPRKVCNGIGIGEFKDSLSINATNIKHFKNCTSISGDLHILPVAFRGDSFTHTPPLDPQELDILKTVKEITGFLLIQAWPENRTDLHAFENLEIIRGRTKQHGQFSLAVVSLNITSLGLRSLKEISDGDVIISGNKNLCYANTINWKKLFGTSGQKTKIISNRGENSCKATGQAETPTPPKPKLSKCILISSLAILLMVSLLLLSLW

SEQ ID NO: 300 - protein, 354 aa, Artificial sequence
  synthetic polypeptide M018
MLLLVTSLLLCELPHPAFLLIPRKVCNGIGIGEFKDSLSINATNIKHFKNCTSISGDLHILPVAFRGDSFTHTPPLDPQELDILKTVKEITGFLLIQAWPENRTDLHAFENLEIIRGRTKQHGQFSLAVVSLNITSLGLRSLKEISDGDVIISGNKNLCYANTINWKKLFGTSGQKTKIISNRGENSCKATGQVCHALCSPEGCWGPEPRDCVSCRNVSRGRECVDKCNLLEGEPREFVENSECIQCHPECLPQAMNITCTGRGPDNCIQCAHYIDGPHCVKTCPAGVMGENNTLVWKYADAGHVCHLCHPNCTYGCTGPGLEGCPTNGTESVLPMWVLALIEIFLTIAVLLAL

SEQ ID NO: 301 - protein, 218 aa, Artificial sequence
  synthetic polypeptide M019
MLLLVTSLLLCELPHPAFLLIPRKVCNGIGIGEFKDSLSINATNIKHFKNCTSISGDLHILPVAFRGDSFTHTPPLDPQELDILKTVKEITGFLLIQAWPENRTDLHAFENLEIIRGRTKQHGQFSLAVVSLNITSLGLRSLKEISDGDVIISGNKNLCYANTINWKKLFGTSGQKTKIISNRGENSCKATGQTESVLPMWVLALIEIFLTIAVLLAL

SEQ ID NO: 302 - protein, 360 aa, Artificial sequence
  synthetic polypeptide M024
MLLLVTSLLLCELPHPAFLLIPRKVCNGIGIGEFKDSLSINATNIKHFKNCTSISGDLHILPVAFRGDSFTHTPPLDPQELDILKTVKEITGFLLIQAWPENRTDLHAFENLEIIRGRTKQHGQFSLAVVSLNITSLGLRSLKEISDGDVIISGNKNLCYANTINWKKLFGTSGQKTKIISNRGENSCKATGQVCHALCSPEGCWGPEPRDCVSCRNVSRGRECVDKCNLLEGEPREFVENSECIQCHPECLPQAMNITCTGRGPDNCIQCAHYIDGPHCVKTCPAGVMGENNTLVWKYADAGHVCHLCHPNCTYGCTGPGLEGCPTNGTPEGSELHIILGLFGLLLLLNCLCGTAWLCC

SEQ ID NO: 303 - protein, 224 aa, Artificial sequence
  synthetic polypeptide M025
MLLLVTSLLLCELPHPAFLLIPRKVCNGIGIGEFKDSLSINATNIKHFKNCTSISGDLHILPVAFRGDSFTHTPPLDPQELDILKTVKEITGFLLIQAWPENRTDLHAFENLEIIRGRTKQHGQFSLAVVSLNITSLGLRSLKEISDGDVIISGNKNLCYANTINWKKLFGTSGQKTKIISNRGENSCKATGQTPEGSELHIILGLFGLLLLLNCLCGTAWLCC

SEQ ID NO: 304 - protein, 359 aa, Artificial sequence
  synthetic polypeptide M030
MLLLVTSLLLCELPHPAFLLIPRKVCNGIGIGEFKDSLSINATNIKHFKNCTSISGDLHILPVAFRGDSFTHTPPLDPQELDILKTVKEITGFLLIQAWPENRTDLHAFENLEIIRGRTKQHGQFSLAVVSLNITSLGLRSLKEISDGDVIISGNKNLCYANTINWKKLFGTSGQKTKIISNRGENSCKATGQVCHALCSPEGCWGPEPRDCVSCRNVSRGRECVDKCNLLEGEPREFVENSECIQCHPECLPQAMNITCTGRGPDNCIQCAHYIDGPHCVKTCPAGVMGENNTLVWKYADAGHVCHLCHPNCTYGCTGPGLEGCPTNGTPSDLDPCCLTLSLILVVILVLLTVLALLS

SEQ ID NO: 305 - protein, 223 aa, Artificial sequence
  synthetic polypeptide M031
MLLLVTSLLLCELPHPAFLLIPRKVCNGIGIGEFKDSLSINATNIKHFKNCTSISGDLHILPVAFRGDSFTHTPPLDPQELDILKTVKEITGFLLIQAWPENRTDLHAFENLEIIRGRTKQHGQFSLAVVSLNITSLGLRSLKEISDGDVIISGNKNLCYANTINWKKLFGTSGQKTKIISNRGENSCKATGQTPSDLDPCCLTLSLILVVILVLLTVLALLS

SEQ ID NO: 306 - protein, 368 aa, Artificial sequence
  synthetic polypeptide M036
MLLLVTSLLLCELPHPAFLLIPRKVCNGIGIGEFKDSLSINATNIKHFKNCTSISGDLHILPVAFRGDSFTHTPPLDPQELDILKTVKEITGFLLIQAWPENRTDLHAFENLEIIRGRTKQHGQFSLAVVSLNITSLGLRSLKEISDGDVIISGNKNLCYANTINWKKLFGTSGQKTKIISNRGENSCKATGQVCHALCSPEGCWGPEPRDCVSCRNVSRGRECVDKCNLLEGEPREFVENSECIQCHPECLPQAMNITCTGRGPDNCIQCAHYIDGPHCVKTCPAGVMGENNTLVWKYADAGHVCHLCHPNCTYGCTGPGLEGCPTNGTLPQMSQFTCCEDFYFPWLLCIIFGIFGLTVMLFVFLFS

SEQ ID NO: 307 - protein, 232 aa, Artificial sequence
  synthetic polypeptide M037
MLLLVTSLLLCELPHPAFLLIPRKVCNGIGIGEFKDSLSINATNIKHFKNCTSISGDLHILPVAFRGDSFTHTPPLDPQELDILKTVKEITGFLLIQAWPENRTDLHAFENLEIIRGRTKQHGQFSLAVVSLNITSLGLRSLKEISDGDVIISGNKNLCYANTINWKKLFGTSGQKTKIISNRGENSCKATGQTLPQMSQFTCCEDFYFPWLLCIIFGIFGLTVMLFVFLFS

SEQ ID NO: 308 - protein, 360 aa, Artificial sequence
  synthetic polypeptide M042
MLLLVTSLLLCELPHPAFLLIPRKVCNGIGIGEFKDSLSINATNIKHFKNCTSISGDLHILPVAFRGDSFTHTPPLDPQELDILKTVKEITGFLLIQAWPENRTDLHAFENLEIIRGRTKQHGQFSLAVVSLNITSLGLRSLKEISDGDVIISGNKNLCYANTINWKKLFGTSGQKTKIISNRGENSCKATGQVCHALCSPEGCWGPEPRDCVSCRNVSRGRECVDKCNLLEGEPREFVENSECIQCHPECLPQAMNITCTGRGPDNCIQCAHYIDGPHCVKTCPAGVMGENNTLVWKYADAGHVCHLCHPNCTYGCTGPGLEGCPTNGHLPDNTLRWKVLPGILCLWGLFLLGCGLSLA

SEQ ID NO: 309 - protein, 224 aa, Artificial sequence
  synthetic polypeptide M043
MLLLVTSLLLCELPHPAFLLIPRKVCNGIGIGEFKDSLSINATNIKHFKNCTSISGDLHILPVAFRGDSFTHTPPLDPQELDILKTVKEITGFLLIQAWPENRTDLHAFENLEIIRGRTKQHGQFSLAVVSLNITSLGLRSLKEISDGDVIISGNKNLCYANTINWKKLFGTSGQKTKIISNRGENSCKATGQHLPDNTLRWKVLPGILCLWGLFLLGCGLSLA

SEQ ID NO: 310 - protein, 359 aa, Artificial sequence
  synthetic polypeptide M048
MLLLVTSLLLCELPHPAFLLIPRKVCNGIGIGEFKDSLSINATNIKHFKNCTSISGDLHILPVAFRGDSFTHTPPLDPQELDILKTVKEITGFLLIQAWPENRTDLHAFENLEIIRGRTKQHGQFSLAVVSLNITSLGLRSLKEISDGDVIISGNKNLCYANTINWKKLFGTSGQKTKIISNRGENSCKATGQVCHALCSPEGCWGPEPRDCVSCRNVSRGRECVDKCNLLEGEPREFVENSECIQCHPECLPQAMNITCTGRGPDNCIQCAHYIDGPHCVKTCPAGVMGENNTLVWKYADAGHVCHLCHPNCTYGCTGPGLEGCPTNGETATETAWISLVTALHLVLGLNAVLGLLLL

SEQ ID NO: 311 - protein, 223 aa, Artificial sequence
  synthetic polypeptide M049
MLLLVTSLLLCELPHPAFLLIPRKVCNGIGIGEFKDSLSINATNIKHFKNCTSISGDLHILPVAFRGDSFTHTPPLDPQELDILKTVKEITGFLLIQAWPENRTDLHAFENLEIIRGRTKQHGQFSLAVVSLNITSLGLRSLKEISDGDVIISGNKNLCYANTINWKKLFGTSGQKTKIISNRGENSCKATGQETATETAWISLVTALHLVLGLNAVLGLLLL

SEQ ID NO: 312 - protein, 368 aa, Artificial sequence
  synthetic polypeptide E006
MLLLVTSLLLCELPHPAFLLIPRKVCNGIGIGEFKDSLSINATNIKHFKNCTSISGDLHILPVAFRGDSFTHTPPLDPQELDILKTVKEITGFLLIQAWPENRTDLHAFENLEIIRGRTKQHGQFSLAVVSLNITSLGLRSLKEISDGDVIISGNKNLCYANTINWKKLFGTSGQKTKIISNRGENSCKATGQVCHALCSPEGCWGPEPRDCVSCRNVSRGRECVDKCNLLEGEPREFVENSECIQCHPECLPQAMNITCTGRGPDNCIQCAHYIDGPHCVKTCPAGVMGENNTLVWKYADAGHVCHLCHPNCTYGCTGPGLEGCPTNGLERIARLEEKVKTLKAQNSELASTANMLREQVAQLKQKV

SEQ ID NO: 313 - protein, 369 aa, Artificial sequence
  synthetic polypeptide E007
MLLLVTSLLLCELPHPAFLLIPRKVCNGIGIGEFKDSLSINATNIKHFKNCTSISGDLHILPVAFRGDSFTHTPPLDPQELDILKTVKEITGFLLIQAWPENRTDLHAFENLEIIRGRTKQHGQFSLAVVSLNITSLGLRSLKEISDGDVIISGNKNLCYANTINWKKLFGTSGQKTKIISNRGENSCKATGQVCHALCSPEGCWGPEPRDCVSCRNVSRGRECVDKCNLLEGEPREFVENSECIQCHPECLPQAMNITCTGRGPDNCIQCAHYIDGPHCVKTCPAGVMGENNTLVWKYADAGHVCHLCHPNCTYGCTGPGLEGCPTNGLERIARLEEKVKTLKAQNSELASTANMLREQVAQLKQKVA

SEQ ID NO: 314 - protein, 370 aa, Artificial sequence
  synthetic polypeptide E008
MLLLVTSLLLCELPHPAFLLIPRKVCNGIGIGEFKDSLSINATNIKHFKNCTSISGDLHILPVAFRGDSFTHTPPLDPQELDILKTVKEITGFLLIQAWPENRTDLHAFENLEIIRGRTKQHGQFSLAVVSLNITSLGLRSLKEISDGDVIISGNKNLCYANTINWKKLFGTSGQKTKIISNRGENSCKATGQVCHALCSPEGCWGPEPRDCVSCRNVSRGRECVDKCNLLEGEPREFVENSECIQCHPECLPQAMNITCTGRGPDNCIQCAHYIDGPHCVKTCPAGVMGENNTLVWKYADAGHVCHLCHPNCTYGCTGPGLEGCPTNGLERIARLEEKVKTLKAQNSELASTANMLREQVAQLKQKVAA

SEQ ID NO: 315 - protein, 371 aa, Artificial sequence
  synthetic polypeptide E009
MLLLVTSLLLCELPHPAFLLIPRKVCNGIGIGEFKDSLSINATNIKHFKNCTSISGDLHILPVAFRGDSFTHTPPLDPQELDILKTVKEITGFLLIQAWPENRTDLHAFENLEIIRGRTKQHGQFSLAVVSLNITSLGLRSLKEISDGDVIISGNKNLCYANTINWKKLFGTSGQKTKIISNRGENSCKATGQVCHALCSPEGCWGPEPRDCVSCRNVSRGRECVDKCNLLEGEPREFVENSECIQCHPECLPQAMNITCTGRGPDNCIQCAHYIDGPHCVKTCPAGVMGENNTLVWKYADAGHVCHLCHPNCTYGCTGPGLEGCPTNGLERIARLEEKVKTLKAQNSELASTANMLREQVAQLKQKVAAA

SEQ ID NO: 316 - protein, 372 aa, Artificial sequence
  synthetic polypeptide E010
MLLLVTSLLLCELPHPAFLLIPRKVCNGIGIGEFKDSLSINATNIKHFKNCTSISGDLHILPVAFRGDSFTHTPPLDPQELDILKTVKEITGFLLIQAWPENRTDLHAFENLEIIRGRTKQHGQFSLAVVSLNITSLGLRSLKEISDGDVIISGNKNLCYANTINWKKLFGTSGQKTKIISNRGENSCKATGQVCHALCSPEGCWGPEPRDCVSCRNVSRGRECVDKCNLLEGEPREFVENSECIQCHPECLPQAMNITCTGRGPDNCIQCAHYIDGPHCVKTCPAGVMGENNTLVWKYADAGHVCHLCHPNCTYGCTGPGLEGCPTNGLERIARLEEKVKTLKAQNSELASTANMLREQVAQLKQKVAAAA

SEQ ID NO: 317 - protein, 69 aa, Artificial sequence
  synthetic polypeptide E011
MTILGTTFGMVFSLLQVVSGEQKLISEEDLLERIARLEEKVKTLKAQNSELASTANMLREQVAQLKQKV

SEQ ID NO: 318 - protein, 70 aa, Artificial sequence
  synthetic polypeptide E012
MTILGTTFGMVFSLLQVVSGEQKLISEEDLLERIARLEEKVKTLKAQNSELASTANMLREQVAQLKQKVA

SEQ ID NO: 319 - protein, 71 aa, Artificial sequence
  synthetic polypeptide E013
MTILGTTFGMVFSLLQVVSGEQKLISEEDLLERIARLEEKVKTLKAQNSELASTANMLREQVAQLKQKVAA

SEQ ID NO: 320 - protein, 72 aa, Artificial sequence
  synthetic polypeptide E014
MTILGTTFGMVFSLLQVVSGEQKLISEEDLLERIARLEEKVKTLKAQNSELASTANMLREQVAQLKQKVAAA

SEQ ID NO: 321 - protein, 73 aa, Artificial sequence
  synthetic polypeptide E015
MTILGTTFGMVFSLLQVVSGEQKLISEEDLLERIARLEEKVKTLKAQNSELASTANMLREQVAQLKQKVAAAA

SEQ ID NO: 322 - protein, 23 aa, Artificial sequence
  synthetic polypeptide T001
LIIGICGGGSLLMVFVALLVFYI

SEQ ID NO: 323 - protein, 21 aa, Artificial sequence
  synthetic polypeptide T002
GIIVTDVIATLLLALGVFCFA

SEQ ID NO: 324 - protein, 26 aa, Artificial sequence
  synthetic polypeptide T003
VMSVATIVIVDICITGGLLLLVYYWS

SEQ ID NO: 325 - protein, 21 aa, Artificial sequence
  synthetic polypeptide T004
GFLFAEIVSIFVLAVGVYFIA

SEQ ID NO: 326 - protein, 21 aa, Artificial sequence
  synthetic polypeptide T005
LCYLLDGILFIYGVILTALFL

SEQ ID NO: 327 - protein, 22 aa, Artificial sequence
  synthetic polypeptide T006
MALIVLGGVAGLLLFIGLGIFF

SEQ ID NO: 328 - protein, 21 aa, Artificial sequence
  synthetic polypeptide T007
IYIWAPLAGTCGVLLLSLVIT

SEQ ID NO: 329 - protein, 23 aa, Artificial sequence
  synthetic polypeptide T008
LGLLVAGVLVLLVSLGVAIHLCC

SEQ ID NO: 330 - protein, 21 aa, Artificial sequence
  synthetic polypeptide T009
ILVIFSGMFLVFTLAGALFLH

SEQ ID NO: 331 - protein, 27 aa, Artificial sequence
  synthetic polypeptide T010
FWVLVVVGGVLACYSLLVTVAFIIFWV

SEQ ID NO: 332 - protein, 22 aa, Artificial sequence
  synthetic polypeptide T011
ALVVIPIIFGILFAILLVLVFI

SEQ ID NO: 333 - protein, 22 aa, Artificial sequence
  synthetic polypeptide T012
IITAEGIILLFCAVVPGTLLLF

SEQ ID NO: 334 - protein, 22 aa, Artificial sequence
  synthetic polypeptide T013
GIIMIQTLLIILFIIVPIFLLL

SEQ ID NO: 335 - protein, 21 aa, Artificial sequence
  synthetic polypeptide T014
FILISSLAILLMVSLLLLSLW

SEQ ID NO: 336 - protein, 21 aa, Artificial sequence
  synthetic polypeptide T015
CILISSLAILLMVSLLLLSLW

SEQ ID NO: 337 - protein, 26 aa, Artificial sequence
  synthetic polypeptide T016
NLGSVYIYVLLIVGTLVCGIVLGFLF

SEQ ID NO: 338 - protein, 19 aa, Artificial sequence
  synthetic polypeptide T017
MWVLALIVIFLTIAVLLAL

SEQ ID NO: 339 - protein, 19 aa, Artificial sequence
  synthetic polypeptide T018
MWVLALIEIFLTIAVLLAL

SEQ ID NO: 340 - protein, 23 aa, Artificial sequence
  synthetic polypeptide T019
IILGLFGLLLLLTCLCGTAWLCC

SEQ ID NO: 341 - protein, 23 aa, Artificial sequence
  synthetic polypeptide T020
IILGLFGLLLLLNCLCGTAWLCC

SEQ ID NO: 342 - protein, 23 aa, Artificial sequence
  synthetic polypeptide T021
LILTLSLILVVILVLLTVLALLS

SEQ ID NO: 343 - protein, 23 aa, Artificial sequence
  synthetic polypeptide T022
CCLTLSLILVVILVLLTVLALLS

SEQ ID NO: 344 - protein, 21 aa, Artificial sequence
  synthetic polypeptide T023
LCYILDAILFLYGIVLTLLYC

SEQ ID NO: 345 - protein, 23 aa, Artificial sequence
  synthetic polypeptide T024
IIVAVVTGIAVAAIVAAVVALIY

SEQ ID NO: 346 - protein, 23 aa, Artificial sequence
  synthetic polypeptide T025
IIVAVVIATAVAAIVAAVVALIY

SEQ ID NO: 347 - protein, 24 aa, Artificial sequence
  synthetic polypeptide T026
FPWLLIIIFGIFGLTVMLFVFLFS

SEQ ID NO: 348 - protein, 24 aa, Artificial sequence
  synthetic polypeptide T027
FPWLLCIIFGIFGLTVMLFVFLFS

SEQ ID NO: 349 - protein, 21 aa, Artificial sequence
  synthetic polypeptide T028
FWLPIGCAAFVVVCILGCILI

SEQ ID NO: 350 - protein, 21 aa, Artificial sequence
  synthetic polypeptide T029
IWLIVGICIALFALPFVIYAA

SEQ ID NO: 351 - protein, 21 aa, Artificial sequence
  synthetic polypeptide T030
IGGIITVFLIALVLTSTIVTL

SEQ ID NO: 352 - protein, 21 aa, Artificial sequence
  synthetic polypeptide T031
SLWIPVVAALLLFLVLSLVFI

SEQ ID NO: 353 - protein, 21 aa, Artificial sequence
  synthetic polypeptide T032
VILISVGTFSLLSVLAGACFF

SEQ ID NO: 354 - protein, 21 aa, Artificial sequence
  synthetic polypeptide T033
FLVLPSLLILLLVIAAGGVIW

SEQ ID NO: 355 - protein, 23 aa, Artificial sequence
  synthetic polypeptide T034
HMIGICVTLTVIIVCSVFIYKIF

SEQ ID NO: 356 - protein, 21 aa, Artificial sequence
  synthetic polypeptide T035
VLLVVILIVVYHVYWLEMVLF

SEQ ID NO: 357 - protein, 21 aa, Artificial sequence
  synthetic polypeptide T036
IYCIIAVCSVFLMLINVLVII

SEQ ID NO: 358 - protein, 21 aa, Artificial sequence
  synthetic polypeptide T037
AYLIGGLIALVAVAVSVVYIY

SEQ ID NO: 359 - protein, 19 aa, Artificial sequence
  synthetic polypeptide T038
VAVAGCVFLLISVLLLSGL

SEQ ID NO: 360 - protein, 25 aa, Artificial sequence
  synthetic polypeptide T039
IPWLGHLLVGLSGAFGFIILVYLLI

SEQ ID NO: 361 - protein, 21 aa, Artificial sequence
  synthetic polypeptide T040
VVISVGSMGLIISLLCVYFWL

SEQ ID NO: 362 - protein, 20 aa, Artificial sequence
  synthetic polypeptide T041
TSLLIALGTLLALVCVFVIC

SEQ ID NO: 363 - protein, 24 aa, Artificial sequence
  synthetic polypeptide T042
LLLGVSVSCIVILAVCLLCYVSIT

SEQ ID NO: 364 - protein, 20 aa, Artificial sequence
  synthetic polypeptide T043
FVIVIMATICFILLILSLIC

SEQ ID NO: 365 - protein, 21 aa, Artificial sequence
  synthetic polypeptide T044
TFLVAGGSLAFGTLLCIAIVL

SEQ ID NO: 366 - protein, 22 aa, Artificial sequence
  synthetic polypeptide T045
AIVVPVCLAFLLTTLLGVLFCF

SEQ ID NO: 367 - protein, 23 aa, Artificial sequence
  synthetic polypeptide T046
ILLTISILSFFSVALLVILACVL

SEQ ID NO: 368 - protein, 27 aa, Artificial sequence
  synthetic polypeptide T047
ILLPPCLTISILSFFSVALLVILACVL

SEQ ID NO: 369 - protein, 21 aa, Artificial sequence
  synthetic polypeptide T048
GNTLVAVSIFLLLTGPTYLLF

SEQ ID NO: 370 - protein, 21 aa, Artificial sequence
  synthetic polypeptide T049
VIIFFAFVLLLSGALAYCLAL

SEQ ID NO: 371 - protein, 22 aa, Artificial sequence
  synthetic polypeptide T050
WMVAVILMASVFMVCLALLGCF

SEQ ID NO: 372 - protein, 21 aa, Artificial sequence
  synthetic polypeptide T051
SLGILSFLGLVAGALALGLWL

SEQ ID NO: 373 - protein, 25 aa, Artificial sequence
  synthetic polypeptide T052
WLIFFASLGSFLSILLVGVLGYLGL

SEQ ID NO: 374 - protein, 21 aa, Artificial sequence
  synthetic polypeptide T053
WMAFVAPSICIAIIMVGIFST

SEQ ID NO: 375 - protein, 24 aa, Artificial sequence
  synthetic polypeptide T054
LYITMLLIVPVIVAGAIIVLLLYL

SEQ ID NO: 376 - protein, 20 aa, Artificial sequence
  synthetic polypeptide T055
FWLPFGFILILVIFVTGLLL

SEQ ID NO: 377 - protein, 23 aa, Artificial sequence
  synthetic polypeptide T056
VAISTSTVLLCGLSAVSLLACYL

SEQ ID NO: 378 - protein, 21 aa, Artificial sequence
  synthetic polypeptide T057
VYWFITGISILLVGSVILLIV

SEQ ID NO: 379 - protein, 21 aa, Artificial sequence
  synthetic polypeptide T058
LLLLSLLVATWVLVAGIYLMW

SEQ ID NO: 380 - protein, 21 aa, Artificial sequence
  synthetic polypeptide T059
WALVWLACLLFAAALSLILLL

SEQ ID NO: 381 - protein, 21 aa, Artificial sequence
  synthetic polypeptide T060
AVAITVPLVVISAFATLFTVM

SEQ ID NO: 382 - protein, 21 aa, Artificial sequence
  synthetic polypeptide T061
LGLLILALLALLTLLGVVLAL

SEQ ID NO: 383 - protein, 21 aa, Artificial sequence
  synthetic polypeptide T062
GMIIAVLILVAVVCLVTVCVI

SEQ ID NO: 384 - protein, 21 aa, Artificial sequence
  synthetic polypeptide T063
GVVLLYILLGTIGTLVAVLAA

SEQ ID NO: 385 - protein, 21 aa, Artificial sequence
  synthetic polypeptide T064
IIFWYVLPISITVFLFSVMGY

SEQ ID NO: 386 - protein, 21 aa, Artificial sequence
  synthetic polypeptide T065
VLALFAFVGFMLILVVVPLFV

SEQ ID NO: 387 - protein, 21 aa, Artificial sequence
  synthetic polypeptide T066
GWNPHLLLLLLLVIVFIPAFW

SEQ ID NO: 388 - protein, 21 aa, Artificial sequence
  synthetic polypeptide T067
YSFSGAFLFSMGFLVAVLCYL

SEQ ID NO: 389 - protein, 21 aa, Artificial sequence
  synthetic polypeptide T068
LLLGMIVFAVMLSILSLIGIF

SEQ ID NO: 390 - protein, 21 aa, Artificial sequence
  synthetic polypeptide T069
VLPGILFLWGLFLLGCGLSLA

SEQ ID NO: 391 - protein, 21 aa, Artificial sequence
  synthetic polypeptide T070
VLPGILCLWGLFLLGCGLSLA

SEQ ID NO: 392 - protein, 24 aa, Artificial sequence
  synthetic polypeptide T071
IILITSLIGGGLLILIILTVAYGL

SEQ ID NO: 393 - protein, 23 aa, Artificial sequence
  synthetic polypeptide T072
AGLYVIVPVIISSSILLLGTLLI

SEQ ID NO: 394 - protein, 25 aa, Artificial sequence
  synthetic polypeptide T073
VGLIIAILIPVAVAVIVGVVTSILC

SEQ ID NO: 395 - protein, 22 aa, Artificial sequence
  synthetic polypeptide T074
ISLVTALHLVLGLSAVLGLLLL

SEQ ID NO: 396 - protein, 22 aa, Artificial sequence
  synthetic polypeptide T075
ISLVTALHLVLGLNAVLGLLLL

SEQ ID NO: 397 - protein, 21 aa, Artificial sequence
  synthetic polypeptide T076
LIHILLPMVFCVLLIMVMCYL

SEQ ID NO: 398 - protein, 24 aa, Artificial sequence
  synthetic polypeptide T077
TTVWISVAVLSAVICLIIVWAVAL

SEQ ID NO: 399 - protein, 21 aa, Artificial sequence
  synthetic polypeptide T078
VAAILGLGLVLGLLGPLAILL

SEQ ID NO: 400 - protein, 28 aa, Artificial sequence
  synthetic polypeptide T079
PVLDAGPVLFWVILVLVVVVGSSAFLLC

SEQ ID NO: 401 - protein, 27 aa, Artificial sequence
  synthetic polypeptide T080
IISFFLALTSTALLFLLFFLTLRFSVV

SEQ ID NO: 402 - protein, 21 aa, Artificial sequence
  synthetic polypeptide T081
WWFLSGSLVIVIVCSTVGLII

SEQ ID NO: 403 - protein, 21 aa, Artificial sequence
  synthetic polypeptide T082
LGWLTVVLLAVAACVLLLTSA

SEQ ID NO: 404 - protein, 117 aa, Artificial sequence
  synthetic polypeptide S036
TKRKKQRSRRNDEELETRAHRVATEERGRKPHQIPASTPQNPATSQHPPPPPGHRSQAPSHRPPPPGHRVQHQPQKRPPAPSGTQVHQQKGPPLPRPRVQPKPPHGAAENSLSPSSN

SEQ ID NO: 405 - protein, 45 aa, Artificial sequence
  synthetic polypeptide S037
GHETGRLSGAADTQALLRNDQVYQPLRDRDDAQYSHLGGNWARNK

SEQ ID NO: 406 - protein, 55 aa, Artificial sequence
  synthetic polypeptide S038
KNRKAKAKPVTRGAGAGGRQRGQNKERPPPVPNPDYEPIRKGQRDLYSGLNQRRI

SEQ ID NO: 407 - protein, 45 aa, Artificial sequence
  synthetic polypeptide S039
GQDGVRQSRASDKQTLLPNDQLYQPLKDREDDQYSHLQGNQLRRN

SEQ ID NO: 408 - protein, 40 aa, Artificial sequence
  synthetic polypeptide S042
CVRCRHRRRQAERMSQIKRLLSEKKTCQCPHRFQKTCSPI

SEQ ID NO: 409 - protein, 32 aa, Artificial sequence
  synthetic polypeptide S043
LYCNHRNRRRVCKCPRPVVKSGDKPSLSARYV

SEQ ID NO: 410 - protein, 48 aa, Artificial sequence
  synthetic polypeptide S044
RRRRARLRFMKQPQGEGISGTFVPQCLHGYYSNTTTSQKLLNPWILKT

SEQ ID NO: 411 - protein, 26 aa, Artificial sequence
  synthetic polypeptide S045
RRRRARLRFMKQLRLHPLEKCSRMDY

SEQ ID NO: 412 - protein, 15 aa, Artificial sequence
  synthetic polypeptide S046
RRRRARLRFMKQFYK

SEQ ID NO: 413 - protein, 48 aa, Artificial sequence
  synthetic polypeptide S047
QRRKYRSNKGESPVEPAEPCRYSCPREEEGSTIPIQEDYRKPEPACSP

SEQ ID NO: 414 - protein, 41 aa, Artificial sequence; identical to SEQ ID NO: 3
  synthetic polypeptide S048

SEQ ID NO: 415 - protein, 41 aa, Artificial sequence; identical to SEQ ID NO: 2
  synthetic polypeptide S049

SEQ ID NO: 416 - protein, 62 aa, Artificial sequence
  synthetic polypeptide S050
KKVAKKPTNKAPHPKQEPQEINFPDDLPGSNTAAPVQETLHGCQPVTQEDGKESRISVQERQ

SEQ ID NO: 417 - protein, 66 aa, Artificial sequence
  synthetic polypeptide S051
SESSEKVAKKPTNKAPHPKQEPQEINFPDDLPGSNTAAPVQETLHGCQPVTQEDGKESRISVQERQ

SEQ ID NO: 418 - protein, 61 aa, Artificial sequence
  synthetic polypeptide S052
RKRWQNEKLGLDAGDEYEDENLYEGLNLDDCSMYEDISRGLQGTYQDVGSLNIGDVQLEKP

SEQ ID NO: 419 - protein, 49 aa, Artificial sequence
  synthetic polypeptide S053
LDKDDSKAGMEEDHTYEGLDIDQTATYEDIVTLRTGEVKWSVGEHPGQE

SEQ ID NO: 420 - protein, 119 aa, Artificial sequence
  synthetic polypeptide S054
KLWRVKKFLIPSVPDPKSIFPGLFEIHQGNFQEWITDTQNVAHLHKMAGAEQESGPEEPLVVQLAKTEAESPRMLDPQTEEKEASGGSLQLPHQPLQGGDVVTIGGFTFVMNDRSYVAL

SEQ ID NO: 421 - protein, 437 aa, Artificial sequence
  synthetic polypeptide S057
RFCGIYGYRLRRKWEEKIPNPSKSHLFQNGSAELWPPGSMSAFTSGSPPHQGPWGSRFPELEGVFPVGFGDSEVSPLTIEDPKHVCDPPSGPDTTPAASDLPTEQPPSPQPGPPAASHTPEKQASSFDFNGPYLGPPHSRSLPDILGQPEPPQEGGSQKSPPPGSLEYLCLPAGGQVQLVPLAQAMGPGQAVEVERRPSQGAAGSPSLESGGGPAPPALGPRVGGQDQKDSPVAIPMSSGDTEDPGVASGYVSSADLVFTPNSGASSVSLVPSLGLPSDQTPSLCPGLASGPPGAPGPVKSGFEGYVELPPIEGRSPRSPRNNPVPPEAKSPVLNPGERPADVSPTSPQPEGLLVLQQVGDYCFLPGLGPGPLSLRSKPSSPGPGPEIKNLDQAFQVKKPPGQAVPQVPVIQLFKALKQQDYLSLPPWEVNKPGEVC

SEQ ID NO: 422 - protein, 54 aa, Artificial sequence
  synthetic polypeptide S058
KRFLRIQRLFPPVPQIKDKLNDNHEVEDEIIWEEFTPEEGKGYREEVLTVKEIT

SEQ ID NO: 423 - protein, 64 aa, Artificial sequence
  synthetic polypeptide S059
KRFLRIQRLFPPVPQIKDKLNDNHEVEDEMGPQRHHRCGWNLYPTPGPSPGSGSSPRLGSESSL

SEQ ID NO: 424 - protein, 186 aa, Artificial sequence
  synthetic polypeptide S062
SPNRKNPLWPSVPDPAHSSLGSWVPTIMEEDAFQLPGLGTPPITKLTVLEEDEKKPVPWESHNSSETCGLPTLVQTYVLQGDPRAVSTQPQSQSGTSDQVLYGQLLGSPTSPGPGHYLRCDSTQPLLAGLTPSPKSYENLWFQASPLGTLVTPAPSQEDDCVFGPLLNFPLLQGIRVHGMEALGSF

SEQ ID NO: 425 - protein, 213 aa, Artificial sequence
  synthetic polypeptide S063
SPNRKNPLWPSVPDPAHSSLGSWVPTIMEELPGPRQGQWLGQTSEMSRALTPHPCVQDAFQLPGLGTPPITKLTVLEEDEKKPVPWESHNSSETCGLPTLVQTYVLQGDPRAVSTQPQSQSGTSDQVLYGQLLGSPTSPGPGHYLRCDSTQPLLAGLTPSPKSYENLWFQASPLGTLVTPAPSQEDDCVFGPLLNFPLLQGIRVHGMEALGSF

SEQ ID NO: 426 - protein, 133 aa, Artificial sequence
  synthetic polypeptide S064
SPNRKNPLWPSVPDPAHSSLGSWVPTIMEEDAFQLPGLGTPPITKLTVLEEDEKKPVPWESHNSSETCGLPTLVQTYVLQGDPRAVSTQPQSQSGTSDQAGPPRRSAYFKDQIMLHPAPPNGLLCLFPITSVL

SEQ ID NO: 427 - protein, 235 aa, Artificial sequence
  synthetic polypeptide S069
HRRALKQKIWPGIPSPESEFEGLFTTHKGNFQLWLYQNDGCLWWSPCTPFTEDPPASLEVLSERCWGTMQAVEPGTDDEGPLLEPVGSEHAQDTYLVLDKWLLPRNPPSEDLPGPGGSVDIVAMDEGSEASSCSSALASKPSPEGASAASFEYTILDPSSQLLRPWTLCPELPPTPPHLKYLYLVVSDSGISTDYSSGDSQGAQGGLSDGPYSNPYENSLIPAAEPLPPSYVACS

SEQ ID NO: 428 - protein, 235 aa, Artificial sequence
  synthetic polypeptide S072
HRRALKQKIWPGIPSPESEFEGLFTTHKGNFQLWLYQNDGCLWWSPCTPFTEDPPASLEVLSERCWGTMQAVEPGTDDEGPLLEPVGSEHAQDTYLVLDKWLLPRNPPSEDLPGPGGSVDIVAMDEGSEASSCSSALASKPSPEGASAASFEYTILDPSSQLLRPWTLCPELPPTPPHLKFLFLVVSDSGISTDYSSGDSQGAQGGLSDGPYSNPYENSLIPAAEPLPPSYVACS

SEQ ID NO: 429 - protein, 42 aa, Artificial sequence
  synthetic polypeptide S074
RLKIQVRKAAITSYEKSDGVYTGLSTRNQETYETLKHEKPPQ

SEQ ID NO: 430 - protein, 77 aa, Artificial sequence
  synthetic polypeptide S075
CRKKRISANSTDPVKAAQFEPPGRQMIAIRKRQPEETNNDYETADGGYMTLNPRAPTDDDKNIYLTLPPNDHVNSNN

SEQ ID NO: 431 - protein, 77 aa, Artificial sequence
  synthetic polypeptide S076
CRKKRISANSTDPVKAAQFEPPGRQMIAIRKRQLEETNNDYETADGGYMTLNPRAPTDDDKNIYLTLPPNDHVNSNN

SEQ ID NO: 432 - protein, 350 aa, Artificial sequence
  synthetic polypeptide S077
KQQRIKMLILPPVPVPKIKGIDPDLLKEGKLEEVNTILAIHDSYKPEFHSDDSWVEFIELDIDEPDEKTEESDTDRLLSSDHEKSHSNLGVKDGDSGRTSCCEPDILETDFNANDIHEGTSEVAQPQRLKGEADLLCLDQKNQNNSPYHDACPATQQPSVIQAEKNKPQPLPTEGAESTHQAAHIQLSNPSSLSNIDFYAQVSDITPAGSVVLSPGQKNKAGMSQCDMHPEMVSLCQENFLMDNAYFCEADAKKCIPVAPHIKVESHIQPSLNQEDIYITTESLTTAAGRPGTGEHVPGSEMPVPDYTSIHIVQSPQGLILNATALPLPDKEFLSSCGYVSTDQLNKIMP

SEQ ID NO: 433 - protein, 38 aa, Artificial sequence
  synthetic polypeptide S080
CWLTKKKYSSSVHDPNGEYMFMRAVNTAKKSRLTDVTL

SEQ ID NO: 434 - protein, 100 aa, Artificial sequence
  synthetic polypeptide S081
KVFLRCINYVFFPSLKPSSSIDEYFSEQPLKNLLLSTSEEQIEKCFIIENISTIATVEETNQTDEDHKKYSSQTSQDSGNYSNEDESESKTSEELQQDFV

SEQ ID NO: 435 - protein, 251 aa, Artificial sequence
  synthetic polypeptide S082
KWIGYICLRNSLPKVLNFHNFLAWPFPNLPPLEAMDMVEVIYINRKKKVWDYNYDDESDSDTEAAPRTSGGGYTMHGLTVRPLGQASATSTESQLIDPESEEEPDLPEVDVELPTMPKDSPQQLELLSGPCERRKSPLQDPFPEEDYSSTEGSGGRITFNVDLNSVFLRVLDDEDSDDLEAPLMLSSHLEEMVDPEDPDNVQSNHLLASGEGTQPTFPSPSSEGLWSEDAPSDQSDTSESDVDLGDGYIMR

SEQ ID NO: 436 - protein, 67 aa, Artificial sequence
  synthetic polypeptide S083
KWIGYICLRNSLPKVLRQGLAKGWNAVAIHRCSHNALQSETPELKQSSCLSFPSSWDYKRASLCPSD

SEQ ID NO: 437 - protein, 223 aa, Artificial sequence
  synthetic polypeptide S084
CFYIKKINPLKEKSIILPKSLISVVRSATLETKPESKYVSLITSYQPFSLEKEVVCEEPLSPATVPGMHTEDNPGKVEHTEELSSITEVVTTEENIPDVVPGSHLTPIERESSSPLSSNQSEPGSIALNSYHSRNCSESDHSRNGFDTDSSCLESHSSLSDSEFPPNNKGEIKTEGQELITVIKAPTSFGYDKPHVLVDLLVDDSGKESLIGYRPTEDSKEFS

SEQ ID NO: 438 - protein, 69 aa, Artificial sequence
  synthetic polypeptide S085
LVLKYRGLIKYWFHTPPSIPLQIEEYLKDPTQPILEALDKDSSPKDDVWDSVSIISFPEKEQEDVLQTL

SEQ ID NO: 439 - protein, 271 aa, Artificial sequence
  synthetic polypeptide S086
KTLMGNPWFQRAKMPRALDFSGHTHPVATFQPSRPESVNDLFLCPQKELTRGVRPTPRVRAPATQQTRWKKDLAEDEEEEDEEDTEDGVSFQPYIEPPSFLGQEHQAPGHSEAGGVDSGRPRAPLVPSEGSSAWDSSDRSWASTVDSSWDRAGSSGYLAEKGPGQGPGGDGHQESLPPPEFSKDSGFLEELPEDNLSSWATWGTLPPEPNLVPGGPPVSLQTLTFCWESSPEEEEEARESEIEDSDAGSWGAESTQRTEDRGRTLGHYMAR

SEQ ID NO: 440 - protein, 242 aa, Artificial sequence
  synthetic polypeptide S087
KTLMGNPWFQRAKMPRALELTRGVRPTPRVRAPATQQTRWKKDLAEDEEEEDEEDTEDGVSFQPYIEPPSFLGQEHQAPGHSEAGGVDSGRPRAPLVPSEGSSAWDSSDRSWASTVDSSWDRAGSSGYLAEKGPGQGPGGDGHQESLPPPEFSKDSGFLEELPEDNLSSWATWGTLPPEPNLVPGGPPVSLQTLTFCWESSPEEEEEARESEIEDSDAGSWGAESTQRTEDRGRTLGHYMAR

SEQ ID NO: 441 - protein, 179 aa, Artificial sequence
  synthetic polypeptide S098
KIDIVLWYRDSCYDFLPIKVLPEVLEKQCGYKLFIYGRDDYVGEDIVEVINENVKKSRRLIIILVRETSGFSWLGGSSEEQIAMYNALVQDGIKVVLLELEKIQDYEKMPESIKFIKQKHGAIRWSGDFTQGPQSAKTRFWKNVRYHMPVQRRSPSSKHQLLSPATKEKLQREAHVPLG

SEQ ID NO: 442 - protein, 210 aa, Artificial sequence
  synthetic polypeptide S099
KIDIVLWYRDSCYDFLPIKASDGKTYDAYILYPKTVGEGSTSDCDIFVFKVLPEVLEKQCGYKLFIYGRDDYVGEDIVEVINENVKKSRRLIIILVRETSGFSWLGGSSEEQIAMYNALVQDGIKVVLLELEKIQDYEKMPESIKFIKQKHGAIRWSGDFTQGPQSAKTRFWKNVRYHMPVQRRSPSSKHQLLSPATKEKLQREAHVPLG

SEQ ID NO: 443 - protein, 182 aa, Artificial sequence
  synthetic polypeptide S100
YRAHFGTDETILDGKEYDIYVSYARNAEEEEFVLLTLRGVLENEFGYKLCIFDRDSLPGGIVTDETLSFIQKSRRLLVVLSPNYVLQGTQALLELKAGLENMASRGNINVILVQYKAVKETKVKELKRAKTVLTVIKWKGEKSKYPQGRFWKQLQVAMPVKKSPRRSSSDEQGLSYSSLKNV

SEQ ID NO: 444 - protein, 299 aa, Artificial sequence
  synthetic polypeptide S101
YRAHFGTDETILDGKEYDIYVSYARNAEEEEFVLLTLRGVLENEFGYKLCIFDRDSLPGGNTVEAVFDFIQRSRRMIVVLSPDYVTEKSISMLEFKLGVMCQNSIATKLIVVEYRPLEHPHPGILQLKESVSFVSWKGEKSKHSGSKFWKALRLALPLRSLSASSGWNESCSSQSDISLDHVQRRRSRLKEPPELQSSERAAGSPPAPGTMSKHRGKSSATCRCCVTYCEGENHLRNKSRAEIHNQPQWETHLCKPVPQESETQWIQNGTRLEPPAPQISALALHHFTDLSNNNDFYIL

SEQ ID NO: 445 - protein, 207 aa, Artificial sequence
  synthetic polypeptide S102
LKMFWIEATLLWRDIAKPYKTRNDGKLYDAYVVYPRNYKSSTDGASRVEHFVHQILPDVLENKCGYTLCIYGRDMLPGEDVVTAVETNIRKSRRHIFILTPQITHNKEFAYEQEVALHCALIQNDAKVILIEMEALSELDMLQAEALQDSLQHLMKVQGTIKWREDHIANKRSLNSKFWKHVRYQMPVPSKIPRKASSLTPLAAQKQ

SEQ ID NO: 446 - protein, 219 aa, Artificial sequence
  synthetic polypeptide S103
NIFKIDIVLWYRSAFHSTETIVDGKLYDAYVLYPKPHKESQRHAVDALVLNILPEVLERQCGYKLFIFGRDEFPGQAVANVIDENVKLCRRLIVIVVPESLGFGLLKNLSEEQIAVYSALIQDGMKVILIELEKIEDYTVMPESIQYIKQKHGAIRWHGDFTEQSQCMKTKFWKTVRYHMPPRRCRPFPPVQLLQHTPCYRTAGPELGSRRKKCTLTTG

SEQ ID NO: 447 - protein, 13 aa, Artificial sequence
  synthetic polypeptide S104
TWQRRQRKSRRTI

SEQ ID NO: 448 - protein, 286 aa, Artificial sequence
  synthetic polypeptide S105
NCRNTGPWLKKVLKCNTPDPSKFFSQLSSEHGGDVQKWLSSPFPSSSFSPGGLAPEISPLEVLERDKVTQLLLQQDKVPEPASLSSNHSLTSCFTNQGYFFFHLPDALEIEACQVYFTYDPYSEEDPDEGVAGAPTGSSPQPLQPLSGEDDAYCTFPSRDDLLLFSPSLLGGPSPPSTAPGGSGAGEERMPPSLQERVPRDWDPQPLGPPTPGVPDLVDFQPPPELVLREAGEEVPDAGPREGVSFPWSRPPGQGEFRALNARLPLNTDAYLSLQELQGQDPTHLV

SEQ ID NO: 449 - protein, 86 aa, Artificial sequence
  synthetic polypeptide S106
ERTMPRIPTLKNLEDLVTEYHGNFSAWSGVSKGLAESLQPDYSERLCLVSEIPPKGGALGEGPGASPCNQHSPYWAPPCYTLKPET

SEQ ID NO: 450 - protein, 53 aa, Artificial sequence
  synthetic polypeptide S109
RRYLVMQRLFPRIPHMKDPIGDSFQNDKLVVWEAGKAGLEECLVTEVQVVQKT

SEQ ID NO: 451 - protein, 569 aa, Artificial sequence
  synthetic polypeptide S110
KIKKEWWDQIPNPARSRLVAIIIQDAQGSQWEKRSRGQEPAKCPHWKNCLTKLLPCFLEHNMKRDEDPHKAAKEMPFQGSGKSAWCPVEISKTVLWPESISVVRCVELFEAPVECEEEEEVEEEKGSFCASPESSRDDFQEGREGIVARLTESLFLDLLGEENGGFCQQDMGESCLLPPSGSTSAHMPWDEFPSAGPKEAPPWGKEQPLHLEPSPPASPTQSPDNLTCTETPLVIAGNPAYRSFSNSLSQSPCPRELGPDPLLARHLEEVEPEMPCVPQLSEPTTVPQPEPETWEQILRRNVLQHGAAAAPVSAPTSGYQEFVHAVEQGGTQASAVVGLGPPGEAGYKAFSSLLASSAVSPEKCGFGASSGEEGYKPFQDLIPGCPGDPAPVPVPLFTFGLDREPPRSPQSSHLPSSSPEHLGLEPGEKVEDMPKPPLPQEQATDPLVDSLGSGIVYSALTCHLCGHLKQCHGQEDGGQTPVMASPCCGCCCGDRSSPPTTPLRAPDPSPGGVPLEASLCPASLAPSGISEKSKSSSSFHPAPGNAQSSSQTPKIVNFVSVGPTYMRVS

SEQ ID NO: 452 - protein, 569 aa, Artificial sequence
  synthetic polypeptide S113
KIKKEWWDQIPNPARSRLVAIIIQDAQGSQWEKRSRGQEPAKCPHWKNCLTKLLPCFLEHNMKRDEDPHKAAKEMPFQGSGKSAWCPVEISKTVLWPESISVVRCVELFEAPVECEEEEEVEEEKGSFCASPESSRDDFQEGREGIVARLTESLFLDLLGEENGGFCQQDMGESCLLPPSGSTSAHMPWDEFPSAGPKEAPPWGKEQPLHLEPSPPASPTQSPDNLTCTETPLVIAGNPAYRSFSNSLSQSPCPRELGPDPLLARHLEEVEPEMPCVPQLSEPTTVPQPEPETWEQILRRNVLQHGAAAAPVSAPTSGYQEFVHAVEQGGTQASAVVGLGPPGEAGYKAFSSLLASSAVSPEKCGFGASSGEEGYKPFQDLIPGCPGDPAPVPVPLFTFGLDREPPRSPQSSHLPSSSPEHLGLEPGEKVEDMPKPPLPQEQATDPLVDSLGSGIVFSALTCHLCGHLKQCHGQEDGGQTPVMASPCCGCCCGDRSSPPTTPLRAPDPSPGGVPLEASLCPASLAPSGISEKSKSSSSFHPAPGNAQSSSQTPKIVNFVSVGPTYMRVS

SEQ ID NO: 453 - protein, 58 aa, Artificial sequence
  synthetic polypeptide S115
KICHLWIKLFPPIPAPKSNIKDLFVTTNYEKAGSSETEIEVICYIEKPGVETLEDSVF

SEQ ID NO: 454 - protein, 82 aa, Artificial sequence
  synthetic polypeptide S116
RFKKTWKLRALKEGKTSMHPPYSLGQLVPERPRPTPVLVPLISPPVSPSSLGSDNTSSHNRPDARDPRSPYDISNTDYFFPR

SEQ ID NO: 455 - protein, 277 aa, Artificial sequence
  synthetic polypeptide S117
NKRDLIKKHIWPNVPDPSKSHIAQWSPHTPPRHNFNSKDQMYSDGNFTDVSVVEIEANDKKPFPEDLKSLDLFKKEKINTEGHSSGIGGSSCMSSSRPSISSSDENESSQNTSSTVQYSTVVHSGYRHQVPSVQVFSRSESTQPLLDSEERPEDLQLVDHVDGGDGILPRQQYFKQNCSQHESSPDISHFERSKQVSSVNEEDFVRLKQQISDHISQSCGSGQMKMFQEVSAADAFGPGTEGQVERFETVGMEAATDEGMPKSYLPQTVRQGGYMPQ

SEQ ID NO: 456 - protein, 196 aa, Artificial sequence
  synthetic polypeptide S120
WKKRIKPIVWPSLPDHKKTLEHLCKKPRKNLNVSFNPESFLDCQIHRVDDIQARDEVEGFLQDTFPQQLEESEKQRLGGDVQSPNCPSEDVVITPESFGRDSSLTCLAGNVSACDAPILSSSRSLDCRESGKNGPHVYQDLLLSLGTTNSTLPPPFSLQSGILTLNPVAQGQPILTSLGSNQEEAYVTMSSFYQNQ

SEQ ID NO: 457 - protein, 35 aa, Artificial sequence
  synthetic polypeptide S121
WKKRIKPIVWPSLPDHKKTLEHLCKKPRKVSVFGA

SEQ ID NO: 458 - protein, 230 aa, Artificial sequence
  synthetic polypeptide S126
KLSPRVKRIFYQNVPSPAMFFQPLYSVHNGNFQTWMGAHGAGVLLSQDCAGTPQGALEPCVQEATALLTCGPARPWKSVALEEEQEGPGTRLPGNLSSEDVLPAGCTEWRVQTLAYLPQEDWAPTSLTRPAPPDSEGSRSSSSSSSSNNNNYCALGCYGGWHLSALPGNTQSSGPIPALACGLSCDHQGLETQQGVAWVLAGHCQRPGLHEDLQGMLLPSVLSKARSWTF

SEQ ID NO: 459 - protein, 322 aa, Artificial sequence
  synthetic polypeptide S129
QLYVRRRKKLPSVLLFKKPSPFIFISQRPSPETQDTIHPLDEEAFLKVSPELKNLDLHGSTDSGFGSTKPSLQTEEPQFLLPDPHPQADRTLGNREPPVLGDSCSSGSSNSTDSGICLQEPSLSPSTGPTWEQQVGSNSRGQDDSGIDLVQNSEGRAGDTQGGSALGHHSPPEPEVPGEEDPAAVAFQGYLRQTRCAEEKATKTGCLEEESPLTDGLGPKFGRCLVDEAGLHPPALAKGYLKQDPLEMTLASSGAPTGQWNQPTEEWSLLALSSCSDLGISDWSFAHDLAPLGCVAAPGGLLGSFNSDLVTLPLISSLQSSE

SEQ ID NO: 460 - protein, 83 aa, Artificial sequence
  synthetic polypeptide S130
ALLWCVYKKTKYAFSPRNSLPQHLKEFLGHPHHNTLLFFSFPLSDENDVFDKLSVIAEDSESGKQNPGDSCSLGTPPGQGPQS

SEQ ID NO: 461 - protein, 31 aa, Artificial sequence
  synthetic polypeptide S135
RLRRGGKDGSPKPGFLASVIPVDRRPGAPNL

SEQ ID NO: 462 - protein, 92 aa, Artificial sequence
  synthetic polypeptide S136
NRAARHLCPPLPTPCASSAIEFPGGKETWQWINPVDFQEEASLQEALVVEMSWDKGERTEPLEKTELPEGAPELALDTELSLEDGDRCKAKM

SEQ ID NO: 463 - protein, 90 aa, Artificial sequence
  synthetic polypeptide S137
NRAARHLCPPLPTPCASSAIEFPGGKETWQWINPVDFQEEASLQEALVVEMSWDKGERTEPLEKTELPEGAPELALDTELSLEDGDRCDR

SEQ ID NO: 464 - protein, 219 aa, Artificial sequence
  synthetic polypeptide S138
HYFQQKVFVLLAALRPQWCSREIPDPANSTCAKKYPIAEEKTQLPLDRLLIDWPTPEDPEPLVISEVLHQVTPVFRHPPCSNWPQREKGIQGHQASEKDMMHSASSPPPPRALQAESRQLVDLYKVLESRGSDPKPENPACPWTVLPAGDLPTHDGYLPSNIDDLPSHEAPLADSLEELEPQHISLSVFPSSSLHPLTFSCGDKLTLDQLKMRCDSLML

SEQ ID NO: 465 - protein, 60 aa, Artificial sequence
  synthetic polypeptide S141
KRLKIIIFPPIPDPGKIFKEMFGDQNDDTLHWKKYDIYEKQTKEETDSVVLIENLKKASQ

SEQ ID NO: 466 - protein, 17 aa, Artificial sequence
  synthetic polypeptide S142
RKPNTYPKMIPEFFCDT

SEQ ID NO: 467 - protein, 39 aa, Artificial sequence
  synthetic polypeptide S143
KSRQTPPLASVEMEAMEALPVTWGTSSRDEDLENCSHHL

SEQ ID NO: 468 - protein, 525 aa, Artificial sequence
  synthetic polypeptide S144
CMTWRLAGPGSEKYSDDTKYTDGLPAADLIPPPLKPRKVWIIYSADHPLYVDVVLKFAQFLLTACGTEVALDLLEEQAISEAGVMTWVGRQKQEMVESNSKIIVLCSRGTRAKWQALLGRGAPVRLRCDHGKPVGDLFTAAMNMILPDFKRPACFGTYVVCYFSEVSCDGDVPDLFGAAPRYPLMDRFEEVYFRIQDLEMFQPGRMHRVGELSGDNYLRSPGGRQLRAALDRFRDWQVRCPDWFECENLYSADDQDAPSLDEEVFEEPLLPPGTGIVKRAPLVREPGSQACLAIDPLVGEEGGAAVAKLEPHLQPRGQPAPQPLHTLVLAAEEGALVAAVEPGPLADGAAVRLALAGEGEACPLLGSPGAGRNSVLFLPVDPEDSPLGSSTPMASPDLLPEDVREHLEGLMLSLFEQSLSCQAQGGCSRPAMVLTDPHTPYEEEQRQSVQSDQGYISRSSPQPPEGLTEMEEEEEEEQDPGKPALPLSPEDLESLRSLQRQLLFRQLQKNSGWDTMGSESEGPSA

SEQ ID NO: 469 - protein, 189 aa, Artificial sequence
  synthetic polypeptide S145
RHERIKKTSFSTTTLLPPIKVLVVYPSEICFHHTICYFTEFLQNHCRSEVILEKWQKKKIAEMGPVQWLATQKKAADKVVFLLSNDVNSVCDGTCGKSEGSPSENSQDLFPLAFNLFCSDLRSQIHLHKYVVVYFREIDTKDDYNALSVCPKYHLMKDATAFCAELLHVKQQVSAGKRSQACHDGCCSL

SEQ ID NO: 470 - protein, 232 aa, Artificial sequence
  synthetic polypeptide S146
KKDHAKGWLRLLKQDVRSGAAARGRAALLLYSADDSGFERLVGALASALCQLPLRVAVDLWSRRELSAQGPVAWFHAQRRQTLQEGGVVVLLFSPGAVALCSEWLQDGVSGPGAHGPHDAFRASLSCVLPDFLQGRAPGSYVGACFDRLLHPDAVPALFRTVPVFTLPSQLPDFLGALQQPRAPRSGRLQERAEQVSRALQPALDSYFHPPGTPAPGRGVGPGAGPGAGDGT

SEQ ID NO: 471 - protein, 219 aa, Artificial sequence
  synthetic polypeptide S147
KKDHAKAAARGRAALLLYSADDSGFERLVGALASALCQLPLRVAVDLWSRRELSAQGPVAWFHAQRRQTLQEGGVVVLLFSPGAVALCSEWLQDGVSGPGAHGPHDAFRASLSCVLPDFLQGRAPGSYVGACFDRLLHPDAVPALFRTVPVFTLPSQLPDFLGALQQPRAPRSGRLQERAEQVSRALQPALDSYFHPPGTPAPGRGVGPGAGPGAGDGT

SEQ ID NO: 472 - protein, 419 aa, Artificial sequence
  synthetic polypeptide S148
CRKKQQENIYSHLDEESSESSTYTAALPRERLRPRPKVFLCYSSKDGQNHMNVVQCFAYFLQDFCGCEVALDLWEDFSLCREGQREWVIQKIHESQFIIVVCSKGMKYFVDKKNYKHKGGGRGSGKGELFLVAVSAIAEKLRQAKQSSSAALSKFIAVYFDYSCEGDVPGILDLSTKYRLMDNLPQLCSHLHSRDHGLQEPGQHTRQGSRRNYFRSKSGRSLYVAICNMHQFIDEEPDWFEKQFVPFHPPPLRYREPVLEKFDSGLVLNDVMCKPGPESDFCLKVEAAVLGATGPADSQHESQHGGLDQDGEARPALDGSAALQPLLHTVKAGSPSDMPRDSGIYDSSVPSSELSLPLMEGLSTDQTETSSLTESVSSSSGLGEEEPPALPSKLLSSGSCKADLGCRSYTDELHAVAPL

SEQ ID NO: 473 - protein, 192 aa, Artificial sequence
  synthetic polypeptide S149
TCRRPQSGPGPARPVLLLHAADSEAQRRLVGALAELLRAALGGGRDVIVDLWEGRHVARVGPLPWLWAARTRVAREQGTVLLLWSGADLRPVSGPDPRAAPLLALLHAAPRPLLLLAYFSRLCAKGDIPPPLRALPRYRLLRDLPRLLRALDARPFAEATSWGRLGARQRRQSRLELCSRLEREAARLADLG

SEQ ID NO: 474 - protein, 191 aa, Artificial sequence
  synthetic polypeptide S154
YRVDLVLFYRHLTRRDETLTDGKTYDAFVSYLKECRPENGEEHTFAVEILPRVLEKHFGYKLCIFERDVVPGGAVVDEIHSLIEKSRRLIIVLSKSYMSNEVRYELESGLHEALVERKIKIILIEFTPVTDFTFLPQSLKLLKSHRVLKWKADKSLSYNSRFWKNLLYLMPAKTVKPGRDEPEVLPVLSES

SEQ ID NO: 475 - protein, 222 aa, Artificial sequence
  synthetic polypeptide S155
SALLYRHWIEIVLLYRTYQSKDQTLGDKKDFDAFVSYAKWSSFPSEATSSLSEEHLALSLFPDVLENKYGYSLCLLERDVAPGGVYAEDIVSIIKRSRRGIFILSPNYVNGPSIFELQAAVNLALDDQTLKLILIKFCYFQEPESLPHLVKKALRVLPTVTWRGLKSVPPNSRFWAKMRYHMPVKNSQGFTWNQLRITSRIFQWKGLSRTETTGRSSQPKEW

SEQ ID NO: 476 - protein, 282 aa, Artificial sequence
  synthetic polypeptide S156
SIYRYIHVGKEKHPANLILIYGNEFDKRFFVPAEKIVINFITLNISDDSKISHQDMSLLGKSSDVSSLNDPQPSGNLRPPQEEEEVKHLGYASHLMEIFCDSEENTEGTSLTQQESLSRTIPPDKTVIEYEYDVRTTDICAGPEEQELSLQEEVSTQGTLLESQAALAVLGPQTLQYSYTPQLQDLDPLAQEHTDSEEGPEEEPSTTLVDWDPQTGRLCIPSLSSFDQDSEGCEPSEGDGLGEEGLLSRLYEEPAPDRPPGENETYLMQFMEEWGLYVQMEN

SEQ ID NO: 477 - protein, 57 aa, Artificial sequence
  synthetic polypeptide S157
WKMGRLLQYSCCPVVVLPDTLKITNSPQKLISCRREEVDACATAVMSPEELLRAWIS

SEQ ID NO: 478 - protein, 285 aa, Artificial sequence
  synthetic polypeptide S158
SLKTHPLWRLWKKIWAVPSPERFFMPLYKGCSGDFKKWVGAPFTGSSLELGPWSPEVPSTLEVYSCHPPRSPAKRLQLTELQEPAELVESDGVPKPSFWPTAQNSGGSAYSEERDRPYGLVSIDTVTVLDAEGPCTWPCSCEDDGYPALDLDAGLEPSPGLEDPLLDAGTTVLSCGCVSAGSPGLGGPLGSLLDRLKPPLADGEDWAGGLPWGGRSPGGVSESEAGSPLAGLDMDTFDSGFVGSDCSSPVECDFTSPGDEGPPRSYLRQWVVIPPPLSSPGPQAS

SEQ ID NO: 479 - protein, 325 aa, Artificial sequence
  synthetic polypeptide S161
SYRYVTKPPAPPNSLNVQRVLTFQPLRFIQEHVLIPVFDLSGPSSLAQPVQYSQIRVSGPREPAGAPQRHSLSEITYLGQPDISILQPSNVPPPQILSPLSYAPNAAPEVGPPSYAPQVTPEAQFPFYAPQAISKVQPSSYAPQATPDSWPPSYGVCMEGSGKDSPTGTLSSPKHLRPKGQLQKEPPAGSCMLGGLSLQEVTSLAMEESQEAKSLHQPLGICTDRTSDPNVLHSGEEGTPQYLKGQLPLLSSVQIEGHPMSLPLQPPSRPCSPSDQGPSPWGLLESLVCPKDEAKSPAPETSDLEQPTELDSLFRGLALTVQWES

SEQ ID NO: 480 - protein, 253 aa, Artificial sequence
  synthetic polypeptide S165
NRSFRTGIKRRILLLIPKWLYEDIPNMKNSNVVKMLQENSELMNNNSSEQVLYVDPMITEIKEIFIPEHKPTDYKKENTGPLETRDYPQNSLFDNTTVVYIPDLNTGYKPQISNFLPEGSHLSNNNEITSLTLKPPVDSLDSGNNPRLQKHPNFAFSVSSVNSLSNTIFLGELSLILNQGECSSPDIQNSVEEETTMLLENDSPSETIPEQTLLPDEFVSCLGIVNEELPSINTYFPQNILESHFNRISLLEK

SEQ ID NO: 481 - protein, 99 aa, Artificial sequence
  synthetic polypeptide S168
TSGRCYHLRHKVLPRWVWEKVPDPANSSSGQPHMEQVPEAQPLGDLPILEVEEMEPPPVMESSQPAQATAPLDSGYEKHFLPTPEELGLLGPPRPQVLA

SEQ ID NO: 482 - protein, 86 aa, Artificial sequence
  synthetic polypeptide S169
TSWVWEKVPDPANSSSGQPHMEQVPEAQPLGDLPILEVEEMEPPPVMESSQPAQATAPLDSGYEKHFLPTPEELGLLGPPRPQVLA

SEQ ID NO: 483 - protein, 189 aa, Artificial sequence
  synthetic polypeptide S170
KKPNKLTHLCWPTVPNPAESSIATWHGDDFKDKLNLKESDDSVNTEDRILKPCSTPSDKLVIDKLVVNFGNVLQEIFTDEARTGQENNLGGEKNGYVTCPFRPDCPLGKSFEELPVSPEIPPRKSQYLRSRMPEGTRPEAKEQLLFSGQSLVPDHLCEEGAPNPYLKNSVTAREFLVSEKLPEHTKGEV

SEQ ID NO: 484 - protein, 106 aa, Artificial sequence
  synthetic polypeptide S171
KKPNKLTHLCWPTVPNPAESSIATWHGDDFKDKLNLKESDDSVNTEDRILKPCSTPSDKLVIDKLVVNFGNVLQEIFTDEARTGQENNLGGEKNGTRILSSCPTSI

SEQ ID NO: 485 - protein, 303 aa, Artificial sequence
  synthetic polypeptide S174
SHQRMKKLFWEDVPNPKNCSWAQGLNFQKPETFEHLFIKHTASVTCGPLLLEPETISEDISVDTSWKNKDEMMPTTVVSLLSTTDLEKGSVCISDQFNSVNFSEAEGTEVTYEDESQRQPFVKYATLISNSKPSETGEEQGLINSSVTKCFSSKNSPLKDSFSNSSWEIEAQAFFILSDQHPNIISPHLTFSEGLDELLKLEGNFPEENNDKKSIYYLGVTSIKKRESGVLLTDKSRVSCPFPAPCLFTDIRVLQDSCSHFVENNINLGTSSKKTFASYMPQFQTCSTQTHKIMENKMCDLTV

SEQ ID NO: 486 - protein, 96 aa, Artificial sequence
  synthetic polypeptide S175
SHQRMKKLFWEDVPNPKNCSWAQGLNFQKMLEGSMFVKSHHHSLISSTQGHKHCGRPQGPLHRKTRDLCSLVYLLTLPPLLSYDPAKSPSVRNTQE

SEQ ID NO: 487 - protein, 34 aa, Artificial sequence
  synthetic polypeptide S176
SHQRMKKLFWEDVPNPKNCSWAQGLNFQKRTDIL

SEQ ID NO: 488 - protein, 44 aa, Artificial sequence
  synthetic polypeptide S177
SHQRMKKLFWEDVPNPKNCSWAQGLNFQKKMPGTKELLGGGWLT

SEQ ID NO: 489 - protein, 239 aa, Artificial sequence
  synthetic polypeptide S180
YRKREWIKETFYPDIPNPENCKALQFQKSVCEGSSALKTLEMNPCTPNNVEVLETRSAFPKIEDTEIISPVAERPEDRSDAEPENHVVVSYCPPIIEEEIPNPAADEAGGTAQVIYIDVQSMYQPQAKPEEEQENDPVGGAGYKPQMHLPINSTVEDIAAEEDLDKTAGYRPQANVNTWNLVSPDSPRSIDSNSEIVSFGSPCSINSRQFLIPPKDEDSPKSNGGGWSFTNFFQNKPND

SEQ ID NO: 490 - protein, 202 aa, Artificial sequence
  synthetic polypeptide S183
YYHGQRHSDEHHHDDSLPHPQQATDDSGHESDSNSNEGRHHLLVSGAGDGPPLCSQNLGAPGGGPDNGPQDPDNTDDNGPQDPDNTDDNGPHDPLPQDPDNTDDNGPQDPDNTDDNGPHDPLPHSPSDSAGNDGGPPQLTEEVENKGGDQGPPLMTDGGGGHSHDSGHGGGDPHLPTLLLGSSGSGGDDDDPHGPVQLSYYD

SEQ ID NO: 491 - protein, 122 aa, Artificial sequence
  synthetic polypeptide S186
RWQFPAHYRRLRHALWPSLPDLHRVLGQYLRDTAALSPPKATVSDTCEEVEPSLLEILPKSSERTPLPLCSSQAQMDYRRLQPSCLGTMPLSVCPPMAESGSCCTTHIANHSYLPLSYWQQP

SEQ ID NO: 492 - protein, 304 aa, Artificial sequence
  synthetic polypeptide S189
MAAGGPGAGSAAPVSSTSSLPLAALNMRVRRRLSLFLNVRTQVAADWTALAEEMDFEYLEIRQLETQADPTGRLLDAWQGRPGASVGRLLELLTKLGRDDVLLELGPSIEEDCQKYILKQQQEEAEKPLQVAAVDSSVPRTAELAGITTLDDPLGHMPERFDAFICYCPSDIQFVQEMIRQLEQTNYRLKLCVSDRDVLPGTCVWSIASELIEKRLARRPRGGCRRMVVVVSDDYLQSKECDFQTKFALSLSPGAHQKRLIPIKYKAMKKEFPSILRFITVCDYTNPCTKSWFWTRLAKALSLP

SEQ ID NO: 493 - protein, 296 aa, Artificial sequence
  synthetic polypeptide S190
MAAGGPGAGSAAPVSSTSSLPLAALNMRVRRRLSLFLNVRTQVAADWTALAEEMDFEYLEIRQLETQADPTGRLLDAWQGRPGASVGRLLELLTKLGRDDVLLELGPSIEEDCQKYILKQQQEEAEKPLQVAAVDSSVPRTAELAGITTLDDPLGHMPERFDAFICYCPSDIQFVQEMIRQLEQTNYRLKLCVSDRDVLPGTCVWSIASELIEKRCRRMVVVVSDDYLQSKECDFQTKFALSLSPGAHQKRLIPIKYKAMKKEFPSILRFITVCDYTNPCTKSWFWTRLAKALSLP

SEQ ID NO: 494 - protein, 251 aa, Artificial sequence
  synthetic polypeptide S191
MAAGGPGAGSAAPVSSTSSLPLAALNMRVRRRLSLFLNVRTQVAADWTALAEEMDFEYLEIRQLETQADPTGRLLDAWQGRPGASVGRLLELLTKLGRDDVLLELGPSIGHMPERFDAFICYCPSDIQFVQEMIRQLEQTNYRLKLCVSDRDVLPGTCVWSIASELIEKRCRRMVVVVSDDYLQSKECDFQTKFALSLSPGAHQKRLIPIKYKAMKKEFPSILRFITVCDYTNPCTKSWFWTRLAKALSLP

SEQ ID NO: 495 - protein, 191 aa, Artificial sequence
  synthetic polypeptide S192
MAAGGPGAGSAAPVSSTSSLPLAALNMRVRRRLSLFLNVRTQVAADWTALAEEMDFEYLEIRQLETQADPTGRLLDAWQGRPGASVGRLLELLTKLGRDDVLLELGPSIEEDCQKYILKQQQEEAEKPLQVAAVDSSVPRTAELAGITTLDDPLGAAGWWWLSLMITCRARNVTSRPNLHSASLQVPIRSD

SEQ ID NO: 496 - protein, 146 aa, Artificial sequence
  synthetic polypeptide S193
MAAGGPGAGSAAPVSSTSSLPLAALNMRVRRRLSLFLNVRTQVAADWTALAEEMDFEYLEIRQLETQADPTGRLLDAWQGRPGASVGRLLELLTKLGRDDVLLELGPSIGAAGWWWLSLMITCRARNVTSRPNLHSASLQVPIRSD

SEQ ID NO: 497 - protein, 172 aa, Artificial sequence
  synthetic polypeptide S194
MAAGGPGAGSAAPVSSTSSLPLAALNMRVRRRLSLFLNVRTQVAADWTALAEEMDFEYLEIRQLETQADPTGRLLDAWQGRPGASVGRLLELLTKLGRDDVLLELGPSIEEDCQKYILKQQQEEAEKPLQVAAVDSSVPRTAELAGITTLDDPLGHMPERFDAFICYCPSDI

SEQ ID NO: 498 - protein, 127 aa, Artificial sequence
  synthetic polypeptide S195
MAAGGPGAGSAAPVSSTSSLPLAALNMRVRRRLSLFLNVRTQVAADWTALAEEMDFEYLEIRQLETQADPTGRLLDAWQGRPGASVGRLLELLTKLGRDDVLLELGPSIGHMPERFDAFICYCPSDI

SEQ ID NO: 499 - protein, 304 aa, Artificial sequence
  synthetic polypeptide S196
MAAGGPGAGSAAPVSSTSSLPLAALNMRVRRRLSLFLNVRTQVAADWTALAEEMDFEYLEIRQLETQADPTGRLLDAWQGRPGASVGRLLELLTKLGRDDVLLELGPSIEEDCQKYILKQQQEEAEKPLQVAAVDSSVPRTAELAGITTLDDPLGHMPERFDAFICYCPSDIQFVQEMIRQLEQTNYRLKLCVSDRDVLPGTCVWSIASELIEKRLARRPRGGCRRMVVVVSDDYLQSKECDFQTKFALSLSPGAHQKRPIPIKYKAMKKEFPSILRFITVCDYTNPCTKSWFWTRLAKALSLP

SEQ ID NO: 500 - protein, 296 aa, Artificial sequence
  synthetic polypeptide S197
MAAGGPGAGSAAPVSSTSSLPLAALNMRVRRRLSLFLNVRTQVAADWTALAEEMDFEYLEIRQLETQADPTGRLLDAWQGRPGASVGRLLELLTKLGRDDVLLELGPSIEEDCQKYILKQQQEEAEKPLQVAAVDSSVPRTAELAGITTLDDPLGHMPERFDAFICYCPSDIQFVQEMIRQLEQTNYRLKLCVSDRDVLPGTCVWSIASELIEKRCRRMVVVVSDDYLQSKECDFQTKFALSLSPGAHQKRPIPIKYKAMKKEFPSILRFITVCDYTNPCTKSWFWTRLAKALSLP

SEQ ID NO: 501 - protein, 251 aa, Artificial sequence
  synthetic polypeptide S198
MAAGGPGAGSAAPVSSTSSLPLAALNMRVRRRLSLFLNVRTQVAADWTALAEEMDFEYLEIRQLETQADPTGRLLDAWQGRPGASVGRLLELLTKLGRDDVLLELGPSIGHMPERFDAFICYCPSDIQFVQEMIRQLEQTNYRLKLCVSDRDVLPGTCVWSIASELIEKRCRRMVVVVSDDYLQSKECDFQTKFALSLSPGAHQKRPIPIKYKAMKKEFPSILRFITVCDYTNPCTKSWFWTRLAKALSLP

SEQ ID NO: 502 - protein, 218 aa, Artificial sequence
  synthetic polypeptide S199
KSQWIKETCYPDIPDPYKSSILSLIKFKENPHLIIMNVSDCIPDAIEVVSKPEGTKIQFLGTRKSLTETELTKPNYLYLLPTEKNHSGPGPCICFENLTYNQAASDSGSCGHVPVSPKAPSMLGLMTSPENVLKALEKNYMNSLGEIPAGETSLNYVSQLASPMFGDKDSLPTNPVEAPHCSEYKMQMAVSLRLALPPPTENSSLSSITLLDPGEHYC

SEQ ID NO: 503 - protein, 364 aa, Artificial sequence
  synthetic polypeptide S202
KGYSMVTCIFPPVPGPKIKGFDAHLLEKGKSEELLSALGCQDFPPTSDYEDLLVEYLEVDDSEDQHLMSVHSKEHPSQGMKPTYLDPDTDSGRGSCDSPSLLSEKCEEPQANPSTFYDPEVIEKPENPETTHTWDPQCISMEGKIPYFHAGGSKCSTWPLPQPSQHNPRSSYHNITDVCELAVGPAGAPATLLNEAGKDALKSSQTIKSREEGKATQQREVESFHSETDQDTPWLLPQEKTPFGSAKPLDYVEIHKVNKDGALSLLPKQRENSGKPKKPGTPENNKEYAKVSGVMDNNILVLVPDPHAKNVACFEESAKEAPPSLEQNQAEKALANFTATSSKCRLQLGGLDYLDPACFTHSFH

SEQ ID NO: 504 - protein, 42 aa, Artificial sequence
  synthetic polypeptide S211
ALYLLRRDQRLPPDAHKPPGGGSFRTPIQEEQADAHSTLAKI

SEQ ID NO: 505 - protein, 188 aa, Artificial sequence
  synthetic polypeptide S212
HRRACRKRIRQKLHLCYPVQTSQPKLELVDSRPRRSSTQLRSGASVTEPVAEERGLMSQPLMETCHSVGAAYLESLPLQDASPAGGPSSPRDLPEPRVSTEHTNNKIEKIYIMKADTVIVGTVKAELPEGRGLAGPAEPELEEELEADHTPHYPEQETEPPLGSCSDVMLSVEEEGKEDPLPTAASGK

SEQ ID NO: 506 - protein, 42 aa, Artificial sequence; identical to SEQ ID NO: 1
  synthetic polypeptide S213

SEQ ID NO: 507 - protein, 60 aa, Artificial sequence; identical to SEQ ID NO: 10
  synthetic polypeptide S214

SEQ ID NO: 508 - protein, 58 aa, Artificial sequence
  synthetic polypeptide S215
QLGLHIWQLRSQCMWPRETQLLLEVPPSTEDARSCQFPEEERGERSAEEKGRLGDLWV

SEQ ID NO: 509 - protein, 51 aa, Artificial sequence
  synthetic polypeptide S216
QLGLHIWQLRKTQLLLEVPPSTEDARSCQFPEEERGERSAEEKGRLGDLWV

SEQ ID NO: 510 - protein, 23 aa, Artificial sequence
  synthetic polypeptide X001
GSGGSEGGGSEGGAATAGSGSGS

SEQ ID NO: 511 - protein, 152 aa, Artificial sequence
  synthetic polypeptide IL7
DCDIEGKDGKQYESVLMVSIDQLLDSMKEIGSNCLNNEFNFFKRHICDANKEGMFLFRAARKLRQFLKMNSTGDFDLHLLKVSEGTTILLNCTGQVKGRKPAALGEAQPTKSLEENKSLKEQKKLNDLCFLKRLLQEIKTCWNKILMGTKEH

SEQ ID NO: 512 - protein, 10 aa, Artificial sequence
  synthetic polypeptide Flexible linker
GGGGSGGGGS

SEQ ID NO: 513 - protein, 244 aa, Artificial sequence
  synthetic polypeptide IL7RA ECD and TM
ESGYAQNGDLEDAELDDYSFSCYSQLEVNGSQHSLTCAFEDPDVNITNLEFEICGALVEVKCLNFRKLQEIYFIETKKFLLIGKSNICVKVGEKSLTCKKIDLTTIVKPEAPFDLSVVYREGANDFVVTFNTSHLQKKYVKVLMHDVAYRQEKDENKWTHVNLSSTKLTLLQRKLQPAAMYEIKVRSIPDHYFKGFWSEWSPSYYFRTPEINNSSGEMDPILLTISILSFFSVALLVILACVLW

SEQ ID NO: 514 - protein, 286 aa, Artificial sequence; identical to SEQ ID NO: 448
  synthetic polypeptide IL2RB ICD

SEQ ID NO: 515 - DNA, 9 bp, Artificial sequence
  synthetic nucleotide Kozak-type sequence
  misc_feature (7)..(7): n = T or U
  misc_feature (9)..(9): n = G may or may not be present
ccaccangn

SEQ ID NO: 516 - DNA, 9 bp, Artificial sequence
  synthetic nucleotide Kozak-type sequence 2
  misc_feature (7)..(7): n = T or U
  misc_feature (9)..(9): n = G may or may not be present
ccgccangn

SEQ ID NO: 517 - DNA, 13 bp, Artificial sequence
  synthetic nucleotide Kozak-type sequence 3
  misc_feature (11)..(11): n = T or U
  misc_feature (13)..(13): n = G may or may not be present
gccgccgccangn

SEQ ID NO: 518 - DNA, 12 bp, Artificial sequence
  synthetic nucleotide Kozak-type sequence 4
  misc_feature (11)..(11): n = T or U
  misc_feature (12)..(12): n = G may or may not be present
gccgccaccann

SEQ ID NO: 519 - DNA, 9 bp, Artificial sequence
  synthetic nucleotide Kozak sequence
gccgccacc

SEQ ID NO: 520 - DNA, 9 bp, Artificial sequence
  synthetic nucleotide triple stop sequence
taatagtga

SEQ ID NO: 521 - DNA, 191 bp, Artificial sequence
  synthetic nucleotide WPRE
gtcctttccatggctgctcgcctgtgttgccacctggattctgcgcgggacgtccttctgctacgtcccttcggccctcaatccagcggaccttccttcccgcggcctgctgccggctctgcggcctcttccgcgtcttcgccttcgccctcagacgagtcggatctccctttgggccgcctccccgcctg